European Patent Application EP 4 424 376 A2, published September 4, 2024. Title: CHIMERIC ANTIGEN RECEPTORS BASED ON SINGLE-DOMAIN ANTIBODIES AND METHODS OF USE THEREOF. Applicant: Legend Biotech Ireland Limited. The sequence listing filed with the application follows.

SEQUENCE LISTING (277 sequences)

SEQ ID NO: 1 - protein, 5 aa, synthetic construct
  source 1..5: note = CD19 single-domain antibody VHH CDR1
INRMG

SEQ ID NO: 2 - protein, 16 aa, synthetic construct
  source 1..16: note = CD19 single-domain antibody VHH CDR2
SITVRGITNYADSVKG

SEQ ID NO: 3 - protein, 9 aa, synthetic construct
  source 1..9: note = CD19 single-domain antibody VHH CDR3
VSSNRDPDY

SEQ ID NO: 4 - protein, 5 aa, synthetic construct
  source 1..5: note = CD20 single-domain antibody VHH CDR1
IGTMG

SEQ ID NO: 5 - protein, 17 aa, synthetic construct
  source 1..17: note = CD20 single-domain antibody VHH CDR2
AIRWSTGGTRYADSVKG

SEQ ID NO: 6 - protein, 20 aa, synthetic construct
  source 1..20: note = CD20 single-domain antibody VHH CDR3
DRLSLDLSGRYHYNPAVYDY

SEQ ID NO: 7 - protein, 11 aa, synthetic construct
  source 1..11: note = BCMA 269A37346 VHH CDR1
SGFTLDYYAIG

SEQ ID NO: 8 - protein, 11 aa, synthetic construct
  source 1..11: note = BCMA 269A37348 VHH CDR1
SGRTFSTYGMA

SEQ ID NO: 9 - protein, 8 aa, synthetic construct
  source 1..8: note = BCMA 269A37917 VHH CDR1
SGRTFTMG

SEQ ID NO: 10 - protein, 11 aa, synthetic construct
  source 1..11: note = BCMA 269A37355 VHH CDR1
SGGIFVINAMG

SEQ ID NO: 11 - protein, 11 aa, synthetic construct
  source 1..11: note = BCMA 269A37915 VHH CDR1
SGRTFSSIVMG

SEQ ID NO: 12 - protein, 11 aa, synthetic construct
  source 1..11: note = BCMA 269A37936 VHH CDR1
SGFTFDRAVIV

SEQ ID NO: 13 - protein, 11 aa, synthetic construct
  source 1..11: note = BCMA 269A37953 VHH CDR1
STYTVNSDVMG

SEQ ID NO: 14 - protein, 11 aa, synthetic construct
  source 1..11: note = BCMA 269A37965 VHH CDR1
SGATLTNDHMA

SEQ ID NO: 15 - protein, 11 aa, synthetic construct
  source 1..11: note = BCMA 269A37972 VHH CDR1
SGGTLSKNTVA

SEQ ID NO: 16 - protein, 11 aa, synthetic construct
  source 1..11: note = BCMA 269A37353 VHH CDR1
SEHTFSSHVMG

SEQ ID NO: 17 - protein, 11 aa, synthetic construct
  source 1..11: note = BCMA 269A37948 VHH CDR1
SGRAFSTYFMA

SEQ ID NO: 18 - protein, 17 aa, synthetic construct
  source 1..17: note = BCMA 269A37346 VHH CDR2
CISRSDGSTYYADSVKG

SEQ ID NO: 19 - protein, 19 aa, synthetic construct
  source 1..19: note = BCMA 269A37348 VHH CDR2
SKASMNYSGRTYYADSVKG

SEQ ID NO: 20 - protein, 17 aa, synthetic construct
  source 1..17: note = BCMA 269A37917 VHH CDR2
AISLSPTLAYYAESVKG

SEQ ID NO: 21 - protein, 16 aa, synthetic construct
  source 1..16: note = BCMA 269A37355 VHH CDR2
SIRGLGRTNYDDSVKG

SEQ ID NO: 22 - protein, 17 aa, synthetic construct
  source 1..17: note = BCMA 269A37915 VHH CDR2
AIMWNDGITYLQDSVKG

SEQ ID NO: 23 - protein, 17 aa, synthetic construct
  source 1..17: note = BCMA 269A37936 VHH CDR2
FIKPSDGTIYYIDSLKG

SEQ ID NO: 24 - protein, 17 aa, synthetic construct
  source 1..17: note = BCMA 269A37953 VHH CDR2
AIMWNDGITYLQDSVKG

SEQ ID NO: 25 - protein, 17 aa, synthetic construct
  source 1..17: note = BCMA 269A37965 VHH CDR2
AIDWSGRTTNYADPVEG

SEQ ID NO: 26 - protein, 17 aa, synthetic construct
  source 1..17: note = BCMA 269A37972 VHH CDR2
SITWDGRTTYYADSVKG

SEQ ID NO: 27 - protein, 17 aa, synthetic construct
  source 1..17: note = BCMA 269A37353 VHH CDR2
VIGWRDISTSYADSVKG

SEQ ID NO: 28 - protein, 17 aa, synthetic construct
  source 1..17: note = BCMA 269A37948 VHH CDR2
GIAWSGGSTAYADSVKG

SEQ ID NO: 29 - protein, 14 aa, synthetic construct
  source 1..14: note = BCMA 269A37346 VHH CDR3
AGADCSGYLRDYEF

SEQ ID NO: 30 - protein, 18 aa, synthetic construct
  source 1..18: note = BCMA 269A37348 VHH CDR3
AGTGCSTYGCFDAQIIDY

SEQ ID NO: 31 - protein, 13 aa, synthetic construct
  source 1..13: note = BCMA 269A37917 VHH CDR3
ADRKSVMSIRPDY

SEQ ID NO: 32 - protein, 13 aa, synthetic construct
  source 1..13: note = BCMA 269A37355 VHH CDR3
VYVTLLGGVNRDY

SEQ ID NO: 33 - protein, 11 aa, synthetic construct
  source 1..11: note = BCMA 269A37915 VHH CDR3
ASKGRYSEYEY

SEQ ID NO: 34 - protein, 17 aa, synthetic construct
  source 1..17: note = BCMA 269A37936 VHH CDR3
ASPEDWYTDWIDWSIYR

SEQ ID NO: 35 - protein, 11 aa, synthetic construct
  source 1..11: note = BCMA 269A37953 VHH CDR3
ASKGRYSEYEY

SEQ ID NO: 36 - protein, 12 aa, synthetic construct
  source 1..12: note = BCMA 269A37965 VHH CDR3
VLRAWISYDNDY

SEQ ID NO: 37 - protein, 12 aa, synthetic construct
  source 1..12: note = BCMA 269A37972 VHH CDR3
DLGKWPAGPADY

SEQ ID NO: 38 - protein, 11 aa, synthetic construct
  source 1..11: note = BCMA 269A37353 VHH CDR3
ARRIDAADFDS

SEQ ID NO: 39 - protein, 11 aa, synthetic construct
  source 1..11: note = BCMA 269A37948 VHH CDR3
SRGIEVEEFGA

SEQ ID NO: 40 - protein, 11 aa, synthetic construct
  source 1..11: note = CD38 38A37333 VHH CDR1
SGLTFSSYPMM

SEQ ID NO: 41 - protein, 11 aa, synthetic construct
  source 1..11: note = CD38 38A37336 VHH CDR1
SGFTFSSNWMY

SEQ ID NO: 42 - protein, 11 aa, synthetic construct
  source 1..11: note = CD38 38A37699 VHH CDR1
SGRIFSINAMG

SEQ ID NO: 43 - protein, 14 aa, synthetic construct
  source 1..14: note = CD38 38A37331 VHH CDR1
SGSIFKVFRVFAMS

SEQ ID NO: 44 - protein, 11 aa, synthetic construct
  source 1..11: note = CD38 38A37717 VHH CDR1
TGKVFSIYDMG

SEQ ID NO: 45 - protein, 11 aa, synthetic construct
  source 1..11: note = CD38 38A37719 VHH CDR1
SASIFTRLPMG

SEQ ID NO: 46 - protein, 9 aa, synthetic construct
  source 1..9: note = CD38 38A37330 VHH CDR1
SGRAYATMA

SEQ ID NO: 47 - protein, 11 aa, synthetic construct
  source 1..11: note = CD38 38A37334 VHH CDR1
SGLTFSSYIMG

SEQ ID NO: 48 - protein, 11 aa, synthetic construct
  source 1..11: note = CD38 38A37730 VHH CDR1
SQGIFTINAMG

SEQ ID NO: 49 - protein, 11 aa, synthetic construct
  source 1..11: note = CD38 38A37340 VHH CDR1
SGRTFSSYAMA

SEQ ID NO: 50 - protein, 11 aa, synthetic construct
  source 1..11: note = CD38 38A37731 VHH CDR1
SGTIVSISTMG

SEQ ID NO: 51 - protein, 8 aa, synthetic construct
  source 1..8: note = CD38 38A37326 VHH CDR1
SGRTYAMG

SEQ ID NO: 52 - protein, 17 aa, synthetic construct
  source 1..17: note = CD38 38A37333 VHH CDR2
RISDSGGYTNYDDSVKG

SEQ ID NO: 53 - protein, 17 aa, synthetic construct
  source 1..17: note = CD38 38A37336 VHH CDR2
TISTDGRGTYYKDSVKG

SEQ ID NO: 54 - protein, 16 aa, synthetic construct
  source 1..16: note = CD38 38A37699 VHH CDR2
AISTAGSTNYGDSVKG

SEQ ID NO: 55 - protein, 16 aa, synthetic construct
  source 1..16: note = CD38 38A37331 VHH CDR2
SISSGETTTYADSVKG

SEQ ID NO: 56 - protein, 16 aa, synthetic construct
  source 1..16: note = CD38 38A37717 VHH CDR2
EITSSGTTHYDDFVSG

SEQ ID NO: 57 - protein, 16 aa, synthetic construct
  source 1..16: note = CD38 38A37719 VHH CDR2
GIVPSGRINYADSVKG

SEQ ID NO: 58 - protein, 17 aa, synthetic construct
  source 1..17: note = CD38 38A37330 VHH CDR2
HLRVSGDTTYYTDSVKG

SEQ ID NO: 59 - protein, 16 aa, synthetic construct
  source 1..16: note = CD38 38A37334 VHH CDR2
EISSGGMTSYADSVKG

SEQ ID NO: 60 - protein, 16 aa, synthetic construct
  source 1..16: note = CD38 38A37730 VHH CDR2
EVSSGGRTDYADSVKG

SEQ ID NO: 61 - protein, 17 aa, synthetic construct
  source 1..17: note = CD38 38A37340 VHH CDR2
SISTSGGITDYADSVKG

SEQ ID NO: 62 - protein, 16 aa, synthetic construct
  source 1..16: note = CD38 38A37731 VHH CDR2
TITRRGRTNYTDSVKG

SEQ ID NO: 63 - protein, 16 aa, synthetic construct
  source 1..16: note = CD38 38A37326 VHH CDR2
TISGAGNTKYADSVKG

SEQ ID NO: 64 - protein, 6 aa, synthetic construct
  source 1..6: note = CD38 38A37333 VHH CDR3
ILGLPT

SEQ ID NO: 65 - protein, 18 aa, synthetic construct
  source 1..18: note = CD38 38A37336 VHH CDR3
KEPRVLMAYLRNLGDFGS

SEQ ID NO: 66 - protein, 8 aa, synthetic construct
  source 1..8: note = CD38 38A37699 VHH CDR3
LNFPPYVY

SEQ ID NO: 67 - protein, 9 aa, synthetic construct
  source 1..9: note = CD38 38A37331 VHH CDR3
ADHTFTGDF

SEQ ID NO: 68 - protein, 8 aa, synthetic construct
  source 1..8: note = CD38 38A37717 VHH CDR3
NHVFGGSY

SEQ ID NO: 69 - protein, 8 aa, synthetic construct
  source 1..8: note = CD38 38A37719 VHH CDR3
ADTFPLPT

SEQ ID NO: 70 - protein, 19 aa, synthetic construct
  source 1..19: note = CD38 38A37330 VHH CDR3
GPYGILAAARVSNPGNYDY

SEQ ID NO: 71 - protein, 16 aa, synthetic construct
  source 1..16: note = CD38 38A37334 VHH CDR3
APERGSIWYSRYEYKY

SEQ ID NO: 72 - protein, 13 aa, synthetic construct
  source 1..13: note = CD38 38A37730 VHH CDR3
VSGWHVFVGDRIV

SEQ ID NO: 73 - protein, 14 aa, synthetic construct
  source 1..14: note = CD38 38A37340 VHH CDR3
ARTWYLRTSLQYDY

SEQ ID NO: 74 - protein, 14 aa, synthetic construct
  source 1..14: note = CD38 38A37731 VHH CDR3
AEVQLDIWASAYDY

SEQ ID NO: 75 - protein, 11 aa, synthetic construct
  source 1..11: note = CD38 38A37326 VHH CDR3
AGKWFPAANEY

SEQ ID NO: 76 - protein, 117 aa, synthetic construct
  source 1..117: note = CD19 single-domain antibody VHH
QVKLEESGGELVQPGGPLRLSCAASGNIFSINRMGWYRQAPGKQRAFVASITVRGITNYADSVKGRFTISVDKSKNTIYLQMNALKPEDTAVYYCNAVSSNRDPDYWGQGTQVTVSS

SEQ ID NO: 77 - protein, 129 aa, synthetic construct
  source 1..129: note = CD20 single-domain antibody VHH
PVQLVESGGGLVQAGDSLRLSCAASGRTFGIGTMGWFRQPPGKEREFVAAIRWSTGGTRYADSVKGRFTISRDNAKLTVDLQMDSLKPEDTAVYYCAADRLSLDLSGRYHYNPAVYDYWGQGTQVTVSS

SEQ ID NO: 78 - protein, 122 aa, synthetic construct
  source 1..122: note = BCMA 269A37346 VHH
QVQLVESGGGLVQPGGSLRLSCEASGFTLDYYAIGWFRQAPGKEREGVICISRSDGSTYYADSVKGRFTISRDNAKKTVYLQMISLKPEDTAAYYCAAGADCSGYLRDYEFRGQGTQVTVSS

SEQ ID NO: 79 - protein, 128 aa, synthetic construct
  source 1..128: note = BCMA 269A37348 VHH
QVKLEESGGRLVQPRGSLRLSCAGSGRTFSTYGMAWFRQAPGKEREFVASKASMNYSGRTYYADSVKGRFTIARDNAKNMVFLQMNNLKPEDTAVYYCAAGTGCSTYGCFDAQIIDYWGKGTLVTVSS

SEQ ID NO: 80 - protein, 118 aa, synthetic construct
  source 1..118: note = BCMA 269A37917 VHH
EVQLVESGGGLVQAGGSLRLSCAASGRTFTMGWFRQAPGKEREFVAAISLSPTLAYYAESVKGRFTISRDNAKNTVVLQMNSLKPEDTALYYCAADRKSVMSIRPDYWGQGTQVTVSS

SEQ ID NO: 81 - protein, 120 aa, synthetic construct
  source 1..120: note = BCMA 269A37355 VHH
AVQLVDSGGGLVQPGGSLRLSCVASGGIFVINAMGWYRQAPGKQRELVASIRGLGRTNYDDSVKGRFTISRDNANNTVYLQMNSLEPEDTAVYYCTVYVTLLGGVNRDYWGQGTQVTVSS

SEQ ID NO: 82 - protein, 119 aa, synthetic construct
  source 1..119: note = BCMA 269A37915 VHH
EVQLVESGGGLVQAGGSLRLSCAASGRTFSSIVMGWFRQAPGKEREFVGAIMWNDGITYLQDSVKGRFTIFRDNAKNTVYLQMNSLKLEDTAVYYCAASKGRYSEYEYWGQGTQVTVSS

SEQ ID NO: 83 - protein, 128 aa, synthetic construct
  source 1..128: note = BCMA 269A37936 VHH
EVQLVESGGGVVQAGGSLTVSCTASGFTFDRAVIVWFRQAPGKGREGVSFIKPSDGTIYYIDSLKGRFTISSDIAKNTVYLQMKSLESEDSAVYYCAASPEDWYTDWIDWSIYRWQHWGQGTQVTVSS

SEQ ID NO: 84 - protein, 119 aa, synthetic construct
  source 1..119: note = BCMA 269A37953 VHH
EVQLVESGGGMVQAGDSLRLSCVQSTYTVNSDVMGWFRQAPGKEREFVGAIMWNDGITYLQDSVKGRFTIFRDNAKNTVYLQMNSLKLEDTAVYYCAASKGRYSEYEYWGQGTQVTVSS

SEQ ID NO: 85 - protein, 120 aa, synthetic construct
  source 1..120: note = BCMA 269A37965 VHH
AVQLVESGGGLVQAGDSLRLSCTASGATLTNDHMAWFRQAPGKGREFVAAIDWSGRTTNYADPVEGRFTISRNNAKNTVYLEMNSLKLEDTAVYYCAVLRAWISYDNDYWGQGTQVTVSS

SEQ ID NO: 86 - protein, 120 aa, synthetic construct
  source 1..120: note = BCMA 269A37972 VHH
QVQLVESGGGLVQAGGSLRLSCAASGGTLSKNTVAWFRQAPGKERGFVASITWDGRTTYYADSVKGRFTISRDNAKNTVYLQMNSLKPEDTAVYVCADLGKWPAGPADYWGQGTQVTVSS

SEQ ID NO: 87 - protein, 119 aa, synthetic construct
  source 1..119: note = BCMA 269A37353 VHH
QVKLEESGGGLVQAGRSLRLSCAASEHTFSSHVMGWFRQAPGKERESVAVIGWRDISTSYADSVKGRFTISRDNAKKTLYLQMNSLKPEDTAVYYCAARRIDAADFDSWGQGTQVTVSS

SEQ ID NO: 88 - protein, 119 aa, synthetic construct
  source 1..119: note = BCMA 269A37948 VHH
AVQLVESGGGLVQAGDSLRLTCTASGRAFSTYFMAWFRQAPGKEREFVAGIAWSGGSTAYADSVKGRFTISRDNAKNTVYLQMNSLKSEDTAVYYCASRGIEVEEFGAWGQGTQVTVSS

SEQ ID NO: 89 - protein, 114 aa, synthetic construct
  source 1..114: note = CD38 38A37333 VHH
DVQLVESGGGLVQPGGSLRLSCVASGLTFSSYPMMWVRQAPGKGLEWVSRISDSGGYTNYDDSVKGRFTISRDNAKNTLYLQMNSLTPEDTAVYYCRILGLPTTGQGTQVTVSS

SEQ ID NO: 90 - protein, 126 aa, synthetic construct
  source 1..126: note = CD38 38A37336 VHH
EVQLVESGGGLVQPGGSLRLSCAASGFTFSSNWMYWVRQAPGKGLEWVATISTDGRGTYYKDSVKGRFTVSRDNAMSTLLLQMNNLKSEDTAVYYCAKEPRVLMAYLRNLGDFGSWGQGTQVTVSS

SEQ ID NO: 91 - protein, 115 aa, synthetic construct
  source 1..115: note = CD38 38A37699 VHH
QVQLVESGGGLVQAGGSLRLSCAASGRIFSINAMGWYRQAPGKQRELVAAISTAGSTNYGDSVKGRFTISRDNAKNTVYLQMNSLKPEDTAVYYCNLNFPPYVYWGQGTQVTVSS

SEQ ID NO: 92 - protein, 119 aa, synthetic construct
  source 1..119: note = CD38 38A37331 VHH
QVKLEESGGGLVQPGESLRLSCSASGSIFKVFRVFAMSWYRQGPGKQRELVASISSGETTTYADSVKGRFTISRDNAKNTAYLQMDSLKPEDTAVYYCNADHTFTGDFWGQGTQVTVSS

SEQ ID NO: 93 - protein, 116 aa, synthetic construct
  source 1..116: note = CD38 38A37717 VHH
EVQLVESGGGLVQAGGSLRLSCIATGKVFSIYDMGWYRQAPGKQRELVAEITSSGTTHYDDFVSGRFTISRDNAKNTVYLQMNTLKAEDTAVYYCRANHVFGGSYWGQGTQVTVSS

SEQ ID NO: 94 - protein, 115 aa, synthetic construct
  source 1..115: note = CD38 38A37719 VHH
QVKLEESGGGSVQTGGSLRLSCAASASIFTRLPMGWYRQAPGKQRELVVGIVPSGRINYADSVKGRFTISRDNAKNTVYLQMNSLRPEDTAVYYCRADTFPLPTWGQGTQVTVSS

SEQ ID NO: 95 - protein, 126 aa, synthetic construct
  source 1..126: note = CD38 38A37330 VHH
QVQLVESGGGLVQAGDSLRLSCAASGRAYATMAWFRQAPGKEREFVAHLRVSGDTTYYTDSVKGRFTISRDNAKNTAYLQMNMLKPEDTAVYYCAAGPYGILAAARVSNPGNYDYWGQGTQVTVSS

SEQ ID NO: 96 - protein, 123 aa, synthetic construct
  source 1..123: note = CD38 38A37334 VHH
EVQLVESGGGLVQAGGSLRLSCAASGLTFSSYIMGWFRQAPGEERELVAEISSGGMTSYADSVKGRFTISRDNAKKTGYLQMNSLKPEDTAVYYCAAPERGSIWYSRYEYKYWGQGTQVTVSS

SEQ ID NO: 97 - protein, 120 aa, synthetic construct
  source 1..120: note = CD38 38A37730 VHH
AVQLVDSGGGLAQTGGSLRLSCAASQGIFTINAMGWYRQVPGKQRELVAEVSSGGRTDYADSVKGRFTISRDNAKNTVYLQMNSLKPEDTGVYYCRVSGWHVFVGDRIVWGQGTLVTVSS

SEQ ID NO: 98 - protein, 123 aa, synthetic construct
  source 1..123: note = CD38 38A37340 VHH
DVQLVESGGGLVQAGDSLRLSCAASGRTFSSYAMAWFRQAPGKEREIVSSISTSGGITDYADSVKGRFTISKDSAKMNTVYLQMNSLEPEDTAVYYCAARTWYLRTSLQYDYWGQGTQVTVSS

SEQ ID NO: 99 - protein, 121 aa, synthetic construct
  source 1..121: note = CD38 38A37731 VHH
QVKLEESGGGLVQAGGSLRLSCVASGTIVSISTMGWYRQAPGKQRELVATITRRGRTNYTDSVKGRFTISRDNAKNTVYLQMNSLKPEDTAVYYCNAEVQLDIWASAYDYWGQGTQVTVAS

SEQ ID NO: 100 - protein, 115 aa, synthetic construct
  source 1..115: note = CD38 38A37326 VHH
EVQLVESGGGLVQAGGSLRLSCAASGRTYAMGWYRQAPGKQRDLVATISGAGNTKYADSVKGRFTISRDNAKNTMYLQMNSLKPEDTAVYYCAAGKWFPAANEYWGQGTQVTVSS

SEQ ID NO: 101 - DNA, 351 bp, synthetic construct
  source 1..351: mol_type = other DNA; note = CD19 single-domain antibody VHH
caggtaaagctggaggagtctgggggagaattggtgcagcctggggggcctctgagactctcctgtgcagcctcgggaaacatcttcagtatcaatcgcatgggctggtaccgccaggctccagggaagcagcgcgcgttcgtcgcatctattactgttcgtggtataacaaactatgcagactccgtgaagggccgattcaccatttctgtagacaagtccaaaaacacgatttatctgcagatgaacgcactcaaacctgaggacacggccgtctattattgtaatgcagtgtcttcaaacagggaccccgactactggggccaggggacccaggtcaccgtctcctca

SEQ ID NO: 102 - DNA, 387 bp, synthetic construct
  source 1..387: mol_type = other DNA; note = CD20 single-domain antibody VHH
ccggtgcagctggtggagtctgggggaggcttggtgcaggctggggattctctgagactctcctgtgctgcctctggacgcaccttcggtattggtaccatgggctggttccgccaacctccagggaaggagcgtgaatttgtagcagctattaggtggagtactggtggcactcgctatgcagactccgtgaagggccgattcaccatctcccgagacaacgccaagctcacggtagatctgcaaatggacagcctgaaacctgaagacacggccgtttattactgtgcagcagatagactgtcccttgatttaagtggtcgttaccactacaaccccgccgtgtatgactattggggccaggggacccaggtcaccgtctcctca

SEQ ID NO: 103 - DNA, 366 bp, synthetic construct
  source 1..366: mol_type = other DNA; note = BCMA 269A37346 VHH
caggtgcagctggtggagtctgggggaggcttggtgcagcctgggggttctctgaggctctcctgtgaagcctctggattcactttggattattatgccataggctggttccgccaggccccagggaaggagcgcgagggggtcatatgtattagtagaagtgatggtagcacatactatgcagactccgtgaagggccgattcaccatctccagagacaacgccaagaaaacggtgtatctgcaaatgatcagcctgaaacctgaggacacggccgcttattactgtgcagcaggggccgattgttcggggtacctacgagattatgagttccgggggcaggggacccaggtcaccgtctcctca

SEQ ID NO: 104 - DNA, 384 bp, synthetic construct
  source 1..384: mol_type = other DNA; note = BCMA 269A37348 VHH
caggtaaagctggaggagtctgggggacgattggtgcagccaaggggctctctgagactctcctgtgcaggctctggacgcactttcagtacctatggtatggcctggttccgccaggctccagggaaggagcgtgagttcgtagcgtctaaagcatcgatgaattacagcggtagaacatactatgcagactccgtgaagggccgattcaccatcgccagagacaacgccaagaacatggtgtttctgcaaatgaacaacctgaagcctgaggacacggccgtttattactgtgcagcgggcactggatgctcaacatatgggtgttttgacgcccagataatagactactggggcaaagggaccctggtcaccgtctcctca

SEQ ID NO: 105 - DNA, 354 bp, synthetic construct
  source 1..354: mol_type = other DNA; note = BCMA 269A37917 VHH
gaggtgcagctggtggagtctgggggaggcttggtgcaggctggggggtctctgagactctcctgtgcagcctctggacgcaccttcaccatggggtggttccgtcaggctccagggaaggagcgtgagtttgtagcagctattagtttgagtcctactttagcatattatgcagagtccgtgaagggccgattcaccatcagccgagacaacgccaagaacacggtggttttgcaaatgaacagcctgaaacctgaggacacggccctttattactgtgcagcagaccggaaatcagtaatgtctattcggcccgactactggggccaggggacccaggtcaccgtctcctca

SEQ ID NO: 106 - DNA, 360 bp, synthetic construct
  source 1..360: mol_type = other DNA; note = BCMA 269A37355 VHH
gccgtgcagctggtggattctgggggaggcttggtgcagcctggggggtctctgagactctcctgtgtagcctctggaggtatcttcgtcatcaatgccatgggctggtaccgccaggctccaggaaagcagcgcgagttggtcgcatctattcgtggactaggcagaacaaactatgacgactccgtgaagggccgattcaccatctccagagacaacgccaacaacacggtgtatctgcagatgaacagcctggaacctgaggacacggccgtctactactgtacagtctacgttacactacttggtggggttaatagggactactggggccaggggacccaggtcaccgtctcctca

SEQ ID NO: 107 - DNA, 357 bp, synthetic construct
  source 1..357: mol_type = other DNA; note = BCMA 269A37915 VHH
gaggtgcagctggtggagtctgggggaggattggtgcaggctgggggctctctgagactctcctgtgcagcctctggacggaccttcagtagcattgtcatgggctggttccgccaggctccagggaaggagcgtgagtttgtaggagcgattatgtggaatgatggtattacatacttgcaagactccgtgaagggccgatttaccatcttcagagacaatgccaagaacacggtgtatctgcaaatgaacagcctgaaacttgaggatacggccgtttattactgtgcagcatccaagggtagatactcggaatatgagtactggggccaggggacccaggtcaccgtctcctca

SEQ ID NO: 108 - DNA, 384 bp, synthetic construct
  source 1..384: mol_type = other DNA; note = BCMA 269A37936 VHH
gaggtgcagctggtggagtctgggggaggcgtggtgcaggctggggggtctctgacagtctcctgtacagcctctggattcactttcgaccgtgctgtcatagtctggttccgccaggcccccgggaagggccgtgagggggtctcatttattaaacctagtgatggcaccatatactacattgactccctgaagggccgattcacgatctccagtgacatcgccaagaatacggtatatctgcaaatgaaaagtctggaatcggaggactcggccgtttattactgtgcggcctcgcctgaggactggtacacggattggatcgactggagtatatatcggtggcagcactggggccaggggacccaggtcactgtctcctca

SEQ ID NO: 109 - DNA, 357 bp, synthetic construct
  source 1..357: mol_type = other DNA; note = BCMA 269A37953 VHH
gaggtgcagctggtggagtctgggggaggaatggtgcaggctggggactctctgagactatcctgtgtgcagtctacttacaccgtcaatagcgatgtcatgggctggttccgccaggctccagggaaggagcgtgagtttgtaggagcgattatgtggaatgatggtattacatacttgcaagactccgtgaagggccgatttaccatcttcagagacaacgccaagaacacggtgtatctgcaaatgaacagcctgaaacttgaggatacggccgtttattactgtgcagcatccaagggtagatactcggaatatgagtactggggccaggggacccaggtcaccgtctcctca

SEQ ID NO: 110 - DNA, 360 bp, synthetic construct
  source 1..360: mol_type = other DNA; note = BCMA 269A37965 VHH
gcggtgcagctggtggagtctgggggaggattggtgcaggctggggactctctgagactctcctgtacagcctctggtgcaaccttgactaacgatcacatggcatggttccgccaggctccagggaaggggcgtgaatttgtagcagctattgactggagtggtcgtaccacaaattacgcagaccccgtagagggccgattcaccatctccagaaacaacgccaagaacacggtgtatctggaaatgaacagcctgaaacttgaggacacggccgtttattactgtgcggtcctccgcgcttggatctcatatgacaatgactactggggccaggggacccaggtcaccgtctcctca

SEQ ID NO: 111 - DNA, 360 bp, synthetic construct
  source 1..360: mol_type = other DNA; note = BCMA 269A37972 VHH
caggtgcagctggtggagtctgggggaggattggtgcaggctgggggctctctgagactctcctgtgcagcctctggaggcaccttaagtaaaaataccgtggcttggttccgccaggctccagggaaggagcgtgggtttgtagcgtctattacctgggatggtcgtacgacatactatgcagactccgtgaagggccgattcaccatctccagagacaacgccaagaacacagtgtatctgcaaatgaacagcctgaaacctgaggatacggccgtttatgtctgtgcagacttagggaaatggcctgcgggcccggcggactactggggccaggggacccaggtcaccgtctcctca

SEQ ID NO: 112 - DNA, 357 bp, synthetic construct
  source 1..357: mol_type = other DNA; note = BCMA 269A37353 VHH
caggtaaagctggaggagtctgggggaggcttggtgcaggctgggcggtctctgagactctcctgtgcagcctctgaacacaccttcagtagccatgtcatgggctggttccgccaggctccagggaaggagcgtgagtctgttgcagttattggctggagagatattagcacaagctatgcagactccgtgaagggccgattcaccatctccagagacaacgccaagaagacgctgtatctgcaaatgaatagcctgaaacctgaggacacggccgtttactactgtgcagcacgtcggatcgacgcagctgactttgattcctgggggcaggggacccaggtcaccgtctcctcg

SEQ ID NO: 113 - DNA, 357 bp, synthetic construct
  source 1..357: mol_type = other DNA; note = BCMA 269A37948 VHH
gcggtgcagctggtggagtctgggggaggattggtgcaggctggggactctctgagactcacctgtacagcctctggacgcgccttcagtacctatttcatggcctggttccgccaggctccagggaaggagcgtgagtttgtagcaggaattgcatggagtggtggtagcacggcgtatgcagactccgtgaagggccgattcaccatctccagagacaacgccaagaacacggtgtatctgcaaatgaacagcctgaaatctgaggacacggccgtttattactgtgccagcagggggattgaggtcgaagagtttggtgcctggggccaggggacccaggtcaccgtctcgtcg

SEQ ID NO: 114 - DNA, 342 bp, synthetic construct
  source 1..342: mol_type = other DNA; note = CD38 38A37333 VHH
gatgtgcagctggtggagtctgggggaggcttggtgcagcctggggggtctctgagactctcctgtgtagcctctggattgaccttcagtagctaccccatgatgtgggtccgccaggctccaggaaaggggctcgagtgggtctcacgtattagcgatagtggtggttacacaaactatgacgactccgtgaagggccgattcaccatctccagagacaacgccaagaacacgctgtatctgcaaatgaacagcctgacacctgaggacacggccgtgtattactgtagaatcctggggttgcccaccacgggccaggggacccaggtcaccgtctcctca

SEQ ID NO: 115 - DNA, 378 bp, synthetic construct
  source 1..378: mol_type = other DNA; note = CD38 38A37336 VHH
gaggtgcagctggtggagtctgggggaggcctggtgcagcctggggggtctctgagactctcctgtgcagcctctggattcaccttcagtagcaactggatgtattgggtccgtcaggctccagggaaggggctcgagtgggtcgcaactattagtactgatggtcgtggaacatactataaagactctgtgaagggccgattcaccgtctccagagacaacgccatgagtacgctgcttctgcaaatgaacaatctgaaatctgaagatacggccgtgtattattgtgcaaaagagccgagggtgttgatggcttacctgcggaacctgggtgactttggttcctggggccaggggacccaggtcaccgtctcctcg

SEQ ID NO: 116 - DNA, 345 bp, synthetic construct
  source 1..345: mol_type = other DNA; note = CD38 38A37699 VHH
caggtgcagctggtggagtctgggggaggcttggtgcaggctggggggtctctgagactctcctgtgcagcctctggaaggatcttcagtatcaatgccatgggctggtaccgccaggctccagggaagcagcgcgagttggtcgccgctattagtacggctggtagcacaaactatggagactccgtgaagggccgattcaccatctccagagacaacgccaagaacacggtgtatctgcaaatgaacagcctgaaacctgaggacacagctgtttattactgtaatttaaattttcccccgtatgtgtactggggccaggggacccaggtcaccgtctcctca

SEQ ID NO: 117 - DNA, 357 bp, synthetic construct
  source 1..357: mol_type = other DNA; note = CD38 38A37331 VHH
caggtaaagctggaggagtctgggggaggtctggtgcagcctggggagtctctgagactctcctgttcagcctctggaagcatcttcaaagttttcagagtctttgccatgagctggtaccgccagggtcccgggaaacagcgcgagttggtcgcatccattagtagtggcgagaccacaacctatgcagactccgtgaagggccgattcaccatctccagagacaacgccaagaatacggcgtatctgcaaatggacagcctgaaacctgaggacacggccgtctattactgtaatgcggatcacacctttacaggagacttctggggccaggggacccaggtcaccgtctcctca

SEQ ID NO: 118 - DNA, 348 bp, synthetic construct
  source 1..348: mol_type = other DNA; note = CD38 38A37717 VHH
gaggtgcagctggtggaaagcggggggggactggtgcaggcaggcgggtcactgagactgtcatgtatcgcaactgggaaggtgtttagcatctacgacatgggctggtataggcaggcaccaggaaagcagagggagctggtggccgagatcaccagctccggcaccacacactacgacgatttcgtgtctggccggtttaccatcagcagagacaacgccaagaatacagtgtatctgcagatgaacaccctgaaggccgaggatacagccgtgtactattgccgggctaatcacgtcttcggcggctcctactgggggcagggaactcaggtcactgtgtcatcc

SEQ ID NO: 119 - DNA, 345 bp, synthetic construct
  source 1..345: mol_type = other DNA; note = CD38 38A37719 VHH
caggtaaagctggaggagtctgggggaggctcggtgcagactggggggtctctgagactctcctgtgcagcctctgcaagcatcttcactaggctgcccatgggctggtaccgccaggctccagggaagcagcgcgagttggtcgtaggcattgttcctagtggtaggataaactatgcagactccgtgaagggccgattcaccatctccagagacaacgccaagaacacggtgtatctgcaaatgaacagcctgcgccctgaggacacagccgtctattactgccgcgccgataccttccccttgcccacctggggccaggggacccaggtcaccgtctcctca

SEQ ID NO: 120 - DNA, 378 bp, synthetic construct
  source 1..378: mol_type = other DNA; note = CD38 38A37330 VHH
caggtgcagctggtggagtctgggggaggattggtgcaggctggggactctctgagactctcctgtgcagcctctggacgcgcctacgctacgatggcctggttccgccaggctccagggaaggagcgtgagtttgtagcacatctgcgcgtgagtggtgataccacttactatacagactccgtgaagggccgattcaccatctccagagacaacgccaagaacacggcgtatctgcaaatgaacatgttgaaacctgaggacacggccgtttattactgtgcagcgggaccgtatggcattcttgccgctgccagggtcagtaatccaggaaattatgattattggggccaggggacccaggtcaccgtctcctca

SEQ ID NO: 121 - DNA, 369 bp, synthetic construct
  source 1..369: mol_type = other DNA; note = CD38 38A37334 VHH
gaggtgcagctggtggagtctgggggaggattggtgcaggctgggggctctctgagactctcctgtgcagcctctggactcaccttcagtagttatattatgggctggttccgccaggctccaggcgaggagcgcgagttggtcgcggaaattagtagcggtggtatgacatcgtatgcagactccgtgaagggccgattcaccatctccagagacaacgccaagaagacggggtatctgcaaatgaacagcctgaaacctgaggacacggccgtttactattgtgcagcccctgagaggggtagtatctggtacagccgctacgaatataagtactggggccaggggacccaggtcaccgtctcctca

SEQ ID NO: 122 - DNA, 360 bp, synthetic construct
  source 1..360: mol_type = other DNA; note = CD38 38A37730 VHH
gccgtgcagctggtggattctgggggaggcttggcgcagactggggggtctctgagactctcctgtgcagcctctcaagggatcttcactatcaatgccatgggctggtaccgccaggttccagggaagcagcgggagttggtcgcagaagttagtagtggtggccgcacagactatgcagactccgtgaagggccgattcaccatctccagagacaacgccaagaacacggtgtacctgcaaatgaacagcctgaaacctgaggacacaggcgtctattattgtcgagtttctggatggcatgtgtttgtcggtgaccgcatagtttggggccagggcaccctggtcactgtctcctca

SEQ ID NO: 123 - DNA, 369 bp, synthetic construct
  source 1..369: mol_type = other DNA; note = CD38 38A37340 VHH
gatgtgcagctggtggagtctgggggaggattggtgcaggctggggactctctgagactctcctgtgcagcctctggacgcaccttcagtagctatgccatggcctggttccgccaggctccagggaaggagcgtgagattgtttcgtctatcagtaccagtggtggtatcacagactatgcagactccgtgaagggccgattcaccatctccaaagacagcgcgaagatgaacacggtgtatctgcaaatgaatagcctagaacctgaggacacggccgtttactactgtgcggcccgtacatggtaccttcgtacttctctccaatatgactattggggccaggggacccaggtcaccgtctcctca

SEQ ID NO: 124 - DNA, 363 bp, synthetic construct
  source 1..363: mol_type = other DNA; note = CD38 38A37731 VHH
caggtaaagctggaggagtctgggggaggcttggtgcaggctggggggtctctgagactctcctgtgtagcctctggaaccatcgtcagtatcagtaccatgggctggtaccgccaggctccagggaagcagcgcgagttggtcgcgactataaccaggcgtggacgcacgaactatacagactccgtgaagggccgattcaccatctccagagacaacgccaaaaacacggtgtatctgcaaatgaacagcctgaaacctgaggacacagccgtctattactgtaatgcagaggtgcaactggatatatgggcatctgcgtatgactactggggccaggggacccaggtcaccgtcgcctca

SEQ ID NO: 125 - DNA, 345 bp, synthetic construct
  source 1..345: mol_type = other DNA; note = CD38 38A37326 VHH
gaggtgcagctggtggagtctgggggaggattggtgcaggctgggggctctctgagactctcctgtgcagcctctggacgcacctatgccatgggctggtatcgccaggctccagggaagcagcgcgacttggtcgcaactattagtggtgcgggtaacacaaagtatgcagactccgtgaagggccgattcaccatctccagagacaacgccaagaacacaatgtatctgcaaatgaacagcctgaaacctgaggacacggccgtttattactgtgccgcgggtaaatggttccctgctgcgaatgagtactggggccaggggacccaggtcaccgtctcctca

SEQ ID NO: 126 - skipped

SEQ ID NO: 127 - protein, 21 aa, synthetic construct
  source 1..21: note = CD8alpha signal peptide
MALPVTALLLPLALLLHAARP

SEQ ID NO: 128 - DNA, 63 bp, synthetic construct
  source 1..63: mol_type = other DNA; note = CD8alpha signal peptide nucleic acid sequence 1
atggccttaccagtgaccgccttgctcctgccgctggccttgctgctccacgccgccaggccg

SEQ ID NO: 129 - DNA, 63 bp, synthetic construct
  source 1..63: mol_type = other DNA; note = CD8alpha signal peptide nucleic acid sequence 2
atggctctgcccgtcactgctctgctgctgcccctggctctgctgctgcacgccgcaagaccc

SEQ ID NO: 130 - protein, 45 aa, synthetic construct
  source 1..45: note = CD8alpha hinge
TTTPAPRPPTPAPTIASQPLSLRPEACRPAAGGAVHTRGLDFACD

SEQ ID NO: 131 - DNA, 135 bp, synthetic construct
  source 1..135: mol_type = other DNA; note = CD8alpha hinge
accacgacgccagcgccgcgaccaccaacaccggcgcccaccatcgcgtcgcagcccctgtccctgcgcccagaggcgtgccggccagcggcggggggcgcagtgcacacgagggggctggacttcgcctgtgat

SEQ ID NO: 132 - protein, 24 aa, synthetic construct
  source 1..24: note = CD8alpha transmembrane
IYIWAPLAGTCGVLLLSLVITLYC

SEQ ID NO: 133 - protein, 27 aa, synthetic construct
  source 1..27: note = CD28 transmembrane
FWVLVVVGGVLACYSLLVTVAFIIFWV

SEQ ID NO: 134 - DNA, 72 bp, synthetic construct
  source 1..72: mol_type = other DNA; note = CD8alpha transmembrane
atctacatctgggcgcccttggccgggacttgtggggtccttctcctgtcactggttatcaccctttactgc

SEQ ID NO: 135 - DNA, 81 bp, synthetic construct
  source 1..81: mol_type = other DNA; note = CD28 transmembrane
ttttgggtgctggtggtggttggtggagtcctggcttgctatagcttgctagtaacagtggcctttattattttctgggtg

SEQ ID NO: 136 - protein, 41 aa, synthetic construct
  source 1..41: note = CD28 cytoplasmic aa sequence
RSKRSRLLHSDYMNMTPRRPGPTRKHYQPYAPPRDFAAYRS

SEQ ID NO: 137 - protein, 42 aa, synthetic construct
  source 1..42: note = CD137 cytoplasmic domain
KRGRKKLLYIFKQPFMRPVQTTQEEDGCSCRFPEEEEGGCEL

SEQ ID NO: 138 - DNA, 123 bp, synthetic construct
  source 1..123: mol_type = other DNA; note = CD28 cytoplasmic na sequence
aggagtaagaggagcaggctcctgcacagtgactacatgaacatgactccccgccgccccgggcccacccgcaagcattaccagccctatgccccaccacgcgacttcgcagcctatcgctcc

SEQ ID NO: 139 - DNA, 126 bp, synthetic construct
  source 1..126: mol_type = other DNA; note = CD137 cytoplasmic domain
aaacggggcagaaagaaactcctgtatatattcaaacaaccatttatgagaccagtacaaactactcaagaggaagatggctgtagctgccgatttccagaagaagaagaaggaggatgtgaactg

SEQ ID NO: 140 - protein, 113 aa, synthetic construct
  source 1..113: note = wt CD3z cytoplasmic domain
RVKFSRSADAPAYQQGQNQLYNELNLGRREEYDVLDKRRGRDPEMGGKPQRRKNPQEGLYNELQKDKMAEAYSEIGMKGERRRGKGHDGLYQGLSTATKDTYDALHMQALPPR

SEQ ID NO: 141 - protein, 113 aa, synthetic construct
  source 1..113: note = Q65K CD3z cytoplasmic domain
RVKFSRSADAPAYKQGQNQLYNELNLGRREEYDVLDKRRGRDPEMGGKPQRRKNPQEGLYNELQKDKMAEAYSEIGMKGERRRGKGHDGLYQGLSTATKDTYDALHMQALPPR

SEQ ID NO: 142 - DNA, 336 bp, synthetic construct
  source 1..336: mol_type = other DNA; note = wt CD3z cytoplasmic domain
agagtgaagttcagcaggagcgcagacgcccccgcgtaccagcagggccagaaccagctctataacgagctcaatctaggacgaagagaggagtacgatgttttggacaagagacgtggccgggaccctgagatggggggaaagccgagaaggaagaaccctcaggaaggcctgtacaatgaactgcagaaagataagatggcggaggcctacagtgagattgggatgaaaggcgagcgccggaggggcaaggggcacgatggcctttaccagggtctcagtacagccaccaaggacacctacgacgcccttcacatgcaggccctgccccctcgc

SEQ ID NO: 143 - DNA, 336 bp, synthetic construct
  source 1..336: mol_type = other DNA; note = Q65K CD3z cytoplasmic domain
agagtgaagttcagcaggagcgcagacgcccccgcgtacaagcagggccagaaccagctctataacgagctcaatctaggacgaagagaggagtacgatgttttggacaagagacgtggccgggaccctgagatggggggaaagccgagaaggaagaaccctcaggaaggcctgtacaatgaactgcagaaagataagatggcggaggcctacagtgagattgggatgaaaggcgagcgccggaggggcaaggggcacgatggcctttaccagggtctcagtacagccaccaaggacacctacgacgcccttcacatgcaggccctgccccctcgc

SEQ ID NO: 144 - protein, 5 aa, synthetic construct
  source 1..5: note = linker sequence 1
GGGGS

SEQ ID NO: 145 - protein, 10 aa, synthetic construct
  source 1..10: note = linker sequence 2
GGGGSGGGGS

SEQ ID NO: 146 - protein, 16 aa, synthetic construct
  source 1..16: note = linker sequence 3
GGGSGGGSGGGSGGGS

SEQ ID NO: 147 - protein, 24 aa, synthetic construct
  source 1..24: note = linker sequence 4
GGGGSGGGGSGGGGGGSGSGGGGS

SEQ ID NO: 148 - protein, 34 aa, synthetic construct
  source 1..34: note = linker sequence 5
GGGGSGGGGSGGGGGGSGSGGGGSGGGGSGGGGS

SEQ ID NO: 149 - protein, 15 aa, synthetic construct
  source 1..15: note = Linker sequence 6
GGGGSGGGGSGGGGS

SEQ ID NO: 150 - protein, 20 aa, synthetic construct
  source 1..20: note = Linker sequence 7
GGGGSGGGGSGGGGSGGGGS

SEQ ID NO: 151 - protein, 25 aa, synthetic construct
  source 1..25: note = Linker sequence 8
GGGGSGGGGSGGGGSGGGGSGGGGS

SEQ ID NO: 152 - protein, 420 aa, synthetic construct
  source 1..420: note = BCMA 269A37346 CAR
MALPVTALLLPLALLLHAARPVNRTRRMHQVQLVESGGGLVQPGGSLRLSCEASGFTLDYYAIGWFRQAPGKEREGVICISRSDGSTYYADSVKGRFTISRDNAKKTVYLQMISLKPEDTAAYYCAAGADCSGYLRDYEFRGQGTQVTVSSTSTTTPAPRPPTPAPTIASQPLSLRPEACRPAAGGAVHTRGLDFACDFWVLVVVGGVLACYSLLVTVAFIIFWVRSKRSRLLHSDYMNMTPRRPGPTRKHYQPYAPPRDFAAYRSKRGRKKLLYIFKQPFMRPVQTTQEEDGCSCRFPEEEEGGCELRVKFSRSADAPAYKQGQNQLYNELNLGRREEYDVLDKRRGRDPEMGGKPRRKNPQEGLYNELQKDKMAEAYSEIGMKGERRRGKGHDGLYQGLSTATKDTYDALHMQALPPR

SEQ ID NO: 153 - protein, 426 aa, synthetic construct
  source 1..426: note = BCMA 269A37348 CAR
MALPVTALLLPLALLLHAARPVNRTRRMHQVKLEESGGRLVQPRGSLRLSCAGSGRTFSTYGMAWFRQAPGKEREFVASKASMNYSGRTYYADSVKGRFTIARDNAKNMVFLQMNNLKPEDTAVYYCAAGTGCSTYGCFDAQIIDYWGKGTLVTVSSTSTTTPAPRPPTPAPTIASQPLSLRPEACRPAAGGAVHTRGLDFACDFWVLVVVGGVLACYSLLVTVAFIIFWVRSKRSRLLHSDYMNMTPRRPGPTRKHYQPYAPPRDFAAYRSKRGRKKLLYIFKQPFMRPVQTTQEEDGCSCRFPEEEEGGCELRVKFSRSADAPAYKQGQNQLYNELNLGRREEYDVLDKRRGRDPEMGGKPRRKNPQEGLYNELQKDKMAEAYSEIGMKGERRRGKGHDGLYQGLSTATKDTYDALHMQALPPR

SEQ ID NO: 154 - protein, 416 aa, synthetic construct
  source 1..416: note = BCMA 269A37917 CAR
MALPVTALLLPLALLLHAARPVNRTRRMHEVQLVESGGGLVQAGGSLRLSCAASGRTFTMGWFRQAPGKEREFVAAISLSPTLAYYAESVKGRFTISRDNAKNTVVLQMNSLKPEDTALYYCAADRKSVMSIRPDYWGQGTQVTVSSTSTTTPAPRPPTPAPTIASQPLSLRPEACRPAAGGAVHTRGLDFACDFWVLVVVGGVLACYSLLVTVAFIIFWVRSKRSRLLHSDYMNMTPRRPGPTRKHYQPYAPPRDFAAYRSKRGRKKLLYIFKQPFMRPVQTTQEEDGCSCRFPEEEEGGCELRVKFSRSADAPAYKQGQNQLYNELNLGRREEYDVLDKRRGRDPEMGGKPRRKNPQEGLYNELQKDKMAEAYSEIGMKGERRRGKGHDGLYQGLSTATKDTYDALHMQALPPR

SEQ ID NO: 155 - protein, 418 aa, synthetic construct
  source 1..418: note = BCMA 269A37355 CAR
MALPVTALLLPLALLLHAARPVNRTRRMHAVQLVDSGGGLVQPGGSLRLSCVASGGIFVINAMGWYRQAPGKQRELVASIRGLGRTNYDDSVKGRFTISRDNANNTVYLQMNSLEPEDTAVYYCTVYVTLLGGVNRDYWGQGTQVTVSSTSTTTPAPRPPTPAPTIASQPLSLRPEACRPAAGGAVHTRGLDFACDFWVLVVVGGVLACYSLLVTVAFIIFWVRSKRSRLLHSDYMNMTPRRPGPTRKHYQPYAPPRDFAAYRSKRGRKKLLYIFKQPFMRPVQTTQEEDGCSCRFPEEEEGGCELRVKFSRSADAPAYKQGQNQLYNELNLGRREEYDVLDKRRGRDPEMGGKPRRKNPQEGLYNELQKDKMAEAYSEIGMKGERRRGKGHDGLYQGLSTATKDTYDALHMQALPPR

SEQ ID NO: 156 - protein, 417 aa, synthetic construct
  source 1..417: note = BCMA 269A37915 CAR
MALPVTALLLPLALLLHAARPVNRTRRMHEVQLVESGGGLVQAGGSLRLSCAASGRTFSSIVMGWFRQAPGKEREFVGAIMWNDGITYLQDSVKGRFTIFRDNAKNTVYLQMNSLKLEDTAVYYCAASKGRYSEYEYWGQGTQVTVSSTSTTTPAPRPPTPAPTIASQPLSLRPEACRPAAGGAVHTRGLDFACDFWVLVVVGGVLACYSLLVTVAFIIFWVRSKRSRLLHSDYMNMTPRRPGPTRKHYQPYAPPRDFAAYRSKRGRKKLLYIFKQPFMRPVQTTQEEDGCSCRFPEEEEGGCELRVKFSRSADAPAYKQGQNQLYNELNLGRREEYDVLDKRRGRDPEMGGKPRRKNPQEGLYNELQKDKMAEAYSEIGMKGERRRGKGHDGLYQGLSTATKDTYDALHMQALPPR

SEQ ID NO: 157 - protein, 426 aa, synthetic construct
  source 1..426: note = BCMA 269A37936 CAR
MALPVTALLLPLALLLHAARPVNRTRRMHEVQLVESGGGVVQAGGSLTVSCTASGFTFDRAVIVWFRQAPGKGREGVSFIKPSDGTIYYIDSLKGRFTISSDIAKNTVYLQMKSLESEDSAVYYCAASPEDWYTDWIDWSIYRWQHWGQGTQVTVSSTSTTTPAPRPPTPAPTIASQPLSLRPEACRPAAGGAVHTRGLDFACDFWVLVVVGGVLACYSLLVTVAFIIFWVRSKRSRLLHSDYMNMTPRRPGPTRKHYQPYAPPRDFAAYRSKRGRKKLLYIFKQPFMRPVQTTQEEDGCSCRFPEEEEGGCELRVKFSRSADAPAYKQGQNQLYNELNLGRREEYDVLDKRRGRDPEMGGKPRRKNPQEGLYNELQKDKMAEAYSEIGMKGERRRGKGHDGLYQGLSTATKDTYDALHMQALPPR

SEQ ID NO: 158 - protein, 417 aa, synthetic construct
  source 1..417: note = BCMA 269A37953 CAR
MALPVTALLLPLALLLHAARPVNRTRRMHEVQLVESGGGMVQAGDSLRLSCVQSTYTVNSDVMGWFRQAPGKEREFVGAIMWNDGITYLQDSVKGRFTIFRDNAKNTVYLQMNSLKLEDTAVYYCAASKGRYSEYEYWGQGTQVTVSSTSTTTPAPRPPTPAPTIASQPLSLRPEACRPAAGGAVHTRGLDFACDFWVLVVVGGVLACYSLLVTVAFIIFWVRSKRSRLLHSDYMNMTPRRPGPTRKHYQPYAPPRDFAAYRSKRGRKKLLYIFKQPFMRPVQTTQEEDGCSCRFPEEEEGGCELRVKFSRSADAPAYKQGQNQLYNELNLGRREEYDVLDKRRGRDPEMGGKPRRKNPQEGLYNELQKDKMAEAYSEIGMKGERRRGKGHDGLYQGLSTATKDTYDALHMQALPPR

SEQ ID NO: 159 - protein, 418 aa, synthetic construct
  source 1..418: note = BCMA 269A37965 CAR
MALPVTALLLPLALLLHAARPVNRTRRMHAVQLVESGGGLVQAGDSLRLSCTASGATLTNDHMAWFRQAPGKGREFVAAIDWSGRTTNYADPVEGRFTISRNNAKNTVYLEMNSLKLEDTAVYYCAVLRAWISYDNDYWGQGTQVTVSSTSTTTPAPRPPTPAPTIASQPLSLRPEACRPAAGGAVHTRGLDFACDFWVLVVVGGVLACYSLLVTVAFIIFWVRSKRSRLLHSDYMNMTPRRPGPTRKHYQPYAPPRDFAAYRSKRGRKKLLYIFKQPFMRPVQTTQEEDGCSCRFPEEEEGGCELRVKFSRSADAPAYKQGQNQLYNELNLGRREEYDVLDKRRGRDPEMGGKPRRKNPQEGLYNELQKDKMAEAYSEIGMKGERRRGKGHDGLYQGLSTATKDTYDALHMQALPPR

SEQ ID NO: 160 - protein, 418 aa, synthetic construct
  source 1..418: note = BCMA 269A37972 CAR
MALPVTALLLPLALLLHAARPVNRTRRMHQVQLVESGGGLVQAGGSLRLSCAASGGTLSKNTVAWFRQAPGKERGFVASITWDGRTTYYADSVKGRFTISRDNAKNTVYLQMNSLKPEDTAVYVCADLGKWPAGPADYWGQGTQVTVSSTSTTTPAPRPPTPAPTIASQPLSLRPEACRPAAGGAVHTRGLDFACDFWVLVVVGGVLACYSLLVTVAFIIFWVRSKRSRLLHSDYMNMTPRRPGPTRKHYQPYAPPRDFAAYRSKRGRKKLLYIFKQPFMRPVQTTQEEDGCSCRFPEEEEGGCELRVKFSRSADAPAYKQGQNQLYNELNLGRREEYDVLDKRRGRDPEMGGKPRRKNPQEGLYNELQKDKMAEAYSEIGMKGERRRGKGHDGLYQGLSTATKDTYDALHMQALPPR

SEQ ID NO: 161 - protein, 417 aa, synthetic construct
  source 1..417: note = BCMA 269A37353 CAR
MALPVTALLLPLALLLHAARPVNRTRRMHQVKLEESGGGLVQAGRSLRLSCAASEHTFSSHVMGWFRQAPGKERESVAVIGWRDISTSYADSVKGRFTISRDNAKKTLYLQMNSLKPEDTAVYYCAARRIDAADFDSWGQGTQVTVSSTSTTTPAPRPPTPAPTIASQPLSLRPEACRPAAGGAVHTRGLDFACDFWVLVVVGGVLACYSLLVTVAFIIFWVRSKRSRLLHSDYMNMTPRRPGPTRKHYQPYAPPRDFAAYRSKRGRKKLLYIFKQPFMRPVQTTQEEDGCSCRFPEEEEGGCELRVKFSRSADAPAYKQGQNQLYNELNLGRREEYDVLDKRRGRDPEMGGKPRRKNPQEGLYNELQKDKMAEAYSEIGMKGERRRGKGHDGLYQGLSTATKDTYDALHMQALPPR

SEQ ID NO: 162 - protein, 417 aa, synthetic construct
  source 1..417: note = BCMA 269A37948 CAR
MALPVTALLLPLALLLHAARPVNRTRRMHAVQLVESGGGLVQAGDSLRLTCTASGRAFSTYFMAWFRQAPGKEREFVAGIAWSGGSTAYADSVKGRFTISRDNAKNTVYLQMNSLKSEDTAVYYCASRGIEVEEFGAWGQGTQVTVSSTSTTTPAPRPPTPAPTIASQPLSLRPEACRPAAGGAVHTRGLDFACDFWVLVVVGGVLACYSLLVTVAFIIFWVRSKRSRLLHSDYMNMTPRRPGPTRKHYQPYAPPRDFAAYRSKRGRKKLLYIFKQPFMRPVQTTQEEDGCSCRFPEEEEGGCELRVKFSRSADAPAYKQGQNQLYNELNLGRREEYDVLDKRRGRDPEMGGKPRRKNPQEGLYNELQKDKMAEAYSEIGMKGERRRGKGHDGLYQGLSTATKDTYDALHMQALPPR

SEQ ID NO: 163 - protein, 411 aa, synthetic construct
  source 1..411: note = CD38 38A37333 CAR
MALPVTALLLPLALLLHAARPVNDVQLVESGGGLVQPGGSLRLSCVASGLTFSSYPMMWVRQAPGKGLEWVSRISDSGGYTNYDDSVKGRFTISRDNAKNTLYLQMNSLTPEDTAVYYCRILGLPTTGQGTQVTVSSTRRMHTSTTTPAPRPPTPAPTIASQPLSLRPEACRPAAGGAVHTRGLDFACDFWVLVVVGGVLACYSLLVTVAFIIFWVRSKRSRLLHSDYMNMTPRRPGPTRKHYQPYAPPRDFAAYRSKRGRKKLLYIFKQPFMRPVQTTQEEDGCSCRFPEEEEGGCELRVKFSRSADAPAYKQGQNQLYNELNLGRREEYDVLDKRRGRDPEMGGKPRRKNPQEGLYNELQKDKMAEAYSEIGMKGERRRGKGHDGLYQGLSTATKDTYDALHMQALPPR

SEQ ID NO: 164 - protein, 423 aa, synthetic construct
  source 1..423: note = CD38 38A37336 CAR
MALPVTALLLPLALLLHAARPVNEVQLVESGGGLVQPGGSLRLSCAASGFTFSSNWMYWVRQAPGKGLEWVATISTDGRGTYYKDSVKGRFTVSRDNAMSTLLLQMNNLKSEDTAVYYCAKEPRVLMAYLRNLGDFGSWGQGTQVTVSSTRRMHTSTTTPAPRPPTPAPTIASQPLSLRPEACRPAAGGAVHTRGLDFACDFWVLVVVGGVLACYSLLVTVAFIIFWVRSKRSRLLHSDYMNMTPRRPGPTRKHYQPYAPPRDFAAYRSKRGRKKLLYIFKQPFMRPVQTTQEEDGCSCRFPEEEEGGCELRVKFSRSADAPAYKQGQNQLYNELNLGRREEYDVLDKRRGRDPEMGGKPRRKNPQEGLYNELQKDKMAEAYSEIGMKGERRRGKGHDGLYQGLSTATKDTYDALHMQALPPR

SEQ ID NO: 165 - protein, 412 aa, synthetic construct
  source 1..412: note = CD38 38A37699 CAR
MALPVTALLLPLALLLHAARPVNQVQLVESGGGLVQAGGSLRLSCAASGRIFSINAMGWYRQAPGKQRELVAAISTAGSTNYGDSVKGRFTISRDNAKNTVYLQMNSLKPEDTAVYYCNLNFPPYVYWGQGTQVTVSSTRRMHTSTTTPAPRPPTPAPTIASQPLSLRPEACRPAAGGAVHTRGLDFACDFWVLVVVGGVLACYSLLVTVAFIIFWVRSKRSRLLHSDYMNMTPRRPGPTRKHYQPYAPPRDFAAYRSKRGRKKLLYIFKQPFMRPVQTTQEEDGCSCRFPEEEEGGCELRVKFSRSADAPAYKQGQNQLYNELNLGRREEYDVLDKRRGRDPEMGGKPRRKNPQEGLYNELQKDKMAEAYSEIGMKGERRRGKGHDGLYQGLSTATKDTYDALHMQALPPR

SEQ ID NO: 166 - protein, 416 aa, synthetic construct
  source 1..416: note = CD38 38A37331 CAR
MALPVTALLLPLALLLHAARPVNQVKLEESGGGLVQPGESLRLSCSASGSIFKVFRVFAMSWYRQGPGKQRELVASISSGETTTYADSVKGRFTISRDNAKNTAYLQMDSLKPEDTAVYYCNADHTFTGDFWGQGTQVTVSSTRRMHTSTTTPAPRPPTPAPTIASQPLSLRPEACRPAAGGAVHTRGLDFACDFWVLVVVGGVLACYSLLVTVAFIIFWVRSKRSRLLHSDYMNMTPRRPGPTRKHYQPYAPPRDFAAYRSKRGRKKLLYIFKQPFMRPVQTTQEEDGCSCRFPEEEEGGCELRVKFSRSADAPAYKQGQNQLYNELNLGRREEYDVLDKRRGRDPEMGGKPRRKNPQEGLYNELQKDKMAEAYSEIGMKGERRRGKGHDGLYQGLSTATKDTYDALHMQALPPR

SEQ ID NO: 167 - protein, 413 aa, synthetic construct
  source 1..413: note = CD38 38A37717 CAR
MALPVTALLLPLALLLHAARPVNEVQLVESGGGLVQAGGSLRLSCIATGKVFSIYDMGWYRQAPGKQRELVAEITSSGTTHYDDFVSGRFTISRDNAKNTVYLQMNTLKAEDTAVYYCRANHVFGGSYWGQGTQVTVSSTRRMHTSTTTPAPRPPTPAPTIASQPLSLRPEACRPAAGGAVHTRGLDFACDFWVLVVVGGVLACYSLLVTVAFIIFWVRSKRSRLLHSDYMNMTPRRPGPTRKHYQPYAPPRDFAAYRSKRGRKKLLYIFKQPFMRPVQTTQEEDGCSCRFPEEEEGGCELRVKFSRSADAPAYKQGQNQLYNELNLGRREEYDVLDKRRGRDPEMGGKPRRKNPQEGLYNELQKDKMAEAYSEIGMKGERRRGKGHDGLYQGLSTATKDTYDALHMQALPPR

SEQ ID NO: 168 - protein, 412 aa, synthetic construct
  source 1..412: note = CD38 38A37719 CAR
MALPVTALLLPLALLLHAARPVNQVKLEESGGGSVQTGGSLRLSCAASASIFTRLPMGWYRQAPGKQRELVVGIVPSGRINYADSVKGRFTISRDNAKNTVYLQMNSLRPEDTAVYYCRADTFPLPTWGQGTQVTVSSTRRMHTSTTTPAPRPPTPAPTIASQPLSLRPEACRPAAGGAVHTRGLDFACDFWVLVVVGGVLACYSLLVTVAFIIFWVRSKRSRLLHSDYMNMTPRRPGPTRKHYQPYAPPRDFAAYRSKRGRKKLLYIFKQPFMRPVQTTQEEDGCSCRFPEEEEGGCELRVKFSRSADAPAYKQGQNQLYNELNLGRREEYDVLDKRRGRDPEMGGKPRRKNPQEGLYNELQKDKMAEAYSEIGMKGERRRGKGHDGLYQGLSTATKDTYDALHMQALPPR

SEQ ID NO: 169 - protein, 423 aa, synthetic construct
  source 1..423: note = CD38 38A37330 CAR
MALPVTALLLPLALLLHAARPVNQVQLVESGGGLVQAGDSLRLSCAASGRAYATMAWFRQAPGKEREFVAHLRVSGDTTYYTDSVKGRFTISRDNAKNTAYLQMNMLKPEDTAVYYCAAGPYGILAAARVSNPGNYDYWGQGTQVTVSSTRRMHTSTTTPAPRPPTPAPTIASQPLSLRPEACRPAAGGAVHTRGLDFACDFWVLVVVGGVLACYSLLVTVAFIIFWVRSKRSRLLHSDYMNMTPRRPGPTRKHYQPYAPPRDFAAYRSKRGRKKLLYIFKQPFMRPVQTTQEEDGCSCRFPEEEEGGCELRVKFSRSADAPAYKQGQNQLYNELNLGRREEYDVLDKRRGRDPEMGGKPRRKNPQEGLYNELQKDKMAEAYSEIGMKGERRRGKGHDGLYQGLSTATKDTYDALHMQALPPR

SEQ ID NO: 170 - protein, 420 aa, synthetic construct
  source 1..420: note = CD38 38A37334 CAR
MALPVTALLLPLALLLHAARPVNEVQLVESGGGLVQAGGSLRLSCAASGLTFSSYIMGWFRQAPGEERELVAEISSGGMTSYADSVKGRFTISRDNAKKTGYLQMNSLKPEDTAVYYCAAPERGSIWYSRYEYKYWGQGTQVTVSSTRRMHTSTTTPAPRPPTPAPTIASQPLSLRPEACRPAAGGAVHTRGLDFACDFWVLVVVGGVLACYSLLVTVAFIIFWVRSKRSRLLHSDYMNMTPRRPGPTRKHYQPYAPPRDFAAYRSKRGRKKLLYIFKQPFMRPVQTTQEEDGCSCRFPEEEEGGCELRVKFSRSADAPAYKQGQNQLYNELNLGRREEYDVLDKRRGRDPEMGGKPRRKNPQEGLYNELQKDKMAEAYSEIGMKGERRRGKGHDGLYQGLSTATKDTYDALHMQALPPR

SEQ ID NO: 171 - protein, 417 aa, synthetic construct
  source 1..417: note = CD38 38A37730 CAR
MALPVTALLLPLALLLHAARPVNAVQLVDSGGGLAQTGGSLRLSCAASQGIFTINAMGWYRQVPGKQRELVAEVSSGGRTDYADSVKGRFTISRDNAKNTVYLQMNSLKPEDTGVYYCRVSGWHVFVGDRIVWGQGTLVTVSSTRRMHTSTTTPAPRPPTPAPTIASQPLSLRPEACRPAAGGAVHTRGLDFACDFWVLVVVGGVLACYSLLVTVAFIIFWVRSKRSRLLHSDYMNMTPRRPGPTRKHYQPYAPPRDFAAYRSKRGRKKLLYIFKQPFMRPVQTTQEEDGCSCRFPEEEEGGCELRVKFSRSADAPAYKQGQNQLYNELNLGRREEYDVLDKRRGRDPEMGGKPRRKNPQEGLYNELQKDKMAEAYSEIGMKGERRRGKGHDGLYQGLSTATKDTYDALHMQALPPR

SEQ ID NO: 172 - protein, 420 aa, synthetic construct
  source 1..420: note = CD38 38A37340 CAR
MALPVTALLLPLALLLHAARPVNDVQLVESGGGLVQAGDSLRLSCAASGRTFSSYAMAWFRQAPGKEREIVSSISTSGGITDYADSVKGRFTISKDSAKMNTVYLQMNSLEPEDTAVYYCAARTWYLRTSLQYDYWGQGTQVTVSSTRRMHTSTTTPAPRPPTPAPTIASQPLSLRPEACRPAAGGAVHTRGLDFACDFWVLVVVGGVLACYSLLVTVAFIIFWVRSKRSRLLHSDYMNMTPRRPGPTRKHYQPYAPPRDFAAYRSKRGRKKLLYIFKQPFMRPVQTTQEEDGCSCRFPEEEEGGCELRVKFSRSADAPAYKQGQNQLYNELNLGRREEYDVLDKRRGRDPEMGGKPRRKNPQEGLYNELQKDKMAEAYSEIGMKGERRRGKGHDGLYQGLSTATKDTYDALHMQALPPR

SEQ ID NO: 173 - protein, 418 aa, synthetic construct
  source 1..418: note = CD38 38A37731 CAR
MALPVTALLLPLALLLHAARPVNQVKLEESGGGLVQAGGSLRLSCVASGTIVSISTMGWYRQAPGKQRELVATITRRGRTNYTDSVKGRFTISRDNAKNTVYLQMNSLKPEDTAVYYCNAEVQLDIWASAYDYWGQGTQVTVASTRRMHTSTTTPAPRPPTPAPTIASQPLSLRPEACRPAAGGAVHTRGLDFACDFWVLVVVGGVLACYSLLVTVAFIIFWVRSKRSRLLHSDYMNMTPRRPGPTRKHYQPYAPPRDFAAYRSKRGRKKLLYIFKQPFMRPVQTTQEEDGCSCRFPEEEEGGCELRVKFSRSADAPAYKQGQNQLYNELNLGRREEYDVLDKRRGRDPEMGGKPRRKNPQEGLYNELQKDKMAEAYSEIGMKGERRRGKGHDGLYQGLSTATKDTYDALHMQALPPR

SEQ ID NO: 174 - protein, 412 aa, synthetic construct
  source 1..412: note = CD38 38A37326 CAR
MALPVTALLLPLALLLHAARPVNEVQLVESGGGLVQAGGSLRLSCAASGRTYAMGWYRQAPGKQRDLVATISGAGNTKYADSVKGRFTISRDNAKNTMYLQMNSLKPEDTAVYYCAAGKWFPAANEYWGQGTQVTVSSTRRMHTSTTTPAPRPPTPAPTIASQPLSLRPEACRPAAGGAVHTRGLDFACDFWVLVVVGGVLACYSLLVTVAFIIFWVRSKRSRLLHSDYMNMTPRRPGPTRKHYQPYAPPRDFAAYRSKRGRKKLLYIFKQPFMRPVQTTQEEDGCSCRFPEEEEGGCELRVKFSRSADAPAYKQGQNQLYNELNLGRREEYDVLDKRRGRDPEMGGKPRRKNPQEGLYNELQKDKMAEAYSEIGMKGERRRGKGHDGLYQGLSTATKDTYDALHMQALPPR

SEQ ID NO: 175 - DNA, 1263 bp, synthetic construct
  source 1..1263: mol_type = other DNA; note = BCMA 269A37346 CAR
atggccttaccagtgaccgccttgctcctgccgctggccttgctgctccacgccgccaggccggttaaccgcacgcgtcgcatgcatcaggtgcagctggtggagtctgggggaggcttggtgcagcctgggggttctctgaggctctcctgtgaagcctctggattcactttggattattatgccataggctggttccgccaggccccagggaaggagcgcgagggggtcatatgtattagtagaagtgatggtagcacatactatgcagactccgtgaagggccgattcaccatctccagagacaacgccaagaaaacggtgtatctgcaaatgatcagcctgaaacctgaggacacggccgcttattactgtgcagcaggggccgattgttcggggtacctacgagattatgagttccgggggcaggggacccaggtcaccgtctcctcaactagtaccacgacgccagcgccgcgaccaccaacaccggcgcccaccatcgcgtcgcagcccctgtccctgcgcccagaggcgtgccggccagcggcggggggcgcagtgcacacgagggggctggacttcgcctgtgatttttgggtgctggtggtggttggtggagtcctggcttgctatagcttgctagtaacagtggcctttattattttctgggtgaggagtaagaggagcaggctcctgcacagtgactacatgaacatgactccccgccgccccgggcccacccgcaagcattaccagccctatgccccaccacgcgacttcgcagcctatcgctccaaacggggcagaaagaaactcctgtatatattcaaacaaccatttatgagaccagtacaaactactcaagaggaagatggctgtagctgccgatttccagaagaagaagaaggaggatgtgaactgagagtgaagttcagcaggagcgcagacgcccccgcgtacaagcagggccagaaccagctctataacgagctcaatctaggacgaagagaggagtacgatgttttggacaagagacgtggccgggaccctgagatggggggaaagccgagaaggaagaaccctcaggaaggcctgtacaatgaactgcagaaagataagatggcggaggcctacagtgagattgggatgaaaggcgagcgccggaggggcaaggggcacgatggcctttaccagggtctcagtacagccaccaaggacacctacgacgcccttcacatgcaggccctgccccctcgctga

SEQ ID NO: 176 - DNA, 1281 bp, synthetic construct
  source 1..1281: mol_type = other DNA; note = BCMA 269A37348 CAR
atggccttaccagtgaccgccttgctcctgccgctggccttgctgctccacgccgccaggccggttaaccgcacgcgtcgcatgcatcaggtaaagctggaggagtctgggggacgattggtgcagccaaggggctctctgagactctcctgtgcaggctctggacgcactttcagtacctatggtatggcctggttccgccaggctccagggaaggagcgtgagttcgtagcgtctaaagcatcgatgaattacagcggtagaacatactatgcagactccgtgaagggccgattcaccatcgccagagacaacgccaagaacatggtgtttctgcaaatgaacaacctgaagcctgaggacacggccgtttattactgtgcagcgggcactggatgctcaacatatgggtgttttgacgcccagataatagactactggggcaaagggaccctggtcaccgtctcctcaactagtaccacgacgccagcgccgcgaccaccaacaccggcgcccaccatcgcgtcgcagcccctgtccctgcgcccagaggcgtgccggccagcggcggggggcgcagtgcacacgagggggctggacttcgcctgtgatttttgggtgctggtggtggttggtggagtcctggcttgctatagcttgctagtaacagtggcctttattattttctgggtgaggagtaagaggagcaggctcctgcacagtgactacatgaacatgactccccgccgccccgggcccacccgcaagcattaccagccctatgccccaccacgcgacttcgcagcctatcgctccaaacggggcagaaagaaactcctgtatatattcaaacaaccatttatgagaccagtacaaactactcaagaggaagatggctgtagctgccgatttccagaagaagaagaaggaggatgtgaactgagagtgaagttcagcaggagcgcagacgcccccgcgtacaagcagggccagaaccagctctataacgagctcaatctaggacgaagagaggagtacgatgttttggacaagagacgtggccgggaccctgagatggggggaaagccgagaaggaagaaccctcaggaaggcctgtacaatgaactgcagaaagataagatggcggaggcctacagtgagattgggatgaaaggcgagcgccggaggggcaaggggcacgatggcctttaccagggtctcagtacagccaccaaggacacctacgacgcccttcacatgcaggccctgccccctcgctga

SEQ ID NO: 177 - DNA, 1251 bp, synthetic construct
  source 1..1251: mol_type = other DNA; note = BCMA 269A37917 CAR
atggccttaccagtgaccgccttgctcctgccgctggccttgctgctccacgccgccaggccggttaaccgcacgcgtcgcatgcatgaggtgcagctggtggagtctgggggaggcttggtgcaggctggggggtctctgagactctcctgtgcagcctctggacgcaccttcaccatggggtggttccgtcaggctccagggaaggagcgtgagtttgtagcagctattagtttgagtcctactttagcatattatgcagagtccgtgaagggccgattcaccatcagccgagacaacgccaagaacacggtggttttgcaaatgaacagcctgaaacctgaggacacggccctttattactgtgcagcagaccggaaatcagtaatgtctattcggcccgactactggggccaggggacccaggtcaccgtctcctcaactagtaccacgacgccagcgccgcgaccaccaacaccggcgcccaccatcgcgtcgcagcccctgtccctgcgcccagaggcgtgccggccagcggcggggggcgcagtgcacacgagggggctggacttcgcctgtgatttttgggtgctggtggtggttggtggagtcctggcttgctatagcttgctagtaacagtggcctttattattttctgggtgaggagtaagaggagcaggctcctgcacagtgactacatgaacatgactccccgccgccccgggcccacccgcaagcattaccagccctatgccccaccacgcgacttcgcagcctatcgctccaaacggggcagaaagaaactcctgtatatattcaaacaaccatttatgagaccagtacaaactactcaagaggaagatggctgtagctgccgatttccagaagaagaagaaggaggatgtgaactgagagtgaagttcagcaggagcgcagacgcccccgcgtacaagcagggccagaaccagctctataacgagctcaatctaggacgaagagaggagtacgatgttttggacaagagacgtggccgggaccctgagatggggggaaagccgagaaggaagaaccctcaggaaggcctgtacaatgaactgcagaaagataagatggcggaggcctacagtgagattgggatgaaaggcgagcgccggaggggcaaggggcacgatggcctttaccagggtctcagtacagccaccaaggacacctacgacgcccttcacatgcaggccctgccccctcgctga

SEQ ID NO: 178 - DNA, 1257 bp, synthetic construct
  source 1..1257: mol_type = other DNA; note = BCMA 269A37355 CAR
atggccttaccagtgaccgccttgctcctgccgctggccttgctgctccacgccgccaggccggttaaccgcacgcgtcgcatgcatgccgtgcagctggtggattctgggggaggcttggtgcagcctggggggtctctgagactctcctgtgtagcctctggaggtatcttcgtcatcaatgccatgggctggtaccgccaggctccaggaaagcagcgcgagttggtcgcatctattcgtggactaggcagaacaaactatgacgactccgtgaagggccgattcaccatctccagagacaacgccaacaacacggtgtatctgcagatgaacagcctggaacctgaggacacggccgtctactactgtacagtctacgttacactacttggtggggttaatagggactactggggccaggggacccaggtcaccgtctcctcaactagtaccacgacgccagcgccgcgaccaccaacaccggcgcccaccatcgcgtcgcagcccctgtccctgcgcccagaggcgtgccggccagcggcggggggcgcagtgcacacgagggggctggacttcgcctgtgatttttgggtgctggtggtggttggtggagtcctggcttgctatagcttgctagtaacagtggcctttattattttctgggtgaggagtaagaggagcaggctcctgcacagtgactacatgaacatgactccccgccgccccgggcccacccgcaagcattaccagccctatgccccaccacgcgacttcgcagcctatcgctccaaacggggcagaaagaaactcctgtatatattcaaacaaccatttatgagaccagtacaaactactcaagaggaagatggctgtagctgccgatttccagaagaagaagaaggaggatgtgaactgagagtgaagttcagcaggagcgcagacgcccccgcgtacaagcagggccagaaccagctctataacgagctcaatctaggacgaagagaggagtacgatgttttggacaagagacgtggccgggaccctgagatggggggaaagccgagaaggaagaaccctcaggaaggcctgtacaatgaactgcagaaagataagatggcggaggcctacagtgagattgggatgaaaggcgagcgccggaggggcaaggggcacgatggcctttaccagggtctcagtacagccaccaaggacacctacgacgcccttcacatgcaggccctgccccctcgctga

SEQ ID NO: 179 - DNA, 1254 bp, synthetic construct
  source 1..1254: mol_type = other DNA; note = BCMA 269A37915 CAR
atggccttaccagtgaccgccttgctcctgccgctggccttgctgctccacgccgccaggccggttaaccgcacgcgtcgcatgcatgaggtgcagctggtggagtctgggggaggattggtgcaggctgggggctctctgagactctcctgtgcagcctctggacggaccttcagtagcattgtcatgggctggttccgccaggctccagggaaggagcgtgagtttgtaggagcgattatgtggaatgatggtattacatacttgcaagactccgtgaagggccgatttaccatcttcagagacaatgccaagaacacggtgtatctgcaaatgaacagcctgaaacttgaggatacggccgtttattactgtgcagcatccaagggtagatactcggaatatgagtactggggccaggggacccaggtcaccgtctcctcaactagtaccacgacgccagcgccgcgaccaccaacaccggcgcccaccatcgcgtcgcagcccctgtccctgcgcccagaggcgtgccggccagcggcggggggcgcagtgcacacgagggggctggacttcgcctgtgatttttgggtgctggtggtggttggtggagtcctggcttgctatagcttgctagtaacagtggcctttattattttctgggtgaggagtaagaggagcaggctcctgcacagtgactacatgaacatgactccccgccgccccgggcccacccgcaagcattaccagccctatgccccaccacgcgacttcgcagcctatcgctccaaacggggcagaaagaaactcctgtatatattcaaacaaccatttatgagaccagtacaaactactcaagaggaagatggctgtagctgccgatttccagaagaagaagaaggaggatgtgaactgagagtgaagttcagcaggagcgcagacgcccccgcgtacaagcagggccagaaccagctctataacgagctcaatctaggacgaagagaggagtacgatgttttggacaagagacgtggccgggaccctgagatggggggaaagccgagaaggaagaaccctcaggaaggcctgtacaatgaactgcagaaagataagatggcggaggcctacagtgagattgggatgaaaggcgagcgccggaggggcaaggggcacgatggcctttaccagggtctcagtacagccaccaaggacacctacgacgcccttcacatgcaggccctgccccctcgctga

SEQ ID NO: 180 - DNA, 1281 bp, synthetic construct
  source 1..1281: mol_type = other DNA; note = BCMA 269A37936 CAR
atggccttaccagtgaccgccttgctcctgccgctggccttgctgctccacgccgccaggccggttaaccgcacgcgtcgcatgcatgaggtgcagctggtggagtctgggggaggcgtggtgcaggctggggggtctctgacagtctcctgtacagcctctggattcactttcgaccgtgctgtcatagtctggttccgccaggcccccgggaagggccgtgagggggtctcatttattaaacctagtgatggcaccatatactacattgactccctgaagggccgattcacgatctccagtgacatcgccaagaatacggtatatctgcaaatgaaaagtctggaatcggaggactcggccgtttattactgtgcggcctcgcctgaggactggtacacggattggatcgactggagtatatatcggtggcagcactggggccaggggacccaggtcactgtctcctcaactagtaccacgacgccagcgccgcgaccaccaacaccggcgcccaccatcgcgtcgcagcccctgtccctgcgcccagaggcgtgccggccagcggcggggggcgcagtgcacacgagggggctggacttcgcctgtgatttttgggtgctggtggtggttggtggagtcctggcttgctatagcttgctagtaacagtggcctttattattttctgggtgaggagtaagaggagcaggctcctgcacagtgactacatgaacatgactccccgccgccccgggcccacccgcaagcattaccagccctatgccccaccacgcgacttcgcagcctatcgctccaaacggggcagaaagaaactcctgtatatattcaaacaaccatttatgagaccagtacaaactactcaagaggaagatggctgtagctgccgatttccagaagaagaagaaggaggatgtgaactgagagtgaagttcagcaggagcgcagacgcccccgcgtacaagcagggccagaaccagctctataacgagctcaatctaggacgaagagaggagtacgatgttttggacaagagacgtggccgggaccctgagatggggggaaagccgagaaggaagaaccctcaggaaggcctgtacaatgaactgcagaaagataagatggcggaggcctacagtgagattgggatgaaaggcgagcgccggaggggcaaggggcacgatggcctttaccagggtctcagtacagccaccaaggacacctacgacgcccttcacatgcaggccctgccccctcgctga

SEQ ID NO: 181 - DNA, 1254 bp, synthetic construct
  source 1..1254: mol_type = other DNA; note = BCMA 269A37953 CAR
atggccttaccagtgaccgccttgctcctgccgctggccttgctgctccacgccgccaggccggttaaccgcacgcgtcgcatgcatgaggtgcagctggtggagtctgggggaggaatggtgcaggctggggactctctgagactatcctgtgtgcagtctacttacaccgtcaatagcgatgtcatgggctggttccgccaggctccagggaaggagcgtgagtttgtaggagcgattatgtggaatgatggtattacatacttgcaagactccgtgaagggccgatttaccatcttcagagacaacgccaagaacacggtgtatctgcaaatgaacagcctgaaacttgaggatacggccgtttattactgtgcagcatccaagggtagatactcggaatatgagtactggggccaggggacccaggtcaccgtctcctcaactagtaccacgacgccagcgccgcgaccaccaacaccggcgcccaccatcgcgtcgcagcccctgtccctgcgcccagaggcgtgccggccagcggcggggggcgcagtgcacacgagggggctggacttcgcctgtgatttttgggtgctggtggtggttggtggagtcctggcttgctatagcttgctagtaacagtggcctttattattttctgggtgaggagtaagaggagcaggctcctgcacagtgactacatgaacatgactccccgccgccccgggcccacccgcaagcattaccagccctatgccccaccacgcgacttcgcagcctatcgctccaaacggggcagaaagaaactcctgtatatattcaaacaaccatttatgagaccagtacaaactactcaagaggaagatggctgtagctgccgatttccagaagaagaagaaggaggatgtgaactgagagtgaagttcagcaggagcgcagacgcccccgcgtacaagcagggccagaaccagctctataacgagctcaatctaggacgaagagaggagtacgatgttttggacaagagacgtggccgggaccctgagatggggggaaagccgagaaggaagaaccctcaggaaggcctgtacaatgaactgcagaaagataagatggcggaggcctacagtgagattgggatgaaaggcgagcgccggaggggcaaggggcacgatggcctttaccagggtctcagtacagccaccaaggacacctacgacgcccttcacatgcaggccctgccccctcgctga

SEQ ID NO: 182 - DNA, 1257 bp, synthetic construct
  source 1..1257: mol_type = other DNA; note = BCMA 269A37965 CAR
atggccttaccagtgaccgccttgctcctgccgctggccttgctgctccacgccgccaggccggttaaccgcacgcgtcgcatgcatgcggtgcagctggtggagtctgggggaggattggtgcaggctggggactctctgagactctcctgtacagcctctggtgcaaccttgactaacgatcacatggcatggttccgccaggctccagggaaggggcgtgaatttgtagcagctattgactggagtggtcgtaccacaaattacgcagaccccgtagagggccgattcaccatctccagaaacaacgccaagaacacggtgtatctggaaatgaacagcctgaaacttgaggacacggccgtttattactgtgcggtcctccgcgcttggatctcatatgacaatgactactggggccaggggacccaggtcaccgtctcctcaactagtaccacgacgccagcgccgcgaccaccaacaccggcgcccaccatcgcgtcgcagcccctgtccctgcgcccagaggcgtgccggccagcggcggggggcgcagtgcacacgagggggctggacttcgcctgtgatttttgggtgctggtggtggttggtggagtcctggcttgctatagcttgctagtaacagtggcctttattattttctgggtgaggagtaagaggagcaggctcctgcacagtgactacatgaacatgactccccgccgccccgggcccacccgcaagcattaccagccctatgccccaccacgcgacttcgcagcctatcgctccaaacggggcagaaagaaactcctgtatatattcaaacaaccatttatgagaccagtacaaactactcaagaggaagatggctgtagctgccgatttccagaagaagaagaaggaggatgtgaactgagagtgaagttcagcaggagcgcagacgcccccgcgtacaagcagggccagaaccagctctataacgagctcaatctaggacgaagagaggagtacgatgttttggacaagagacgtggccgggaccctgagatggggggaaagccgagaaggaagaaccctcaggaaggcctgtacaatgaactgcagaaagataagatggcggaggcctacagtgagattgggatgaaaggcgagcgccggaggggcaaggggcacgatggcctttaccagggtctcagtacagccaccaaggacacctacgacgcccttcacatgcaggccctgccccctcgctga

SEQ ID NO: 183 - DNA, 1257 bp, synthetic construct
  source 1..1257: mol_type = other DNA; note = BCMA 269A37972 CAR
atggccttaccagtgaccgccttgctcctgccgctggccttgctgctccacgccgccaggccggttaaccgcacgcgtcgcatgcatcaggtgcagctggtggagtctgggggaggattggtgcaggctgggggctctctgagactctcctgtgcagcctctggaggcaccttaagtaaaaataccgtggcttggttccgccaggctccagggaaggagcgtgggtttgtagcgtctattacctgggatggtcgtacgacatactatgcagactccgtgaagggccgattcaccatctccagagacaacgccaagaacacagtgtatctgcaaatgaacagcctgaaacctgaggatacggccgtttatgtctgtgcagacttagggaaatggcctgcgggcccggcggactactggggccaggggacccaggtcaccgtctcctcaactagtaccacgacgccagcgccgcgaccaccaacaccggcgcccaccatcgcgtcgcagcccctgtccctgcgcccagaggcgtgccggccagcggcggggggcgcagtgcacacgagggggctggacttcgcctgtgatttttgggtgctggtggtggttggtggagtcctggcttgctatagcttgctagtaacagtggcctttattattttctgggtgaggagtaagaggagcaggctcctgcacagtgactacatgaacatgactccccgccgccccgggcccacccgcaagcattaccagccctatgccccaccacgcgacttcgcagcctatcgctccaaacggggcagaaagaaactcctgtatatattcaaacaaccatttatgagaccagtacaaactactcaagaggaagatggctgtagctgccgatttccagaagaagaagaaggaggatgtgaactgagagtgaagttcagcaggagcgcagacgcccccgcgtacaagcagggccagaaccagctctataacgagctcaatctaggacgaagagaggagtacgatgttttggacaagagacgtggccgggaccctgagatggggggaaagccgagaaggaagaaccctcaggaaggcctgtacaatgaactgcagaaagataagatggcggaggcctacagtgagattgggatgaaaggcgagcgccggaggggcaaggggcacgatggcctttaccagggtctcagtacagccaccaaggacacctacgacgcccttcacatgcaggccctgccccctcgctga

SEQ ID NO: 184 - DNA, 1254 bp, synthetic construct
  source 1..1254: mol_type = other DNA; note = BCMA 269A37353 CAR
atggccttaccagtgaccgccttgctcctgccgctggccttgctgctccacgccgccaggccggttaaccgcacgcgtcgcatgcatcaggtaaagctggaggagtctgggggaggcttggtgcaggctgggcggtctctgagactctcctgtgcagcctctgaacacaccttcagtagccatgtcatgggctggttccgccaggctccagggaaggagcgtgagtctgttgcagttattggctggagagatattagcacaagctatgcagactccgtgaagggccgattcaccatctccagagacaacgccaagaagacgctgtatctgcaaatgaatagcctgaaacctgaggacacggccgtttactactgtgcagcacgtcggatcgacgcagctgactttgattcctgggggcaggggacccaggtcaccgtctcctcgactagtaccacgacgccagcgccgcgaccaccaacaccggcgcccaccatcgcgtcgcagcccctgtccctgcgcccagaggcgtgccggccagcggcggggggcgcagtgcacacgagggggctggacttcgcctgtgatttttgggtgctggtggtggttggtggagtcctggcttgctatagcttgctagtaacagtggcctttattattttctgggtgaggagtaagaggagcaggctcctgcacagtgactacatgaacatgactccccgccgccccgggcccacccgcaagcattaccagccctatgccccaccacgcgacttcgcagcctatcgctccaaacggggcagaaagaaactcctgtatatattcaaacaaccatttatgagaccagtacaaactactcaagaggaagatggctgtagctgccgatttccagaagaagaagaaggaggatgtgaactgagagtgaagttcagcaggagcgcagacgcccccgcgtacaagcagggccagaaccagctctataacgagctcaatctaggacgaagagaggagtacgatgttttggacaagagacgtggccgggaccctgagatggggggaaagccgagaaggaagaaccctcaggaaggcctgtacaatgaactgcagaaagataagatggcggaggcctacagtgagattgggatgaaaggcgagcgccggaggggcaaggggcacgatggcctttaccagggtctcagtacagccaccaaggacacctacgacgcccttcacatgcaggccctgccccctcgctga

SEQ ID NO: 185 - DNA, 1254 bp, synthetic construct
  source 1..1254: mol_type = other DNA; note = BCMA 269A37948 CAR
atggccttaccagtgaccgccttgctcctgccgctggccttgctgctccacgccgccaggccggttaaccgcacgcgtcgcatgcatgcggtgcagctggtggagtctgggggaggattggtgcaggctggggactctctgagactcacctgtacagcctctggacgcgccttcagtacctatttcatggcctggttccgccaggctccagggaaggagcgtgagtttgtagcaggaattgcatggagtggtggtagcacggcgtatgcagactccgtgaagggccgattcaccatctccagagacaacgccaagaacacggtgtatctgcaaatgaacagcctgaaatctgaggacacggccgtttattactgtgccagcagggggattgaggtcgaagagtttggtgcctggggccaggggacccaggtcaccgtctcgtcgactagtaccacgacgccagcgccgcgaccaccaacaccggcgcccaccatcgcgtcgcagcccctgtccctgcgcccagaggcgtgccggccagcggcggggggcgcagtgcacacgagggggctggacttcgcctgtgatttttgggtgctggtggtggttggtggagtcctggcttgctatagcttgctagtaacagtggcctttattattttctgggtgaggagtaagaggagcaggctcctgcacagtgactacatgaacatgactccccgccgccccgggcccacccgcaagcattaccagccctatgccccaccacgcgacttcgcagcctatcgctccaaacggggcagaaagaaactcctgtatatattcaaacaaccatttatgagaccagtacaaactactcaagaggaagatggctgtagctgccgatttccagaagaagaagaaggaggatgtgaactgagagtgaagttcagcaggagcgcagacgcccccgcgtacaagcagggccagaaccagctctataacgagctcaatctaggacgaagagaggagtacgatgttttggacaagagacgtggccgggaccctgagatggggggaaagccgagaaggaagaaccctcaggaaggcctgtacaatgaactgcagaaagataagatggcggaggcctacagtgagattgggatgaaaggcgagcgccggaggggcaaggggcacgatggcctttaccagggtctcagtacagccaccaaggacacctacgacgcccttcacatgcaggccctgccccctcgctga

SEQ ID NO: 186 - DNA, 1236 bp, synthetic construct
  source 1..1236: mol_type = other DNA; note = CD38 38A37333 CAR
atggccttaccagtgaccgccttgctcctgccgctggccttgctgctccacgccgccaggccggttaacgatgtgcagctggtggagtctgggggaggcttggtgcagcctggggggtctctgagactctcctgtgtagcctctggattgaccttcagtagctaccccatgatgtgggtccgccaggctccaggaaaggggctcgagtgggtctcacgtattagcgatagtggtggttacacaaactatgacgactccgtgaagggccgattcaccatctccagagacaacgccaagaacacgctgtatctgcaaatgaacagcctgacacctgaggacacggccgtgtattactgtagaatcctggggttgcccaccacgggccaggggacccaggtcaccgtctcctcaacgcgtcgcatgcatactagtaccacgacgccagcgccgcgaccaccaacaccggcgcccaccatcgcgtcgcagcccctgtccctgcgcccagaggcgtgccggccagcggcggggggcgcagtgcacacgagggggctggacttcgcctgtgatttttgggtgctggtggtggttggtggagtcctggcttgctatagcttgctagtaacagtggcctttattattttctgggtgaggagtaagaggagcaggctcctgcacagtgactacatgaacatgactccccgccgccccgggcccacccgcaagcattaccagccctatgccccaccacgcgacttcgcagcctatcgctccaaacggggcagaaagaaactcctgtatatattcaaacaaccatttatgagaccagtacaaactactcaagaggaagatggctgtagctgccgatttccagaagaagaagaaggaggatgtgaactgagagtgaagttcagcaggagcgcagacgcccccgcgtacaagcagggccagaaccagctctataacgagctcaatctaggacgaagagaggagtacgatgttttggacaagagacgtggccgggaccctgagatggggggaaagccgagaaggaagaaccctcaggaaggcctgtacaatgaactgcagaaagataagatggcggaggcctacagtgagattgggatgaaaggcgagcgccggaggggcaaggggcacgatggcctttaccagggtctcagtacagccaccaaggacacctacgacgcccttcacatgcaggccctgccccctcgctga

SEQ ID NO: 187 - DNA, 1272 bp, synthetic construct
  source 1..1272: mol_type = other DNA; note = CD38 38A37336 CAR
atggccttaccagtgaccgccttgctcctgccgctggccttgctgctccacgccgccaggccggttaacgaggtgcagctggtggagtctgggggaggcctggtgcagcctggggggtctctgagactctcctgtgcagcctctggattcaccttcagtagcaactggatgtattgggtccgtcaggctccagggaaggggctcgagtgggtcgcaactattagtactgatggtcgtggaacatactataaagactctgtgaagggccgattcaccgtctccagagacaacgccatgagtacgctgcttctgcaaatgaacaatctgaaatctgaagatacggccgtgtattattgtgcaaaagagccgagggtgttgatggcttacctgcggaacctgggtgactttggttcctggggccaggggacccaggtcaccgtctcctcgacgcgtcgcatgcatactagtaccacgacgccagcgccgcgaccaccaacaccggcgcccaccatcgcgtcgcagcccctgtccctgcgcccagaggcgtgccggccagcggcggggggcgcagtgcacacgagggggctggacttcgcctgtgatttttgggtgctggtggtggttggtggagtcctggcttgctatagcttgctagtaacagtggcctttattattttctgggtgaggagtaagaggagcaggctcctgcacagtgactacatgaacatgactccccgccgccccgggcccacccgcaagcattaccagccctatgccccaccacgcgacttcgcagcctatcgctccaaacggggcagaaagaaactcctgtatatattcaaacaaccatttatgagaccagtacaaactactcaagaggaagatggctgtagctgccgatttccagaagaagaagaaggaggatgtgaactgagagtgaagttcagcaggagcgcagacgcccccgcgtacaagcagggccagaaccagctctataacgagctcaatctaggacgaagagaggagtacgatgttttggacaagagacgtggccgggaccctgagatggggggaaagccgagaaggaagaaccctcaggaaggcctgtacaatgaactgcagaaagataagatggcggaggcctacagtgagattgggatgaaaggcgagcgccggaggggcaaggggcacgatggcctttaccagggtctcagtacagccaccaaggacacctacgacgcccttcacatgcaggccctgccccctcgctga

SEQ ID NO: 188 - DNA, 1239 bp, synthetic construct
  source 1..1239: mol_type = other DNA; note = CD38 38A37669 CAR
atggccttaccagtgaccgccttgctcctgccgctggccttgctgctccacgccgccaggccggttaaccaggtgcagctggtggagtctgggggaggcttggtgcaggctggggggtctctgagactctcctgtgcagcctctggaaggatcttcagtatcaatgccatgggctggtaccgccaggctccagggaagcagcgcgagttggtcgccgctattagtacggctggtagcacaaactatggagactccgtgaagggccgattcaccatctccagagacaacgccaagaacacggtgtatctgcaaatgaacagcctgaaacctgaggacacagctgtttattactgtaatttaaattttcccccgtatgtgtactggggccaggggacccaggtcaccgtctcctcaacgcgtcgcatgcatactagtaccacgacgccagcgccgcgaccaccaacaccggcgcccaccatcgcgtcgcagcccctgtccctgcgcccagaggcgtgccggccagcggcggggggcgcagtgcacacgagggggctggacttcgcctgtgatttttgggtgctggtggtggttggtggagtcctggcttgctatagcttgctagtaacagtggcctttattattttctgggtgaggagtaagaggagcaggctcctgcacagtgactacatgaacatgactccccgccgccccgggcccacccgcaagcattaccagccctatgccccaccacgcgacttcgcagcctatcgctccaaacggggcagaaagaaactcctgtatatattcaaacaaccatttatgagaccagtacaaactactcaagaggaagatggctgtagctgccgatttccagaagaagaagaaggaggatgtgaactgagagtgaagttcagcaggagcgcagacgcccccgcgtacaagcagggccagaaccagctctataacgagctcaatctaggacgaagagaggagtacgatgttttggacaagagacgtggccgggaccctgagatggggggaaagccgagaaggaagaaccctcaggaaggcctgtacaatgaactgcagaaagataagatggcggaggcctacagtgagattgggatgaaaggcgagcgccggaggggcaaggggcacgatggcctttaccagggtctcagtacagccaccaaggacacctacgacgcccttcacatgcaggccctgccccctcgctga

SEQ ID NO: 189 - DNA, 1251 bp, synthetic construct
  source 1..1251: mol_type = other DNA; note = CD38 38A37331 CAR
atggccttaccagtgaccgccttgctcctgccgctggccttgctgctccacgccgccaggccggttaaccaggtaaagctggaggagtctgggggaggtctggtgcagcctggggagtctctgagactctcctgttcagcctctggaagcatcttcaaagttttcagagtctttgccatgagctggtaccgccagggtcccgggaaacagcgcgagttggtcgcatccattagtagtggcgagaccacaacctatgcagactccgtgaagggccgattcaccatctccagagacaacgccaagaatacggcgtatctgcaaatggacagcctgaaacctgaggacacggccgtctattactgtaatgcggatcacacctttacaggagacttctggggccaggggacccaggtcaccgtctcctcaacgcgtcgcatgcatactagtaccacgacgccagcgccgcgaccaccaacaccggcgcccaccatcgcgtcgcagcccctgtccctgcgcccagaggcgtgccggccagcggcggggggcgcagtgcacacgagggggctggacttcgcctgtgatttttgggtgctggtggtggttggtggagtcctggcttgctatagcttgctagtaacagtggcctttattattttctgggtgaggagtaagaggagcaggctcctgcacagtgactacatgaacatgactccccgccgccccgggcccacccgcaagcattaccagccctatgccccaccacgcgacttcgcagcctatcgctccaaacggggcagaaagaaactcctgtatatattcaaacaaccatttatgagaccagtacaaactactcaagaggaagatggctgtagctgccgatttccagaagaagaagaaggaggatgtgaactgagagtgaagttcagcaggagcgcagacgcccccgcgtacaagcagggccagaaccagctctataacgagctcaatctaggacgaagagaggagtacgatgttttggacaagagacgtggccgggaccctgagatggggggaaagccgagaaggaagaaccctcaggaaggcctgtacaatgaactgcagaaagataagatggcggaggcctacagtgagattgggatgaaaggcgagcgccggaggggcaaggggcacgatggcctttaccagggtctcagtacagccaccaaggacacctacgacgcccttcacatgcaggccctgccccctcgctga

SEQ ID NO: 190 - DNA, 1242 bp, synthetic construct
  source 1..1242: mol_type = other DNA; note = CD38 38A37717 CAR
atggccttaccagtgaccgccttgctcctgccgctggccttgctgctccacgccgccaggccggttaacgaggtgcagctggtggaaagcggggggggactggtgcaggcaggcgggtcactgagactgtcatgtatcgcaactgggaaggtgtttagcatctacgacatgggctggtataggcaggcaccaggaaagcagagggagctggtggccgagatcaccagctccggcaccacacactacgacgatttcgtgtctggccggtttaccatcagcagagacaacgccaagaatacagtgtatctgcagatgaacaccctgaaggccgaggatacagccgtgtactattgccgggctaatcacgtcttcggcggctcctactgggggcagggaactcaggtcactgtgtcatccacgcgtcgcatgcatactagtaccacgacgccagcgccgcgaccaccaacaccggcgcccaccatcgcgtcgcagcccctgtccctgcgcccagaggcgtgccggccagcggcggggggcgcagtgcacacgagggggctggacttcgcctgtgatttttgggtgctggtggtggttggtggagtcctggcttgctatagcttgctagtaacagtggcctttattattttctgggtgaggagtaagaggagcaggctcctgcacagtgactacatgaacatgactccccgccgccccgggcccacccgcaagcattaccagccctatgccccaccacgcgacttcgcagcctatcgctccaaacggggcagaaagaaactcctgtatatattcaaacaaccatttatgagaccagtacaaactactcaagaggaagatggctgtagctgccgatttccagaagaagaagaaggaggatgtgaactgagagtgaagttcagcaggagcgcagacgcccccgcgtacaagcagggccagaaccagctctataacgagctcaatctaggacgaagagaggagtacgatgttttggacaagagacgtggccgggaccctgagatggggggaaagccgagaaggaagaaccctcaggaaggcctgtacaatgaactgcagaaagataagatggcggaggcctacagtgagattgggatgaaaggcgagcgccggaggggcaaggggcacgatggcctttaccagggtctcagtacagccaccaaggacacctacgacgcccttcacatgcaggccctgccccctcgctga

SEQ ID NO: 191 - DNA, 1239 bp, synthetic construct
  source 1..1239: mol_type = other DNA; note = CD38 38A37719 CAR
atggccttaccagtgaccgccttgctcctgccgctggccttgctgctccacgccgccaggccggttaaccaggtaaagctggaggagtctgggggaggctcggtgcagactggggggtctctgagactctcctgtgcagcctctgcaagcatcttcactaggctgcccatgggctggtaccgccaggctccagggaagcagcgcgagttggtcgtaggcattgttcctagtggtaggataaactatgcagactccgtgaagggccgattcaccatctccagagacaacgccaagaacacggtgtatctgcaaatgaacagcctgcgccctgaggacacagccgtctattactgccgcgccgataccttccccttgcccacctggggccaggggacccaggtcaccgtctcctcaacgcgtcgcatgcatactagtaccacgacgccagcgccgcgaccaccaacaccggcgcccaccatcgcgtcgcagcccctgtccctgcgcccagaggcgtgccggccagcggcggggggcgcagtgcacacgagggggctggacttcgcctgtgatttttgggtgctggtggtggttggtggagtcctggcttgctatagcttgctagtaacagtggcctttattattttctgggtgaggagtaagaggagcaggctcctgcacagtgactacatgaacatgactccccgccgccccgggcccacccgcaagcattaccagccctatgccccaccacgcgacttcgcagcctatcgctccaaacggggcagaaagaaactcctgtatatattcaaacaaccatttatgagaccagtacaaactactcaagaggaagatggctgtagctgccgatttccagaagaagaagaaggaggatgtgaactgagagtgaagttcagcaggagcgcagacgcccccgcgtacaagcagggccagaaccagctctataacgagctcaatctaggacgaagagaggagtacgatgttttggacaagagacgtggccgggaccctgagatggggggaaagccgagaaggaagaaccctcaggaaggcctgtacaatgaactgcagaaagataagatggcggaggcctacagtgagattgggatgaaaggcgagcgccggaggggcaaggggcacgatggcctttaccagggtctcagtacagccaccaaggacacctacgacgcccttcacatgcaggccctgccccctcgctga

SEQ ID NO: 192 - DNA, 1272 bp, synthetic construct
  source 1..1272: mol_type = other DNA; note = CD38 38A37330 CAR
atggccttaccagtgaccgccttgctcctgccgctggccttgctgctccacgccgccaggccggttaaccaggtgcagctggtggagtctgggggaggattggtgcaggctggggactctctgagactctcctgtgcagcctctggacgcgcctacgctacgatggcctggttccgccaggctccagggaaggagcgtgagtttgtagcacatctgcgcgtgagtggtgataccacttactatacagactccgtgaagggccgattcaccatctccagagacaacgccaagaacacggcgtatctgcaaatgaacatgttgaaacctgaggacacggccgtttattactgtgcagcgggaccgtatggcattcttgccgctgccagggtcagtaatccaggaaattatgattattggggccaggggacccaggtcaccgtctcctcaacgcgtcgcatgcatactagtaccacgacgccagcgccgcgaccaccaacaccggcgcccaccatcgcgtcgcagcccctgtccctgcgcccagaggcgtgccggccagcggcggggggcgcagtgcacacgagggggctggacttcgcctgtgatttttgggtgctggtggtggttggtggagtcctggcttgctatagcttgctagtaacagtggcctttattattttctgggtgaggagtaagaggagcaggctcctgcacagtgactacatgaacatgactccccgccgccccgggcccacccgcaagcattaccagccctatgccccaccacgcgacttcgcagcctatcgctccaaacggggcagaaagaaactcctgtatatattcaaacaaccatttatgagaccagtacaaactactcaagaggaagatggctgtagctgccgatttccagaagaagaagaaggaggatgtgaactgagagtgaagttcagcaggagcgcagacgcccccgcgtacaagcagggccagaaccagctctataacgagctcaatctaggacgaagagaggagtacgatgttttggacaagagacgtggccgggaccctgagatggggggaaagccgagaaggaagaaccctcaggaaggcctgtacaatgaactgcagaaagataagatggcggaggcctacagtgagattgggatgaaaggcgagcgccggaggggcaaggggcacgatggcctttaccagggtctcagtacagccaccaaggacacctacgacgcccttcacatgcaggccctgccccctcgctga

SEQ ID NO: 193 - DNA, 1263 bp, synthetic construct
  source 1..1263: mol_type = other DNA; note = CD38 38A37334 CAR
atggccttaccagtgaccgccttgctcctgccgctggccttgctgctccacgccgccaggccggttaacgaggtgcagctggtggagtctgggggaggattggtgcaggctgggggctctctgagactctcctgtgcagcctctggactcaccttcagtagttatattatgggctggttccgccaggctccaggcgaggagcgcgagttggtcgcggaaattagtagcggtggtatgacatcgtatgcagactccgtgaagggccgattcaccatctccagagacaacgccaagaagacggggtatctgcaaatgaacagcctgaaacctgaggacacggccgtttactattgtgcagcccctgagaggggtagtatctggtacagccgctacgaatataagtactggggccaggggacccaggtcaccgtctcctcaacgcgtcgcatgcatactagtaccacgacgccagcgccgcgaccaccaacaccggcgcccaccatcgcgtcgcagcccctgtccctgcgcccagaggcgtgccggccagcggcggggggcgcagtgcacacgagggggctggacttcgcctgtgatttttgggtgctggtggtggttggtggagtcctggcttgctatagcttgctagtaacagtggcctttattattttctgggtgaggagtaagaggagcaggctcctgcacagtgactacatgaacatgactccccgccgccccgggcccacccgcaagcattaccagccctatgccccaccacgcgacttcgcagcctatcgctccaaacggggcagaaagaaactcctgtatatattcaaacaaccatttatgagaccagtacaaactactcaagaggaagatggctgtagctgccgatttccagaagaagaagaaggaggatgtgaactgagagtgaagttcagcaggagcgcagacgcccccgcgtacaagcagggccagaaccagctctataacgagctcaatctaggacgaagagaggagtacgatgttttggacaagagacgtggccgggaccctgagatggggggaaagccgagaaggaagaaccctcaggaaggcctgtacaatgaactgcagaaagataagatggcggaggcctacagtgagattgggatgaaaggcgagcgccggaggggcaaggggcacgatggcctttaccagggtctcagtacagccaccaaggacacctacgacgcccttcacatgcaggccctgccccctcgctga

SEQ ID NO: 194 - DNA, 1254 bp, synthetic construct
  source 1..1254: mol_type = other DNA; note = CD38 38A37730 CAR
atggccttaccagtgaccgccttgctcctgccgctggccttgctgctccacgccgccaggccggttaacgccgtgcagctggtggattctgggggaggcttggcgcagactggggggtctctgagactctcctgtgcagcctctcaagggatcttcactatcaatgccatgggctggtaccgccaggttccagggaagcagcgggagttggtcgcagaagttagtagtggtggccgcacagactatgcagactccgtgaagggccgattcaccatctccagagacaacgccaagaacacggtgtacctgcaaatgaacagcctgaaacctgaggacacaggcgtctattattgtcgagtttctggatggcatgtgtttgtcggtgaccgcatagtttggggccagggcaccctggtcactgtctcctcaacgcgtcgcatgcatactagtaccacgacgccagcgccgcgaccaccaacaccggcgcccaccatcgcgtcgcagcccctgtccctgcgcccagaggcgtgccggccagcggcggggggcgcagtgcacacgagggggctggacttcgcctgtgatttttgggtgctggtggtggttggtggagtcctggcttgctatagcttgctagtaacagtggcctttattattttctgggtgaggagtaagaggagcaggctcctgcacagtgactacatgaacatgactccccgccgccccgggcccacccgcaagcattaccagccctatgccccaccacgcgacttcgcagcctatcgctccaaacggggcagaaagaaactcctgtatatattcaaacaaccatttatgagaccagtacaaactactcaagaggaagatggctgtagctgccgatttccagaagaagaagaaggaggatgtgaactgagagtgaagttcagcaggagcgcagacgcccccgcgtacaagcagggccagaaccagctctataacgagctcaatctaggacgaagagaggagtacgatgttttggacaagagacgtggccgggaccctgagatggggggaaagccgagaaggaagaaccctcaggaaggcctgtacaatgaactgcagaaagataagatggcggaggcctacagtgagattgggatgaaaggcgagcgccggaggggcaaggggcacgatggcctttaccagggtctcagtacagccaccaaggacacctacgacgcccttcacatgcaggccctgccccctcgctga

SEQ ID NO: 195 - DNA, 1263 bp, synthetic construct
  source 1..1263: mol_type = other DNA; note = CD38 38A37340 CAR
atggccttaccagtgaccgccttgctcctgccgctggccttgctgctccacgccgccaggccggttaacgatgtgcagctggtggagtctgggggaggattggtgcaggctggggactctctgagactctcctgtgcagcctctggacgcaccttcagtagctatgccatggcctggttccgccaggctccagggaaggagcgtgagattgtttcgtctatcagtaccagtggtggtatcacagactatgcagactccgtgaagggccgattcaccatctccaaagacagcgcgaagatgaacacggtgtatctgcaaatgaatagcctagaacctgaggacacggccgtttactactgtgcggcccgtacatggtaccttcgtacttctctccaatatgactattggggccaggggacccaggtcaccgtctcctcaacgcgtcgcatgcatactagtaccacgacgccagcgccgcgaccaccaacaccggcgcccaccatcgcgtcgcagcccctgtccctgcgcccagaggcgtgccggccagcggcggggggcgcagtgcacacgagggggctggacttcgcctgtgatttttgggtgctggtggtggttggtggagtcctggcttgctatagcttgctagtaacagtggcctttattattttctgggtgaggagtaagaggagcaggctcctgcacagtgactacatgaacatgactccccgccgccccgggcccacccgcaagcattaccagccctatgccccaccacgcgacttcgcagcctatcgctccaaacggggcagaaagaaactcctgtatatattcaaacaaccatttatgagaccagtacaaactactcaagaggaagatggctgtagctgccgatttccagaagaagaagaaggaggatgtgaactgagagtgaagttcagcaggagcgcagacgcccccgcgtacaagcagggccagaaccagctctataacgagctcaatctaggacgaagagaggagtacgatgttttggacaagagacgtggccgggaccctgagatggggggaaagccgagaaggaagaaccctcaggaaggcctgtacaatgaactgcagaaagataagatggcggaggcctacagtgagattgggatgaaaggcgagcgccggaggggcaaggggcacgatggcctttaccagggtctcagtacagccaccaaggacacctacgacgcccttcacatgcaggccctgccccctcgctga

SEQ ID NO: 196 - DNA, 1257 bp, synthetic construct
  source 1..1257: mol_type = other DNA; note = CD38 38A37731 CAR
atggccttaccagtgaccgccttgctcctgccgctggccttgctgctccacgccgccaggccggttaaccaggtaaagctggaggagtctgggggaggcttggtgcaggctggggggtctctgagactctcctgtgtagcctctggaaccatcgtcagtatcagtaccatgggctggtaccgccaggctccagggaagcagcgcgagttggtcgcgactataaccaggcgtggacgcacgaactatacagactccgtgaagggccgattcaccatctccagagacaacgccaaaaacacggtgtatctgcaaatgaacagcctgaaacctgaggacacagccgtctattactgtaatgcagaggtgcaactggatatatgggcatctgcgtatgactactggggccaggggacccaggtcaccgtcgcctcaacgcgtcgcatgcatactagtaccacgacgccagcgccgcgaccaccaacaccggcgcccaccatcgcgtcgcagcccctgtccctgcgcccagaggcgtgccggccagcggcggggggcgcagtgcacacgagggggctggacttcgcctgtgatttttgggtgctggtggtggttggtggagtcctggcttgctatagcttgctagtaacagtggcctttattattttctgggtgaggagtaagaggagcaggctcctgcacagtgactacatgaacatgactccccgccgccccgggcccacccgcaagcattaccagccctatgccccaccacgcgacttcgcagcctatcgctccaaacggggcagaaagaaactcctgtatatattcaaacaaccatttatgagaccagtacaaactactcaagaggaagatggctgtagctgccgatttccagaagaagaagaaggaggatgtgaactgagagtgaagttcagcaggagcgcagacgcccccgcgtacaagcagggccagaaccagctctataacgagctcaatctaggacgaagagaggagtacgatgttttggacaagagacgtggccgggaccctgagatggggggaaagccgagaaggaagaaccctcaggaaggcctgtacaatgaactgcagaaagataagatggcggaggcctacagtgagattgggatgaaaggcgagcgccggaggggcaaggggcacgatggcctttaccagggtctcagtacagccaccaaggacacctacgacgcccttcacatgcaggccctgccccctcgctga

SEQ ID NO: 197 - DNA, 1239 bp, synthetic construct
  source 1..1239: mol_type = other DNA; note = CD38 38A37326 CAR
atggccttaccagtgaccgccttgctcctgccgctggccttgctgctccacgccgccaggccggttaacgaggtgcagctggtggagtctgggggaggattggtgcaggctgggggctctctgagactctcctgtgcagcctctggacgcacctatgccatgggctggtatcgccaggctccagggaagcagcgcgacttggtcgcaactattagtggtgcgggtaacacaaagtatgcagactccgtgaagggccgattcaccatctccagagacaacgccaagaacacaatgtatctgcaaatgaacagcctgaaacctgaggacacggccgtttattactgtgccgcgggtaaatggttccctgctgcgaatgagtactggggccaggggacccaggtcaccgtctcctcaacgcgtcgcatgcatactagtaccacgacgccagcgccgcgaccaccaacaccggcgcccaccatcgcgtcgcagcccctgtccctgcgcccagaggcgtgccggccagcggcggggggcgcagtgcacacgagggggctggacttcgcctgtgatttttgggtgctggtggtggttggtggagtcctggcttgctatagcttgctagtaacagtggcctttattattttctgggtgaggagtaagaggagcaggctcctgcacagtgactacatgaacatgactccccgccgccccgggcccacccgcaagcattaccagccctatgccccaccacgcgacttcgcagcctatcgctccaaacggggcagaaagaaactcctgtatatattcaaacaaccatttatgagaccagtacaaactactcaagaggaagatggctgtagctgccgatttccagaagaagaagaaggaggatgtgaactgagagtgaagttcagcaggagcgcagacgcccccgcgtacaagcagggccagaaccagctctataacgagctcaatctaggacgaagagaggagtacgatgttttggacaagagacgtggccgggaccctgagatggggggaaagccgagaaggaagaaccctcaggaaggcctgtacaatgaactgcagaaagataagatggcggaggcctacagtgagattgggatgaaaggcgagcgccggaggggcaaggggcacgatggcctttaccagggtctcagtacagccaccaaggacacctacgacgcccttcacatgcaggccctgccccctcgctga

SEQ ID NO: 198 - protein, 495 aa, synthetic construct
  source 1..495: note = BCMAx2 269A37946 GSI5014 CAR
MALPVTALLLPLALLLHAARPQVQLVESGGGLVQPGGSLRLSCEASGFTLDYYAIGWFRQAPGKEREGVICISRSDGSTYYADSVKGRFTISRDNAKKTVYLQMISLKPEDTAAYYCAAGADCSGYLRDYEFRGQGTQVTVSSGGGGSQVQLVESGGGLVQPGGSLRLSCEASGFTLDYYAIGWFRQAPGKEREGVICISRSDGSTYYADSVKGRFTISRDNAKKTVYLQMISLKPEDTAAYYCAAGADCSGYLRDYEFRGQGTQVTVSSTSTTTPAPRPPTPAPTIASQPLSLRPEACRPAAGGAVHTRGLDFACDIYIWAPLAGTCGVLLLSLVITLYCKRGRKKLLYIFKQPFMRPVQTTQEEDGCSCRFPEEEEGGCELRVKFSRSADAPAYQQGQNQLYNELNLGRREEYDVLDKRRGRDPEMGGKPRRKNPQEGLYNELQKDKMAEAYSEIGMKGERRRGKGHDGLYQGLSTATKDTYDALHMQALPPR

SEQ ID NO: 199 - protein, 622 aa, synthetic construct
  source 1..622: note = BCMAx3 269A37946 GSI5015 CAR
MALPVTALLLPLALLLHAARPQVQLVESGGGLVQPGGSLRLSCEASGFTLDYYAIGWFRQAPGKEREGVICISRSDGSTYYADSVKGRFTISRDNAKKTVYLQMISLKPEDTAAYYCAAGADCSGYLRDYEFRGQGTQVTVSSGGGGSQVQLVESGGGLVQPGGSLRLSCEASGFTLDYYAIGWFRQAPGKEREGVICISRSDGSTYYADSVKGRFTISRDNAKKTVYLQMISLKPEDTAAYYCAAGADCSGYLRDYEFRGQGTQVTVSSGGGGSQVQLVESGGGLVQPGGSLRLSCEASGFTLDYYAIGWFRQAPGKEREGVICISRSDGSTYYADSVKGRFTISRDNAKKTVYLQMISLKPEDTAAYYCAAGADCSGYLRDYEFRGQGTQVTVSSTSTTTPAPRPPTPAPTIASQPLSLRPEACRPAAGGAVHTRGLDFACDIYIWAPLAGTCGVLLLSLVITLYCKRGRKKLLYIFKQPFMRPVQTTQEEDGCSCRFPEEEEGGCELRVKFSRSADAPAYQQGQNQLYNELNLGRREEYDVLDKRRGRDPEMGGKPRRKNPQEGLYNELQKDKMAEAYSEIGMKGERRRGKGHDGLYQGLSTATKDTYDALHMQALPPR

SEQ ID NO: 200 - protein, 483 aa, synthetic construct
  source 1..483: note = CD38x2 38A37717 GSI5016 CAR
MALPVTALLLPLALLLHAARPEVQLVESGGGLVQAGGSLRLSCIATGKVFSIYDMGWYRQAPGKQRELVAEITSSGTTHYDDFVSGRFTISRDNAKNTVYLQMNTLKAEDTAVYYCRANHVFGGSYWGQGTQVTVSSGGGGSEVQLVESGGGLVQAGGSLRLSCIATGKVFSIYDMGWYRQAPGKQRELVAEITSSGTTHYDDFVSGRFTISRDNAKNTVYLQMNTLKAEDTAVYYCRANHVFGGSYWGQGTQVTVSSTSTTTPAPRPPTPAPTIASQPLSLRPEACRPAAGGAVHTRGLDFACDIYIWAPLAGTCGVLLLSLVITLYCKRGRKKLLYIFKQPFMRPVQTTQEEDGCSCRFPEEEEGGCELRVKFSRSADAPAYQQGQNQLYNELNLGRREEYDVLDKRRGRDPEMGGKPRRKNPQEGLYNELQKDKMAEAYSEIGMKGERRRGKGHDGLYQGLSTATKDTYDALHMQALPPR

SEQ ID NO: 201 - protein, 604 aa, synthetic construct
  source 1..604: note = CD38x3 38A37717 GSI5017 CAR
MALPVTALLLPLALLLHAARPEVQLVESGGGLVQAGGSLRLSCIATGKVFSIYDMGWYRQAPGKQRELVAEITSSGTTHYDDFVSGRFTISRDNAKNTVYLQMNTLKAEDTAVYYCRANHVFGGSYWGQGTQVTVSSGGGGSEVQLVESGGGLVQAGGSLRLSCIATGKVFSIYDMGWYRQAPGKQRELVAEITSSGTTHYDDFVSGRFTISRDNAKNTVYLQMNTLKAEDTAVYYCRANHVFGGSYWGQGTQVTVSSGGGGSEVQLVESGGGLVQAGGSLRLSCIATGKVFSIYDMGWYRQAPGKQRELVAEITSSGTTHYDDFVSGRFTISRDNAKNTVYLQMNTLKAEDTAVYYCRANHVFGGSYWGQGTQVTVSSTSTTTPAPRPPTPAPTIASQPLSLRPEACRPAAGGAVHTRGLDFACDIYIWAPLAGTCGVLLLSLVITLYCKRGRKKLLYIFKQPFMRPVQTTQEEDGCSCRFPEEEEGGCELRVKFSRSADAPAYQQGQNQLYNELNLGRREEYDVLDKRRGRDPEMGGKPRRKNPQEGLYNELQKDKMAEAYSEIGMKGERRRGKGHDGLYQGLSTATKDTYDALHMQALPPR

SEQ ID NO: 202 - DNA, 1488 bp, synthetic construct
  source 1..1488: mol_type = other DNA; note = BCMAx2 269A37946 GSI5014 CAR
atggctctgcccgtcactgctctgctgctgcccctggctctgctgctgcacgctgctcgccctcaggtccagctggtggaaagcggaggaggcctggtgcagccaggaggcagcctgaggctgtcctgcgaggcctctggcttcaccctggactactatgccatcggctggtttaggcaggcacctggaaaggagagggagggagtgatctgtatctctcgcagcgacggcagcacatactatgccgattccgtgaagggccggttcaccatcagcagagacaacgccaagaagacagtgtacctgcagatgatctccctgaagcctgaggataccgcagcatactattgcgcagcaggagcagactgtagcggatacctgagggattatgagtttaggggacagggaacccaggtgacagtgagctccggaggaggaggctcccaggtgcagctggtggagtctggaggcggcctggtgcagcctggaggcagcctgagactgagctgtgaagcttccggatttaccctggactactatgcaatcggatggtttaggcaggcaccaggaaaggagagagaaggcgtgatctgtatctccagatctgacggctctacatactatgccgatagtgtcaaaggacggttcaccatctctagagataatgccaagaagacagtctatctgcagatgattagcctgaagcccgaggacacagccgcctattactgcgcagcaggagcagattgtagtgggtatctgagggactatgagtttcgggggcaggggacacaggtgacagtgagttctactagtaccacgacgccagcgccgcgaccaccaacaccggcgcccaccatcgcgtcgcagcccctgtccctgcgcccagaggcgtgccggccagcggcggggggcgcagtgcacacgagggggctggacttcgcctgtgatatctacatctgggcgcccttggccgggacttgtggggtccttctcctgtcactggttatcaccctttactgcaaacggggcagaaagaaactcctgtatatattcaaacaaccatttatgagaccagtacaaactactcaagaggaagatggctgtagctgccgatttccagaagaagaagaaggaggatgtgaactgagagtgaagttcagcaggagcgcagacgcccccgcgtaccagcagggccagaaccagctctataacgagctcaatctaggacgaagagaggagtacgatgttttggacaagagacgtggccgggaccctgagatggggggaaagccgagaaggaagaaccctcaggaaggcctgtacaatgaactgcagaaagataagatggcggaggcctacagtgagattgggatgaaaggcgagcgccggaggggcaaggggcacgatggcctttaccagggtctcagtacagccaccaaggacacctacgacgcccttcacatgcaggccctgccccctcgctaa

SEQ ID NO: 203 - DNA, 1869 bp, synthetic construct
  source 1..1869: mol_type = other DNA; note = BCMAx3 269A37946 GSI5015 CAR
atggctctgcccgtcactgctctgctgctgcctctggccctgctgctgcacgccgcacgccctcaggtccagctggtcgagtcaggaggaggcctggtgcagccaggaggctccctgcggctgtcttgcgaggccagcggcttcaccctggactactatgccatcggctggtttaggcaggcacctggaaaggagagggagggagtgatctgtatctccagatctgacggctccacatactatgccgattctgtgaagggccggttcaccatctctagagacaacgccaagaagacagtgtacctgcagatgatcagcctgaagcccgaggataccgcagcatactattgcgcagcaggagcagactgttccggatacctgagggattatgagtttaggggacagggaacccaggtgacagtgagctccggaggaggaggctcccaggtgcagctggtggagtctggaggcggcctggtgcagcctggaggctccctgaggctgtcttgcgaggcaagcggcttcaccctggattactatgcaatcggatggtttaggcaggcaccaggaaaggagagagaaggcgtgatctgtatcagccgctccgacggcagtacctactatgccgattccgtcaaaggccggttcaccatctccagagacaatgccaagaagacagtctatctgcagatgatctctctgaagcctgaggatacagccgcctattactgtgccgcaggagcagactgtagtggctatctgagagattatgagtttcgcggccagggcacccaggtgacagtgtctagcggaggaggaggcagccaggtccagctggtggaatccggcggaggcctggtgcagcccggcggctccctgagactgtcctgtgaagcctccggatttactctggattattacgctattggatggttcagacaggcccctggcaaagaaagagaaggggtgatctgtatctctcggagcgacggctctacatactatgccgatagcgtcaagggaagatttaccatctccagagataatgccaagaagacagtgtatctgcagatgatttccctgaagcccgaggacactgccgcctattactgtgcagcaggagcagattgtagcgggtatctgcgggattatgaatttagaggacagggcactcaggtgacagtctcaagcactagtaccacgacgccagcgccgcgaccaccaacaccggcgcccaccatcgcgtcgcagcccctgtccctgcgcccagaggcgtgccggccagcggcggggggcgcagtgcacacgagggggctggacttcgcctgtgatatctacatctgggcgcccttggccgggacttgtggggtccttctcctgtcactggttatcaccctttactgcaaacggggcagaaagaaactcctgtatatattcaaacaaccatttatgagaccagtacaaactactcaagaggaagatggctgtagctgccgatttccagaagaagaagaaggaggatgtgaactgagagtgaagttcagcaggagcgcagacgcccccgcgtaccagcagggccagaaccagctctataacgagctcaatctaggacgaagagaggagtacgatgttttggacaagagacgtggccgggaccctgagatggggggaaagccgagaaggaagaaccctcaggaaggcctgtacaatgaactgcagaaagataagatggcggaggcctacagtgagattgggatgaaaggcgagcgccggaggggcaaggggcacgatggcctttaccagggtctcagtacagccaccaaggacacctacgacgcccttcacatgcaggccctgccccctcgctaa

SEQ ID NO: 204 - DNA, 1452 bp, synthetic construct
  source 1..1452: mol_type = other DNA; note = CD38x2 38A37717 GSI5016 CAR
atggccctgcctgtcaccgctctgctgctgcctctggccctgctgctgcacgctgctagacccgaagtccagctggtcgaaagtgggggaggcctggtgcaggcaggaggcagcctgaggctgtcctgcatcgccaccggcaaggtgttcagcatctacgacatgggatggtataggcaggcaccaggaaagcagagagagctggtggccgagatcacaagctccggcaccacacactacgacgatttcgtgtccggccggtttaccatctctagagacaacgccaagaatacagtgtatctgcagatgaacaccctgaaggccgaggatacagccgtgtactattgccgggccaatcacgtgttcggaggatcctactggggacagggaacccaggtgacagtgtctagcggaggaggaggatctgaggtgcagctggtggagagcggaggcggcctggtgcaggccggaggctctctgagactgagctgtattgctaccggcaaggtgttttctatctacgatatgggctggtataggcaggcacctggaaagcagagggagctggtggctgaaatcacctcctctggaactacccattacgacgatttcgtgagcggcaggtttaccatctcccgcgataatgctaaaaacaccgtctacctgcagatgaatactctgaaagctgaagacacagccgtgtactattgtcgggctaaccatgtcttcgggggctcctattgggggcagggaactcaggtcaccgtgtcatcaactagtaccacgacgccagcgccgcgaccaccaacaccggcgcccaccatcgcgtcgcagcccctgtccctgcgcccagaggcgtgccggccagcggcggggggcgcagtgcacacgagggggctggacttcgcctgtgatatctacatctgggcgcccttggccgggacttgtggggtccttctcctgtcactggttatcaccctttactgcaaacggggcagaaagaaactcctgtatatattcaaacaaccatttatgagaccagtacaaactactcaagaggaagatggctgtagctgccgatttccagaagaagaagaaggaggatgtgaactgagagtgaagttcagcaggagcgcagacgcccccgcgtaccagcagggccagaaccagctctataacgagctcaatctaggacgaagagaggagtacgatgttttggacaagagacgtggccgggaccctgagatggggggaaagccgagaaggaagaaccctcaggaaggcctgtacaatgaactgcagaaagataagatggcggaggcctacagtgagattgggatgaaaggcgagcgccggaggggcaaggggcacgatggcctttaccagggtctcagtacagccaccaaggacacctacgacgcccttcacatgcaggccctgccccctcgctaa

SEQ ID NO: 205 - DNA, 1815 bp, synthetic construct
  source 1..1815: mol_type = other DNA; note = CD38x3 38A37717 GSI5017 CAR
atggctctgcctgtcaccgcactgctgctgcccctggccctgctgctgcacgccgcaagacctgaagtccagctggtcgaatccggaggaggcctggtgcaggcaggaggctccctgcggctgtcttgcatcgccaccggcaaggtgttcagcatctacgacatgggctggtataggcaggcaccaggaaagcagagggagctggtggccgagatcacaagctccggcaccacacactacgacgatttcgtgtccggccggtttaccatctctagagacaacgccaagaatacagtgtatctgcagatgaacaccctgaaggccgaggatacagccgtgtactattgccgggccaatcacgtgttcggaggatcttactggggacagggaacccaggtgacagtgtctagcggaggaggaggatccgaggtgcagctggtggagtctggaggcggcctggtgcaggccggaggcagcctgagactgtcctgtattgctaccggcaaggtgttttccatctacgatatgggctggtatcggcaggcccctggcaagcagagagagctggtggctgaaatcacatcctctggaactacccattacgacgatttcgtgagcggcaggtttaccatctcccgcgataatgctaaaaacaccgtctacctgcagatgaatactctgaaagctgaagacaccgctgtgtactattgcagagctaaccatgtgttcggaggaagctattggggccagggcactcaggtgacagtgagctccggcggcggcggcagtgaagtgcagctggtggagtccggagggggcctggtgcaggccggcggctctctgcgcctgagctgtattgcaactggaaaagtgttttccatttatgatatgggatggtacagacaggcccctgggaaacagagagagctggtggcagaaatcacctctagtggaactacccactatgatgatttcgtgtctggccggtttaccatcagcagggataatgctaaaaacactgtctacctgcagatgaacactctgaaagctgaagataccgccgtgtactattgtagggctaaccatgtctttggggggtcatactgggggcaggggactcaggtcaccgtctcatccactagtaccacgacgccagcgccgcgaccaccaacaccggcgcccaccatcgcgtcgcagcccctgtccctgcgcccagaggcgtgccggccagcggcggggggcgcagtgcacacgagggggctggacttcgcctgtgatatctacatctgggcgcccttggccgggacttgtggggtccttctcctgtcactggttatcaccctttactgcaaacggggcagaaagaaactcctgtatatattcaaacaaccatttatgagaccagtacaaactactcaagaggaagatggctgtagctgccgatttccagaagaagaagaaggaggatgtgaactgagagtgaagttcagcaggagcgcagacgcccccgcgtaccagcagggccagaaccagctctataacgagctcaatctaggacgaagagaggagtacgatgttttggacaagagacgtggccgggaccctgagatggggggaaagccgagaaggaagaaccctcaggaaggcctgtacaatgaactgcagaaagataagatggcggaggcctacagtgagattgggatgaaaggcgagcgccggaggggcaaggggcacgatggcctttaccagggtctcagtacagccaccaaggacacctacgacgcccttcacatgcaggccctgccccctcgctaa

SEQ ID NO: 206 - protein, 502 aa, synthetic construct
  source 1..502: note = CD19XCD20 single-domain antibody-based bispecific CAR
MALPVTALLLPLALLLHAARPQVKLEESGGELVQPGGPLRLSCAASGNIFSINRMGWYRQAPGKQRAFVASITVRGITNYADSVKGRFTISVDKSKNTIYLQMNALKPEDTAVYYCNAVSSNRDPDYWGQGTQVTVSSGGGSGGGSGGGSGGGSPVQLVESGGGLVQAGDSLRLSCAASGRTFGIGTMGWFRQPPGKEREFVAAIRWSTGGTRYADSVKGRFTISRDNAKLTVDLQMDSLKPEDTAVYYCAADRLSLDLSGRYHYNPAVYDYWGQGTQVTVSSIEVMYPPPYLDNEKSNGTIIHVKGKHLCPSPLFPGPSKPFWVLVVVGGVLACYSLLVTVAFIIFWVRSKRSRLLHSDYMNMTPRRPGPTRKHYQPYAPPRDFAAYRSRVKFSRSADAPAYQQGQNQLYNELNLGRREEYDVLDKRRGRDPEMGGKPRRKNPQEGLYNELQKDKMAEAYSEIGMKGERRRGKGHDGLYQGLSTATKDTYDALHMQALPPR

SEQ ID NO: 207 - protein, 489 aa, synthetic construct
  source 1..489: note = CD38xBCMA 38A37717 269A37346 GSI5001 CAR
MALPVTALLLPLALLLHAARPEVQLVESGGGLVQAGGSLRLSCIATGKVFSIYDMGWYRQAPGKQRELVAEITSSGTTHYDDFVSGRFTISRDNAKNTVYLQMNTLKAEDTAVYYCRANHVFGGSYWGQGTQVTVSSGGGGSQVQLVESGGGLVQPGGSLRLSCEASGFTLDYYAIGWFRQAPGKEREGVICISRSDGSTYYADSVKGRFTISRDNAKKTVYLQMISLKPEDTAAYYCAAGADCSGYLRDYEFRGQGTQVTVSSTSTTTPAPRPPTPAPTIASQPLSLRPEACRPAAGGAVHTRGLDFACDIYIWAPLAGTCGVLLLSLVITLYCKRGRKKLLYIFKQPFMRPVQTTQEEDGCSCRFPEEEEGGCELRVKFSRSADAPAYQQGQNQLYNELNLGRREEYDVLDKRRGRDPEMGGKPRRKNPQEGLYNELQKDKMAEAYSEIGMKGERRRGKGHDGLYQGLSTATKDTYDALHMQALPPR

SEQ ID NO: 208 - protein, 494 aa, synthetic construct
  source 1..494: note = CD38xBCMA 38A37717 269A37346 GSI5002 CAR
MALPVTALLLPLALLLHAARPEVQLVESGGGLVQAGGSLRLSCIATGKVFSIYDMGWYRQAPGKQRELVAEITSSGTTHYDDFVSGRFTISRDNAKNTVYLQMNTLKAEDTAVYYCRANHVFGGSYWGQGTQVTVSSGGGGSGGGGSQVQLVESGGGLVQPGGSLRLSCEASGFTLDYYAIGWFRQAPGKEREGVICISRSDGSTYYADSVKGRFTISRDNAKKTVYLQMISLKPEDTAAYYCAAGADCSGYLRDYEFRGQGTQVTVSSTSTTTPAPRPPTPAPTIASQPLSLRPEACRPAAGGAVHTRGLDFACDIYIWAPLAGTCGVLLLSLVITLYCKRGRKKLLYIFKQPFMRPVQTTQEEDGCSCRFPEEEEGGCELRVKFSRSADAPAYQQGQNQLYNELNLGRREEYDVLDKRRGRDPEMGGKPRRKNPQEGLYNELQKDKMAEAYSEIGMKGERRRGKGHDGLYQGLSTATKDTYDALHMQALPPR

SEQ ID NO: 209 - protein, 500 aa, synthetic construct
  source 1..500: note = CD38xBCMA 38A37717 269A37346 GSI5003 CAR
MALPVTALLLPLALLLHAARPEVQLVESGGGLVQAGGSLRLSCIATGKVFSIYDMGWYRQAPGKQRELVAEITSSGTTHYDDFVSGRFTISRDNAKNTVYLQMNTLKAEDTAVYYCRANHVFGGSYWGQGTQVTVSSGGGSGGGSGGGSGGGSQVQLVESGGGLVQPGGSLRLSCEASGFTLDYYAIGWFRQAPGKEREGVICISRSDGSTYYADSVKGRFTISRDNAKKTVYLQMISLKPEDTAAYYCAAGADCSGYLRDYEFRGQGTQVTVSSTSTTTPAPRPPTPAPTIASQPLSLRPEACRPAAGGAVHTRGLDFACDIYIWAPLAGTCGVLLLSLVITLYCKRGRKKLLYIFKQPFMRPVQTTQEEDGCSCRFPEEEEGGCELRVKFSRSADAPAYQQGQNQLYNELNLGRREEYDVLDKRRGRDPEMGGKPRRKNPQEGLYNELQKDKMAEAYSEIGMKGERRRGKGHDGLYQGLSTATKDTYDALHMQALPPR

SEQ ID NO: 210 - protein, 508 aa, synthetic construct
  source 1..508: note = CD38xBCMA 38A37717 269A37346 GSI5004 CAR
MALPVTALLLPLALLLHAARPEVQLVESGGGLVQAGGSLRLSCIATGKVFSIYDMGWYRQAPGKQRELVAEITSSGTTHYDDFVSGRFTISRDNAKNTVYLQMNTLKAEDTAVYYCRANHVFGGSYWGQGTQVTVSSGGGGSGGGGSGGGGGGSGSGGGGSQVQLVESGGGLVQPGGSLRLSCEASGFTLDYYAIGWFRQAPGKEREGVICISRSDGSTYYADSVKGRFTISRDNAKKTVYLQMISLKPEDTAAYYCAAGADCSGYLRDYEFRGQGTQVTVSSTSTTTPAPRPPTPAPTIASQPLSLRPEACRPAAGGAVHTRGLDFACDIYIWAPLAGTCGVLLLSLVITLYCKRGRKKLLYIFKQPFMRPVQTTQEEDGCSCRFPEEEEGGCELRVKFSRSADAPAYQQGQNQLYNELNLGRREEYDVLDKRRGRDPEMGGKPRRKNPQEGLYNELQKDKMAEAYSEIGMKGERRRGKGHDGLYQGLSTATKDTYDALHMQALPPR

SEQ ID NO: 211 - protein, 518 aa, synthetic construct
  source 1..518: note = CD38xBCMA 38A37717 269A37346 GSI5005 CAR
MALPVTALLLPLALLLHAARPEVQLVESGGGLVQAGGSLRLSCIATGKVFSIYDMGWYRQAPGKQRELVAEITSSGTTHYDDFVSGRFTISRDNAKNTVYLQMNTLKAEDTAVYYCRANHVFGGSYWGQGTQVTVSSGGGGSGGGGSGGGGGGSGSGGGGSGGGGSGGGGSQVQLVESGGGLVQPGGSLRLSCEASGFTLDYYAIGWFRQAPGKEREGVICISRSDGSTYYADSVKGRFTISRDNAKKTVYLQMISLKPEDTAAYYCAAGADCSGYLRDYEFRGQGTQVTVSSTSTTTPAPRPPTPAPTIASQPLSLRPEACRPAAGGAVHTRGLDFACDIYIWAPLAGTCGVLLLSLVITLYCKRGRKKLLYIFKQPFMRPVQTTQEEDGCSCRFPEEEEGGCELRVKFSRSADAPAYQQGQNQLYNELNLGRREEYDVLDKRRGRDPEMGGKPRRKNPQEGLYNELQKDKMAEAYSEIGMKGERRRGKGHDGLYQGLSTATKDTYDALHMQALPPR

SEQ ID NO: 212 - protein, 489 aa, synthetic construct
  source 1..489: note = BCMAxCD38 269A37346 38A37717 GSI5006 CAR
MALPVTALLLPLALLLHAARPQVQLVESGGGLVQPGGSLRLSCEASGFTLDYYAIGWFRQAPGKEREGVICISRSDGSTYYADSVKGRFTISRDNAKKTVYLQMISLKPEDTAAYYCAAGADCSGYLRDYEFRGQGTQVTVSSGGGGSEVQLVESGGGLVQAGGSLRLSCIATGKVFSIYDMGWYRQAPGKQRELVAEITSSGTTHYDDFVSGRFTISRDNAKNTVYLQMNTLKAEDTAVYYCRANHVFGGSYWGQGTQVTVSSTSTTTPAPRPPTPAPTIASQPLSLRPEACRPAAGGAVHTRGLDFACDIYIWAPLAGTCGVLLLSLVITLYCKRGRKKLLYIFKQPFMRPVQTTQEEDGCSCRFPEEEEGGCELRVKFSRSADAPAYQQGQNQLYNELNLGRREEYDVLDKRRGRDPEMGGKPRRKNPQEGLYNELQKDKMAEAYSEIGMKGERRRGKGHDGLYQGLSTATKDTYDALHMQALPPR

SEQ ID NO: 213 - protein, 494 aa, synthetic construct
  source 1..494: note = BCMAxCD38 269A37346 38A37717 GSI5007 CAR
MALPVTALLLPLALLLHAARPQVQLVESGGGLVQPGGSLRLSCEASGFTLDYYAIGWFRQAPGKEREGVICISRSDGSTYYADSVKGRFTISRDNAKKTVYLQMISLKPEDTAAYYCAAGADCSGYLRDYEFRGQGTQVTVSSGGGGSGGGGSEVQLVESGGGLVQAGGSLRLSCIATGKVFSIYDMGWYRQAPGKQRELVAEITSSGTTHYDDFVSGRFTISRDNAKNTVYLQMNTLKAEDTAVYYCRANHVFGGSYWGQGTQVTVSSTSTTTPAPRPPTPAPTIASQPLSLRPEACRPAAGGAVHTRGLDFACDIYIWAPLAGTCGVLLLSLVITLYCKRGRKKLLYIFKQPFMRPVQTTQEEDGCSCRFPEEEEGGCELRVKFSRSADAPAYQQGQNQLYNELNLGRREEYDVLDKRRGRDPEMGGKPRRKNPQEGLYNELQKDKMAEAYSEIGMKGERRRGKGHDGLYQGLSTATKDTYDALHMQALPPR

SEQ ID NO: 214 - protein, 500 aa, synthetic construct
  source 1..500: note = BCMAxCD38 269A37346 38A37717 GSI5008 CAR
MALPVTALLLPLALLLHAARPQVQLVESGGGLVQPGGSLRLSCEASGFTLDYYAIGWFRQAPGKEREGVICISRSDGSTYYADSVKGRFTISRDNAKKTVYLQMISLKPEDTAAYYCAAGADCSGYLRDYEFRGQGTQVTVSSGGGSGGGSGGGSGGGSEVQLVESGGGLVQAGGSLRLSCIATGKVFSIYDMGWYRQAPGKQRELVAEITSSGTTHYDDFVSGRFTISRDNAKNTVYLQMNTLKAEDTAVYYCRANHVFGGSYWGQGTQVTVSSTSTTTPAPRPPTPAPTIASQPLSLRPEACRPAAGGAVHTRGLDFACDIYIWAPLAGTCGVLLLSLVITLYCKRGRKKLLYIFKQPFMRPVQTTQEEDGCSCRFPEEEEGGCELRVKFSRSADAPAYQQGQNQLYNELNLGRREEYDVLDKRRGRDPEMGGKPRRKNPQEGLYNELQKDKMAEAYSEIGMKGERRRGKGHDGLYQGLSTATKDTYDALHMQALPPR

SEQ ID NO: 215 - protein, 510 aa, synthetic construct
  source 1..510: note = BCMAxCD38 269A37346 38A37717 GSI5009 CAR
MALPVTALLLPLALLLHAARPQVQLVESGGGLVQPGGSLRLSCEASGFTLDYYAIGWFRQAPGKEREGVICISRSDGSTYYADSVKGRFTISRDNAKKTVYLQMISLKPEDTAAYYCAAGADCSGYLRDYEFRGQGTQVTVSSGGGGSGGGGSGGGGGGSGSGGGGSEVQLVESGGGLVQAGGSLRLSCIATGKVFSIYDMGWYRQAPGKQRELVAEITSSGTTHYDDFVSGRFTISRDNAKNTVYLQMNTLKAEDTAVYYCRANHVFGGSYWGQGTQVTVSSTSTSTTTPAPRPPTPAPTIASQPLSLRPEACRPAAGGAVHTRGLDFACDIYIWAPLAGTCGVLLLSLVITLYCKRGRKKLLYIFKQPFMRPVQTTQEEDGCSCRFPEEEEGGCELRVKFSRSADAPAYQQGQNQLYNELNLGRREEYDVLDKRRGRDPEMGGKPRRKNPQEGLYNELQKDKMAEAYSEIGMKGERRRGKGHDGLYQGLSTATKDTYDALHMQALPPR

SEQ ID NO: 216 - protein, 518 aa, synthetic construct
  source 1..518: note = BCMAxCD38 269A37346 38A37717 GSI5010 CAR
MALPVTALLLPLALLLHAARPQVQLVESGGGLVQPGGSLRLSCEASGFTLDYYAIGWFRQAPGKEREGVICISRSDGSTYYADSVKGRFTISRDNAKKTVYLQMISLKPEDTAAYYCAAGADCSGYLRDYEFRGQGTQVTVSSGGGGSGGGGSGGGGGGSGSGGGGSGGGGSGGGGSEVQLVESGGGLVQAGGSLRLSCIATGKVFSIYDMGWYRQAPGKQRELVAEITSSGTTHYDDFVSGRFTISRDNAKNTVYLQMNTLKAEDTAVYYCRANHVFGGSYWGQGTQVTVSSTSTTTPAPRPPTPAPTIASQPLSLRPEACRPAAGGAVHTRGLDFACDIYIWAPLAGTCGVLLLSLVITLYCKRGRKKLLYIFKQPFMRPVQTTQEEDGCSCRFPEEEEGGCELRVKFSRSADAPAYQQGQNQLYNELNLGRREEYDVLDKRRGRDPEMGGKPRRKNPQEGLYNELQKDKMAEAYSEIGMKGERRRGKGHDGLYQGLSTATKDTYDALHMQALPPR

SEQ ID NO: 217 - DNA, 1521 bp, synthetic construct
  source 1..1521: mol_type = other DNA; note = CD19XCD20 single-domain antibody-based bispecific CAR
gccgccaccatggccttaccagtgaccgccttgctcctgccgctggccttgctgctccacgccgccaggccgcaggtaaagctggaggagtctgggggagaattggtgcagcctggggggcctctgagactctcctgtgcagcctcgggaaacatcttcagtatcaatcgcatgggctggtaccgccaggctccagggaagcagcgcgcgttcgtcgcatctattactgttcgtggtataacaaactatgcagactccgtgaagggccgattcaccatttctgtagacaagtccaaaaacacgatttatctgcagatgaacgcactcaaacctgaggacacggccgtctattattgtaatgcagtgtcttcaaacagggaccccgactactggggccaggggacccaggtcaccgtctcctcaggcggcggcagcggcggcggcagcggcggcggcagcggcggcggcagcccggtgcagctggtggagtctgggggaggcttggtgcaggctggggattctctgagactctcctgtgctgcctctggacgcaccttcggtattggtaccatgggctggttccgccaacctccagggaaggagcgtgaatttgtagcagctattaggtggagtactggtggcactcgctatgcagactccgtgaagggccgattcaccatctcccgagacaacgccaagctcacggtagatctgcaaatggacagcctgaaacctgaagacacggccgtttattactgtgcagcagatagactgtcccttgatttaagtggtcgttaccactacaaccccgccgtgtatgactattggggccaggggacccaggtcaccgtctcctcaattgaagttatgtatcctcctccttacctagacaatgagaagagcaatggaaccattatccatgtgaaagggaaacacctttgtccaagtcccctatttcccggaccttctaagcccttttgggtgctggtggtggttggtggagtcctggcttgctatagcttgctagtaacagtggcctttattattttctgggtgaggagtaagaggagcaggctcctgcacagtgactacatgaacatgactccccgccgccccgggcccacccgcaagcattaccagccctatgccccaccacgcgacttcgcagcctatcgctccagagtgaagttcagcaggagcgcagacgcccccgcgtaccagcagggccagaaccagctctataacgagctcaatctaggacgaagagaggagtacgatgttttggacaagagacgtggccgggaccctgagatggggggaaagccgagaaggaagaaccctcaggaaggcctgtacaatgaactgcagaaagataagatggcggaggcctacagtgagattgggatgaaaggcgagcgccggaggggcaaggggcacgatggcctttaccagggtctcagtacagccaccaaggacacctacgacgcccttcacatgcaggccctgccccctcgctgataa

SEQ ID NO: 218 - DNA, 1470 bp, synthetic construct
  source 1..1470: mol_type = other DNA; note = CD38xBCMA 38A37717 269A37346 GSI5001 CAR
atggctctgcccgtcactgctctgctgctgcccctggctctgctgctgcacgccgcaagacccgaagtccagctggtggaatctggcggaggcctggtgcaggcaggaggcagcctgaggctgtcctgcatcgccaccggcaaggtgttctccatctacgacatgggctggtatcggcaggccccaggcaagcagagagagctggtggccgagatcacaagctccggcaccacacactacgacgatttcgtgtctggccggtttaccatcagcagagacaacgccaagaatacagtgtatctgcagatgaacaccctgaaggccgaggatacagccgtgtactattgtcgggccaatcacgtgtttggaggaagctactggggacagggaacccaggtgacagtgtctagcggaggaggaggcagccaggtgcagctggtggagtccggaggaggcctggtgcagccaggaggctctctgaggctgagctgcgaggcatccggattcaccctggactactatgccatcggctggtttaggcaggcacctggaaaggagagggagggagtgatctgtatctccagatctgacggctccacatactatgccgattctgtgaagggcaggttcaccatctctcgcgataacgccaagaagacagtctacctgcagatgatcagcctgaagcccgaggacaccgcagcatactattgcgcagcaggagcagattgtagtggctatctgagggactacgagttccgagggcaggggacacaggtgaccgtgagcagcactagtaccacgacgccagcgccgcgaccaccaacaccggcgcccaccatcgcgtcgcagcccctgtccctgcgcccagaggcgtgccggccagcggcggggggcgcagtgcacacgagggggctggacttcgcctgtgatatctacatctgggcgcccttggccgggacttgtggggtccttctcctgtcactggttatcaccctttactgcaaacggggcagaaagaaactcctgtatatattcaaacaaccatttatgagaccagtacaaactactcaagaggaagatggctgtagctgccgatttccagaagaagaagaaggaggatgtgaactgagagtgaagttcagcaggagcgcagacgcccccgcgtaccagcagggccagaaccagctctataacgagctcaatctaggacgaagagaggagtacgatgttttggacaagagacgtggccgggaccctgagatggggggaaagccgagaaggaagaaccctcaggaaggcctgtacaatgaactgcagaaagataagatggcggaggcctacagtgagattgggatgaaaggcgagcgccggaggggcaaggggcacgatggcctttaccagggtctcagtacagccaccaaggacacctacgacgcccttcacatgcaggccctgccccctcgctaa

SEQ ID NO: 219 - DNA, 1485 bp, synthetic construct
  source 1..1485: mol_type = other DNA; note = CD38xBCMA 38A37717 269A37346 GSI5002 CAR
atggctctgcccgtcactgctctgctgctgcccctggctctgctgctgcacgctgctcgccctgaagtccagctggtcgaatccggcggaggcctggtgcaggcaggaggcagcctgaggctgtcctgcatcgccaccggcaaggtgttctccatctacgacatgggctggtatcggcaggccccaggcaagcagagagagctggtggccgagatcacaagctccggcaccacacactacgacgatttcgtgtccggccggtttaccatctctagagacaacgccaagaatacagtgtatctgcagatgaacaccctgaaggccgaggatacagccgtgtactattgtcgggccaatcacgtgtttggaggatcctactggggacagggaacccaggtgacagtgtctagcggaggaggaggatctggcggaggaggcagccaggtgcagctggtggagtctggaggaggcctggtgcagccaggaggctctctgaggctgagctgcgaggcatccggattcaccctggactactatgccatcggctggtttaggcaggcacctggaaaggagagggagggagtgatctgtatctccagatctgacggcagcacatactatgccgattccgtgaagggcaggttcaccatctctcgcgataacgccaagaagacagtctacctgcagatgatcagcctgaagcccgaggacaccgcagcatactattgcgcagcaggagcagattgtagcggctatctgagggattatgagtttagagggcagggaacacaggtgacagtgagcagcactagtaccacgacgccagcgccgcgaccaccaacaccggcgcccaccatcgcgtcgcagcccctgtccctgcgcccagaggcgtgccggccagcggcggggggcgcagtgcacacgagggggctggacttcgcctgtgatatctacatctgggcgcccttggccgggacttgtggggtccttctcctgtcactggttatcaccctttactgcaaacggggcagaaagaaactcctgtatatattcaaacaaccatttatgagaccagtacaaactactcaagaggaagatggctgtagctgccgatttccagaagaagaagaaggaggatgtgaactgagagtgaagttcagcaggagcgcagacgcccccgcgtaccagcagggccagaaccagctctataacgagctcaatctaggacgaagagaggagtacgatgttttggacaagagacgtggccgggaccctgagatggggggaaagccgagaaggaagaaccctcaggaaggcctgtacaatgaactgcagaaagataagatggcggaggcctacagtgagattgggatgaaaggcgagcgccggaggggcaaggggcacgatggcctttaccagggtctcagtacagccaccaaggacacctacgacgcccttcacatgcaggccctgccccctcgctaa

SEQ ID NO: 220 - DNA, 1503 bp, synthetic construct
  source 1..1503: mol_type = other DNA; note = CD38xBCMA 38A37717 269A37346 GSI5003 CAR
atggccctgcctgtcaccgcactgctgctgcccctggctctgctgctgcacgccgcacgccctgaagtccagctggtcgagtccgggggaggcctggtgcaggcaggaggcagcctgaggctgtcctgcatcgccaccggcaaggtgttctccatctacgacatgggctggtatcggcaggccccaggcaagcagagagagctggtggccgagatcacaagctccggcaccacacactacgacgatttcgtgagcggccggtttaccatctccagagacaacgccaagaatacagtgtatctgcagatgaacaccctgaaggccgaggatacagccgtgtactattgtcgggccaatcacgtgtttggaggatcctactggggacagggaacccaggtgacagtgtctagcggcggcggctctggaggaggaagcggaggaggatctggaggaggctctcaggtgcagctggtggagagcggaggaggcctggtgcagccaggaggcagcctgcggctgtcctgcgaggcctctggcttcaccctggactactatgccatcggctggtttaggcaggcacctggaaaggagagggagggagtgatctgtatctccagatctgacggctctacatactatgccgatagcgtgaagggcaggttcaccatctcccgcgataacgccaagaagacagtctacctgcagatgatctctctgaagcccgaggacaccgcagcatactattgcgcagcaggagcagattgtagcgggtatctgcgggattatgagtttagaggacaggggacacaggtcacagtcagttccactagtaccacgacgccagcgccgcgaccaccaacaccggcgcccaccatcgcgtcgcagcccctgtccctgcgcccagaggcgtgccggccagcggcggggggcgcagtgcacacgagggggctggacttcgcctgtgatatctacatctgggcgcccttggccgggacttgtggggtccttctcctgtcactggttatcaccctttactgcaaacggggcagaaagaaactcctgtatatattcaaacaaccatttatgagaccagtacaaactactcaagaggaagatggctgtagctgccgatttccagaagaagaagaaggaggatgtgaactgagagtgaagttcagcaggagcgcagacgcccccgcgtaccagcagggccagaaccagctctataacgagctcaatctaggacgaagagaggagtacgatgttttggacaagagacgtggccgggaccctgagatggggggaaagccgagaaggaagaaccctcaggaaggcctgtacaatgaactgcagaaagataagatggcggaggcctacagtgagattgggatgaaaggcgagcgccggaggggcaaggggcacgatggcctttaccagggtctcagtacagccaccaaggacacctacgacgcccttcacatgcaggccctgccccctcgctaa

SEQ ID NO: 221 - DNA, 1527 bp, synthetic construct
  source 1..1527: mol_type = other DNA; note = CD38xBCMA 38A37717 269A37346 GSI5004 CAR
atggctctgcctgtgaccgccctgctgctgcccctggctctgctgctgcacgccgcacgacccgaagtccagctggtggaatctgggggaggcctggtgcaggcaggaggctctctgaggctgagctgcatcgccaccggcaaggtgttctctatctacgacatgggctggtatcggcaggccccaggcaagcagagagagctggtggccgagatcacaagctccggcaccacacactacgacgatttcgtgagcggccggtttaccatctccagagacaacgccaagaatacagtgtatctgcagatgaacaccctgaaggccgaggatacagccgtgtactattgtcgggccaatcacgtgtttggaggaagctactggggacagggaacccaggtgacagtgtctagcggaggaggaggatccggaggaggaggatctggaggcggcggcggcggctccggctctggcggcggcggctcccaggtgcagctggtggagtctggaggaggcctggtgcagccaggaggctccctgcggctgtcttgcgaggccagcggcttcaccctggactactatgccatcggctggtttaggcaggcacctggaaaggagagggagggagtgatctgtatcagcagatccgacggctctacatactatgccgatagcgtgaagggcaggttcaccatcagccgcgataacgccaagaagacagtctacctgcagatgatctccctgaagcccgaggacaccgcagcatactattgcgcagcaggagcagattgtagcggctatctgcgggattacgagtttagaggacagggcacccaggtcaccgtctcaagcactagtaccacgacgccagcgccgcgaccaccaacaccggcgcccaccatcgcgtcgcagcccctgtccctgcgcccagaggcgtgccggccagcggcggggggcgcagtgcacacgagggggctggacttcgcctgtgatatctacatctgggcgcccttggccgggacttgtggggtccttctcctgtcactggttatcaccctttactgcaaacggggcagaaagaaactcctgtatatattcaaacaaccatttatgagaccagtacaaactactcaagaggaagatggctgtagctgccgatttccagaagaagaagaaggaggatgtgaactgagagtgaagttcagcaggagcgcagacgcccccgcgtaccagcagggccagaaccagctctataacgagctcaatctaggacgaagagaggagtacgatgttttggacaagagacgtggccgggaccctgagatggggggaaagccgagaaggaagaaccctcaggaaggcctgtacaatgaactgcagaaagataagatggcggaggcctacagtgagattgggatgaaaggcgagcgccggaggggcaaggggcacgatggcctttaccagggtctcagtacagccaccaaggacacctacgacgcccttcacatgcaggccctgccccctcgctaa

SEQ ID NO: 222 - DNA, 1557 bp, synthetic construct
  source 1..1557: mol_type = other DNA; note = CD38xBCMA 38A37717 269A37346 GSI5005 CAR
atggctctgcctgtcactgctctgctgctgcccctggccctgctgctgcacgctgctagacccgaagtccagctggtggagtccggcggaggcctggtgcaggcaggaggctctctgaggctgagctgcatcgccaccggcaaggtgttcagcatctacgacatgggctggtatcggcaggccccaggcaagcagagagagctggtggccgagatcacaagctccggcaccacacactacgacgatttcgtgagcggccggtttaccatctccagagacaacgccaagaatacagtgtatctgcagatgaacaccctgaaggccgaggatacagccgtgtactattgtcgggccaatcacgtgtttggaggaagctactggggacagggaacccaggtgacagtgtctagcggaggaggaggatccggaggaggaggatctggaggcggcggcggcggctccggctctggcggcggcggcagtggaggcggcggctccggcggcggcggctctcaggtgcagctggtggagtccggaggaggcctggtgcagccaggaggctccctgcggctgtcttgcgaggccagcggcttcaccctggactactatgccatcggctggtttaggcaggcacctggaaaggagagggagggagtgatctgtatcagcagatccgacggctctacatactatgccgatagcgtgaagggcaggttcaccatctcccgcgataacgccaagaagacagtctacctgcagatgatctctctgaagcccgaggacaccgcagcatactattgcgcagcaggagcagattgttcaggctatctgcgggattatgagtttcggggacaggggacacaggtcacagtctccagcactagtaccacgacgccagcgccgcgaccaccaacaccggcgcccaccatcgcgtcgcagcccctgtccctgcgcccagaggcgtgccggccagcggcggggggcgcagtgcacacgagggggctggacttcgcctgtgatatctacatctgggcgcccttggccgggacttgtggggtccttctcctgtcactggttatcaccctttactgcaaacggggcagaaagaaactcctgtatatattcaaacaaccatttatgagaccagtacaaactactcaagaggaagatggctgtagctgccgatttccagaagaagaagaaggaggatgtgaactgagagtgaagttcagcaggagcgcagacgcccccgcgtaccagcagggccagaaccagctctataacgagctcaatctaggacgaagagaggagtacgatgttttggacaagagacgtggccgggaccctgagatggggggaaagccgagaaggaagaaccctcaggaaggcctgtacaatgaactgcagaaagataagatggcggaggcctacagtgagattgggatgaaaggcgagcgccggaggggcaaggggcacgatggcctttaccagggtctcagtacagccaccaaggacacctacgacgcccttcacatgcaggccctgccccctcgctaa

SEQ ID NO: 223 - DNA, 1470 bp, synthetic construct
  source 1..1470: mol_type = other DNA; note = BCMAxCD38 269A37346 38A37717 GSI5006 CAR
atggctctgcccgtcaccgctctgctgctgcctctggctctgctgctgcacgccgcccgccctcaggtccagctggtcgagtcaggaggaggcctggtgcagccaggaggcagcctgaggctgtcctgcgaggcctctggcttcaccctggactactatgccatcggctggtttaggcaggcacctggaaaggagagggagggagtgatctgtatctcccgctctgacggctctacatactatgccgatagcgtgaagggccggttcaccatctctagagacaacgccaagaagacagtgtacctgcagatgatcagcctgaagccagaggataccgcagcatactattgcgcagcaggagcagactgttccggatacctgagggattatgagtttaggggacagggaacccaggtgacagtgagctccggcggcggcggcagcgaggtgcagctggtggagtccggaggaggcctggtgcaggcaggaggcagcctgcggctgtcctgcatcgccaccggcaaggtgttcagcatctacgatatgggatggtataggcaggcaccaggaaagcagagagagctggtggccgagatcacatctagcggcaccacacactacgacgatttcgtgtccggccggtttactatttccagggacaacgccaagaatacagtgtatctgcagatgaataccctgaaggccgaggatacagccgtgtactattgtagagcaaatcatgtcttcggggggtcctattgggggcagggcactcaggtcaccgtctcctcaactagtaccacgacgccagcgccgcgaccaccaacaccggcgcccaccatcgcgtcgcagcccctgtccctgcgcccagaggcgtgccggccagcggcggggggcgcagtgcacacgagggggctggacttcgcctgtgatatctacatctgggcgcccttggccgggacttgtggggtccttctcctgtcactggttatcaccctttactgcaaacggggcagaaagaaactcctgtatatattcaaacaaccatttatgagaccagtacaaactactcaagaggaagatggctgtagctgccgatttccagaagaagaagaaggaggatgtgaactgagagtgaagttcagcaggagcgcagacgcccccgcgtaccagcagggccagaaccagctctataacgagctcaatctaggacgaagagaggagtacgatgttttggacaagagacgtggccgggaccctgagatggggggaaagccgagaaggaagaaccctcaggaaggcctgtacaatgaactgcagaaagataagatggcggaggcctacagtgagattgggatgaaaggcgagcgccggaggggcaaggggcacgatggcctttaccagggtctcagtacagccaccaaggacacctacgacgcccttcacatgcaggccctgccccctcgctaa

SEQ ID NO: 224 - DNA, 1485 bp, synthetic construct
  source 1..1485: mol_type = other DNA; note = BCMAxCD38 269A37346 38A37717 GSI5007 CAR
atggctctgcccgtcactgctctgctgctgcctctggctctgctgctgcacgccgctcgcccacaggtccagctggtcgaatcagggggaggcctggtgcagccaggaggcagcctgaggctgtcctgcgaggcctctggcttcaccctggactactatgccatcggctggtttaggcaggcacctggaaaggagagggagggagtgatctgtatctcccgctctgacggctccacatactatgccgattctgtgaagggccggttcaccatctctagagacaacgccaagaagacagtgtacctgcagatgatcagcctgaagccagaggataccgcagcatactattgcgcagcaggagcagactgttccggatacctgagggattatgagtttaggggacagggaacccaggtgacagtgagctccggaggaggaggatctggcggaggaggcagcgaggtgcagctggtggagtccggcggcggcctggtgcaggccggcggcagcctgcggctgtcctgcatcgccaccggcaaggtgttctctatctacgatatgggatggtataggcaggcaccaggaaagcagagagagctggtggccgagatcacatctagcggcaccacacactacgacgatttcgtgagcggccggtttaccatctccagagacaacgccaagaatacagtgtatctgcagatgaataccctgaaggccgaggatacagccgtgtactattgtagagccaaccatgtcttcggcgggtcatactgggggcagggaactcaggtcactgtcagcagcactagtaccacgacgccagcgccgcgaccaccaacaccggcgcccaccatcgcgtcgcagcccctgtccctgcgcccagaggcgtgccggccagcggcggggggcgcagtgcacacgagggggctggacttcgcctgtgatatctacatctgggcgcccttggccgggacttgtggggtccttctcctgtcactggttatcaccctttactgcaaacggggcagaaagaaactcctgtatatattcaaacaaccatttatgagaccagtacaaactactcaagaggaagatggctgtagctgccgatttccagaagaagaagaaggaggatgtgaactgagagtgaagttcagcaggagcgcagacgcccccgcgtaccagcagggccagaaccagctctataacgagctcaatctaggacgaagagaggagtacgatgttttggacaagagacgtggccgggaccctgagatggggggaaagccgagaaggaagaaccctcaggaaggcctgtacaatgaactgcagaaagataagatggcggaggcctacagtgagattgggatgaaaggcgagcgccggaggggcaaggggcacgatggcctttaccagggtctcagtacagccaccaaggacacctacgacgcccttcacatgcaggccctgccccctcgctaa

SEQ ID NO: 225 - DNA, 1503 bp, synthetic construct
  source 1..1503: mol_type = other DNA; note = BCMAxCD38 269A37346 38A37717 GSI5008 CAR
atggctctgcccgtcactgctctgctgctgcctctggctctgctgctgcacgccgcaaggcctcaggtccagctggtcgaatcagggggaggcctggtgcagccaggaggcagcctgaggctgtcctgcgaggcctctggcttcaccctggactactatgccatcggctggtttaggcaggcacctggaaaggagagggagggagtgatctgtatctcccgctctgacggcagcacatactatgccgattccgtgaagggccggttcaccatctccagagacaacgccaagaagacagtgtacctgcagatgatctctctgaagccagaggataccgcagcatactattgcgcagcaggagcagactgttccggatacctgagggattatgagtttaggggacagggaacccaggtgacagtgagctccggaggaggaagcggaggaggatccggaggcggctctggcggcggcagcgaggtgcagctggtggagtccggcggcggcctggtgcaggccggcggctccctgcggctgtcttgcatcgccaccggcaaggtgttcagcatctacgatatgggatggtataggcaggcaccaggaaagcagagagagctggtggccgagatcacatctagcggcaccacacactacgacgatttcgtgtctggccggtttaccatcagtagggacaacgccaagaatacagtgtatctgcagatgaataccctgaaggccgaggatacagccgtgtactattgtagagctaaccatgtcttcggggggtcatactgggggcagggcactcaggtcactgtctcatccactagtaccacgacgccagcgccgcgaccaccaacaccggcgcccaccatcgcgtcgcagcccctgtccctgcgcccagaggcgtgccggccagcggcggggggcgcagtgcacacgagggggctggacttcgcctgtgatatctacatctgggcgcccttggccgggacttgtggggtccttctcctgtcactggttatcaccctttactgcaaacggggcagaaagaaactcctgtatatattcaaacaaccatttatgagaccagtacaaactactcaagaggaagatggctgtagctgccgatttccagaagaagaagaaggaggatgtgaactgagagtgaagttcagcaggagcgcagacgcccccgcgtaccagcagggccagaaccagctctataacgagctcaatctaggacgaagagaggagtacgatgttttggacaagagacgtggccgggaccctgagatggggggaaagccgagaaggaagaaccctcaggaaggcctgtacaatgaactgcagaaagataagatggcggaggcctacagtgagattgggatgaaaggcgagcgccggaggggcaaggggcacgatggcctttaccagggtctcagtacagccaccaaggacacctacgacgcccttcacatgcaggccctgccccctcgctaa

SEQ ID NO: 226 - DNA, 1533 bp, synthetic construct
  source 1..1533: mol_type = other DNA; note = BCMAxCD38 269A37346 38A37717 GSI5009 CAR
atggctctgcccgtcaccgcactgctgctgcctctggctctgctgctgcacgccgcaaggcctcaggtccagctggtcgaatcagggggaggcctggtgcagccaggaggctctctgaggctgagctgcgaggcatccggattcaccctggactactatgccatcggctggtttaggcaggcacctggaaaggagagggagggagtgatctgtatctcccgctctgacggcagcacatactatgccgattccgtgaagggccggttcaccatcagcagagacaacgccaagaagacagtgtacctgcagatgatctccctgaagccagaggataccgcagcatactattgcgcagcaggagcagactgttctggatacctgagggattatgagtttaggggacagggaacccaggtgacagtgagctccggaggaggaggatccggcggaggaggctctggcggcggcggcggcggcagcggctccggcggcggcggctccgaggtgcagctggtggagtctggaggaggcctggtgcaggcaggaggctctctgcggctgagctgcatcgccaccggcaaggtgttcagcatctacgatatgggatggtataggcaggcaccaggaaagcagagagagctggtggccgagatcacatctagcggcaccacacactacgacgatttcgtgtctggccggtttactatttccagggacaacgccaagaatacagtgtatctgcagatgaataccctgaaggccgaggatacagccgtgtactattgtagagctaatcacgtcttcggcggctcttattgggggcagggaactcaggtcactgtgtcatccactagtactagtaccacgacgccagcgccgcgaccaccaacaccggcgcccaccatcgcgtcgcagcccctgtccctgcgcccagaggcgtgccggccagcggcggggggcgcagtgcacacgagggggctggacttcgcctgtgatatctacatctgggcgcccttggccgggacttgtggggtccttctcctgtcactggttatcaccctttactgcaaacggggcagaaagaaactcctgtatatattcaaacaaccatttatgagaccagtacaaactactcaagaggaagatggctgtagctgccgatttccagaagaagaagaaggaggatgtgaactgagagtgaagttcagcaggagcgcagacgcccccgcgtaccagcagggccagaaccagctctataacgagctcaatctaggacgaagagaggagtacgatgttttggacaagagacgtggccgggaccctgagatggggggaaagccgagaaggaagaaccctcaggaaggcctgtacaatgaactgcagaaagataagatggcggaggcctacagtgagattgggatgaaaggcgagcgccggaggggcaaggggcacgatggcctttaccagggtctcagtacagccaccaaggacacctacgacgcccttcacatgcaggccctgccccctcgctaa

SEQ ID NO: 227 - DNA, 1557 bp, synthetic construct
  source 1..1557: mol_type = other DNA; note = BCMAxCD38 269A37346 38A37717 GSI5010 CAR
atggctctgcccgtcaccgctctgctgctgcccctggctctgctgctgcacgctgctcgccctcaggtccagctggtcgaatcaggaggaggcctggtgcagccaggaggctctctgaggctgagctgcgaggcatccggattcaccctggactactatgccatcggctggtttaggcaggcacctggaaaggagagggagggagtgatctgtatctcccgctctgacggcagcacatactatgccgattccgtgaagggccggttcaccatctccagagacaacgccaagaagacagtgtacctgcagatgatctctctgaagccagaggataccgcagcatactattgcgcagcaggagcagactgtagcggatacctgagggattatgagtttaggggacagggaacccaggtgacagtgagctccggaggaggaggatccggcggaggaggctctggaggcggcggcggcggcagcggctcaggaggcggaggaagcggcggcggcggctccggcggcggcggctctgaggtgcagctggtggagagcggaggaggcctggtgcaggcaggaggctctctgcggctgagctgcatcgccaccggcaaggtgttctccatctacgatatgggatggtataggcaggcaccaggaaagcagagagagctggtggccgagatcacatctagcggcaccacacactacgacgatttcgtgtctggccggtttaccatcagtagggacaacgccaagaatacagtgtatctgcagatgaataccctgaaggccgaggatacagccgtgtactattgtagagctaatcatgtgtttggagggtcatactgggggcagggaactcaggtcactgtctcatcaactagtaccacgacgccagcgccgcgaccaccaacaccggcgcccaccatcgcgtcgcagcccctgtccctgcgcccagaggcgtgccggccagcggcggggggcgcagtgcacacgagggggctggacttcgcctgtgatatctacatctgggcgcccttggccgggacttgtggggtccttctcctgtcactggttatcaccctttactgcaaacggggcagaaagaaactcctgtatatattcaaacaaccatttatgagaccagtacaaactactcaagaggaagatggctgtagctgccgatttccagaagaagaagaaggaggatgtgaactgagagtgaagttcagcaggagcgcagacgcccccgcgtaccagcagggccagaaccagctctataacgagctcaatctaggacgaagagaggagtacgatgttttggacaagagacgtggccgggaccctgagatggggggaaagccgagaaggaagaaccctcaggaaggcctgtacaatgaactgcagaaagataagatggcggaggcctacagtgagattgggatgaaaggcgagcgccggaggggcaaggggcacgatggcctttaccagggtctcagtacagccaccaaggacacctacgacgcccttcacatgcaggccctgccccctcgctaa

SEQ ID NO: 228 - DNA, 663 bp, synthetic construct
  source 1..663: mol_type = other DNA; note = CD28 TM and CD28-CD3 zeta intracellular signaling domain
attgaagttatgtatcctcctccttacctagacaatgagaagagcaatggaaccattatccatgtgaaagggaaacacctttgtccaagtcccctatttcccggaccttctaagcccttttgggtgctggtggtggttggtggagtcctggcttgctatagcttgctagtaacagtggcctttattattttctgggtgaggagtaagaggagcaggctcctgcacagtgactacatgaacatgactccccgccgccccgggcccacccgcaagcattaccagccctatgccccaccacgcgacttcgcagcctatcgctccagagtgaagttcagcaggagcgcagacgcccccgcgtaccagcagggccagaaccagctctataacgagctcaatctaggacgaagagaggagtacgatgttttggacaagagacgtggccgggaccctgagatggggggaaagccgagaaggaagaaccctcaggaaggcctgtacaatgaactgcagaaagataagatggcggaggcctacagtgagattgggatgaaaggcgagcgccggaggggcaaggggcacgatggcctttaccagggtctcagtacagccaccaaggacacctacgacgcccttcacatgcaggccctgccccctcgctgataa

SEQ ID NO: 229 - DNA, 23 bp, synthetic construct
  source 1..23: mol_type = other DNA; note = upstream primer CALL001
gtcctggctgctcttctacaagg

SEQ ID NO: 230 - DNA, 23 bp, synthetic construct
  source 1..23: mol_type = other DNA; note = downstream primer CALLOO2
ggtacgtgctgttgaactgttcc

SEQ ID NO: 231 - DNA, 29 bp, synthetic construct
  source 1..29: mol_type = other DNA; note = upstream primer BACK-1
gatgtgcagctgcaggagtctggaggagg

SEQ ID NO: 232 - DNA, 29 bp, synthetic construct
  source 1..29: mol_type = other DNA; note = downstream primer BACK-2
gatgtgcagctgcaggagtctgggggagg

SEQ ID NO: 233 - DNA, 34 bp, synthetic construct
  source 1..34: mol_type = other DNA; note = downstream primer PMCF
ctagtgcggccgctgaggagacggtgacctgggt

SEQ ID NO: 234-238 - skipped (5 entries)

SEQ ID NO: 239 - DNA, 2307 bp, synthetic construct
  source 1..2307: mol_type = other DNA; note = tandem BCMA, CD38 269A37346 38A37717 GSI5013 CAR
atggccttaccagtgaccgccttgctcctgccgctggccttgctgctccacgccgccaggccggttaacgaggtgcagctggtggaaagcggggggggactggtgcaggcaggcgggtcactgagactgtcatgtatcgcaactgggaaggtgtttagcatctacgacatgggctggtataggcaggcaccaggaaagcagagggagctggtggccgagatcaccagctccggcaccacacactacgacgatttcgtgtctggccggtttaccatcagcagagacaacgccaagaatacagtgtatctgcagatgaacaccctgaaggccgaggatacagccgtgtactattgccgggctaatcacgtcttcggcggctcctactgggggcagggaactcaggtcactgtgtcatccacgcgtcgcatgcatactagtaccacgacgccagcgccgcgaccaccaacaccggcgcccaccatcgcgtcgcagcccctgtccctgcgcccagaggcgtgccggccagcggcggggggcgcagtgcacacgagggggctggacttcgcctgtgatatctacatctgggcgcccttggccgggacttgtggggtccttctcctgtcactggttatcaccctttactgcaaacggggcagaaagaaactcctgtatatattcaaacaaccatttatgagaccagtacaaactactcaagaggaagatggctgtagctgccgatttccagaagaagaagaaggaggatgtgaactgagagtgaagttcagcaggagcgcagacgcccccgcgtaccagcagggccagaaccagctctataacgagctcaatctaggacgaagagaggagtacgatgttttggacaagagacgtggccgggaccctgagatggggggaaagccgagaaggaagaaccctcaggaaggcctgtacaatgaactgcagaaagataagatggcggaggcctacagtgagattgggatgaaaggcgagcgccggaggggcaaggggcacgatggcctttaccagggtctcagtacagccaccaaggacacctacgacgcccttcacatgcaggccctgccccctcgcggcagtggagagggcagaggaagtctgctaacatgcggtgacgtcgaggagaatcctggcccaggatccatggccttaccagtgaccgccttgctcctgccgctggccttgctgctccacgccgccaggccggttaaccgcacgcgtcgcatgcatcaggtgcagctggtggagtctgggggaggcttggtgcagcctgggggttctctgaggctctcctgtgaagcctctggattcactttggattattatgccataggctggttccgccaggccccagggaaggagcgcgagggggtcatatgtattagtagaagtgatggtagcacatactatgcagactccgtgaagggccgattcaccatctccagagacaacgccaagaaaacggtgtatctgcaaatgatcagcctgaaacctgaggacacggccgcttattactgtgcagcaggggccgattgttcggggtacctacgagattatgagttccgggggcaggggacccaggtcaccgtctcctcaactagtaccacgacgccagcgccgcgaccaccaacaccggcgcccaccatcgcgtcgcagcccctgtccctgcgcccagaggcgtgccggccagcggcggggggcgcagtgcacacgagggggctggacttcgcctgtgatatctacatctgggcgcccttggccgggacttgtggggtccttctcctgtcactggttatcaccctttactgcaaacggggcagaaagaaactcctgtatatattcaaacaaccatttatgagaccagtacaaactactcaagaggaagatggctgtagctgccgatttccagaagaagaagaaggaggatgtgaactgagagtgaagttcagcaggagcgcagacgcccccgcgtaccagcagggccagaaccagctctataacgagctcaatctaggacgaagagaggagtacgatgttttggacaagagacgtggccgggaccctgagatggggggaaagccgagaaggaagaaccctcaggaaggcctgtacaatgaactgcagaaagataagatggcggaggcctacagtgagattgggatgaaaggcgagcgccggaggggcaaggggcacgatggcctttaccagggtctcagtacagccaccaaggacacctacgacgcccttcacatgcaggccctgccccctcgctaa

SEQ ID NO: 240 - protein, 30 aa, synthetic construct
  source 1..30: note = CD19 VHH FR1
QVKLEESGGELVQPGGPLRLSCAASGNIFS

SEQ ID NO: 241 - protein, 14 aa, synthetic construct
  source 1..14: note = CD19 VHH FR2
WYRQAPGKQRAFVA

SEQ ID NO: 242 - protein, 32 aa, synthetic construct
  source 1..32: note = CD19 VHH FR3
RFTISVDKSKNTIYLQMNALKPEDTAVYYCNA

SEQ ID NO: 243 - protein, 11 aa, synthetic construct
  source 1..11: note = CD19 VHH FR4
WGQGTQVTVSS

SEQ ID NO: 244 - protein, 30 aa, synthetic construct
  source 1..30: note = CD20 VHH FR1
PVQLVESGGGLVQAGDSLRLSCAASGRTFG

SEQ ID NO: 245 - protein, 14 aa, synthetic construct
  source 1..14: note = CD20 VHH FR2
WFRQPPGKEREFVA

SEQ ID NO: 246 - protein, 32 aa, synthetic construct
  source 1..32: note = CD20 VHH FR3
RFTISRDNAKLTVDLQMDSLKPEDTAVYYCAA

SEQ ID NO: 247 - protein, 11 aa, synthetic construct
  source 1..11: note = CD20 VHH FR4
WGQGTQVTVSS

SEQ ID NO: 248 - protein, 357 aa, synthetic construct
  source 1..357: note = CD19 CAR
MALPVTALLLPLALLLHAARPQVKLEESGGELVQPGGPLRLSCAASGNIFSINRMGWYRQAPGKQRAFVASITVRGITNYADSVKGRFTISVDKSKNTIYLQMNALKPEDTAVYYCNAVSSNRDPDYWGQGTQVTVSSIEVMYPPPYLDNEKSNGTIIHVKGKHLCPSPLFPGPSKPFWVLVVVGGVLACYSLLVTVAFIIFWVRSKRSRLLHSDYMNMTPRRPGPTRKHYQPYAPPRDFAAYRSRVKFSRSADAPAYQQGQNQLYNELNLGRREEYDVLDKRRGRDPEMGGKPRRKNPQEGLYNELQKDKMAEAYSEIGMKGERRRGKGHDGLYQGLSTATKDTYDALHMQALPPR

SEQ ID NO: 249 - protein, 369 aa, synthetic construct
  source 1..369: note = CD20 CAR
MALPVTALLLPLALLLHAARPPVQLVESGGGLVQAGDSLRLSCAASGRTFGIGTMGWFRQPPGKEREFVAAIRWSTGGTRYADSVKGRFTISRDNAKLTVDLQMDSLKPEDTAVYYCAADRLSLDLSGRYHYNPAVYDYWGQGTQVTVSSIEVMYPPPYLDNEKSNGTIIHVKGKHLCPSPLFPGPSKPFWVLVVVGGVLACYSLLVTVAFIIFWVRSKRSRLLHSDYMNMTPRRPGPTRKHYQPYAPPRDFAAYRSRVKFSRSADAPAYQQGQNQLYNELNLGRREEYDVLDKRRGRDPEMGGKPRRKNPQEGLYNELQKDKMAEAYSEIGMKGERRRGKGHDGLYQGLSTATKDTYDALHMQALPPR

SEQ ID NO: 250 - DNA, 1077 bp, synthetic construct
  source 1..1077: mol_type = other DNA; note = CD19 CAR
atggccttaccagtgaccgccttgctcctgccgctggccttgctgctccacgccgccaggccgcaggtaaagctggaggagtctgggggagaattggtgcagcctggggggcctctgagactctcctgtgcagcctcgggaaacatcttcagtatcaatcgcatgggctggtaccgccaggctccagggaagcagcgcgcgttcgtcgcatctattactgttcgtggtataacaaactatgcagactccgtgaagggccgattcaccatttctgtagacaagtccaaaaacacgatttatctgcagatgaacgcactcaaacctgaggacacggccgtctattattgtaatgcagtgtcttcaaacagggaccccgactactggggccaggggacccaggtcaccgtctcctcaattgaagttatgtatcctcctccttacctagacaatgagaagagcaatggaaccattatccatgtgaaagggaaacacctttgtccaagtcccctatttcccggaccttctaagcccttttgggtgctggtggtggttggtggagtcctggcttgctatagcttgctagtaacagtggcctttattattttctgggtgaggagtaagaggagcaggctcctgcacagtgactacatgaacatgactccccgccgccccgggcccacccgcaagcattaccagccctatgccccaccacgcgacttcgcagcctatcgctccagagtgaagttcagcaggagcgcagacgcccccgcgtaccagcagggccagaaccagctctataacgagctcaatctaggacgaagagaggagtacgatgttttggacaagagacgtggccgggaccctgagatggggggaaagccgagaaggaagaaccctcaggaaggcctgtacaatgaactgcagaaagataagatggcggaggcctacagtgagattgggatgaaaggcgagcgccggaggggcaaggggcacgatggcctttaccagggtctcagtacagccaccaaggacacctacgacgcccttcacatgcaggccctgccccctcgctgataa

SEQ ID NO: 251 - DNA, 1113 bp, synthetic construct
  source 1..1113: mol_type = other DNA; note = CD20 CAR
atggccttaccagtgaccgccttgctcctgccgctggccttgctgctccacgccgccaggccgccggtgcagctggtggagtctgggggaggcttggtgcaggctggggattctctgagactctcctgtgctgcctctggacgcaccttcggtattggtaccatgggctggttccgccaacctccagggaaggagcgtgaatttgtagcagctattaggtggagtactggtggcactcgctatgcagactccgtgaagggccgattcaccatctcccgagacaacgccaagctcacggtagatctgcaaatggacagcctgaaacctgaagacacggccgtttattactgtgcagcagatagactgtcccttgatttaagtggtcgttaccactacaaccccgccgtgtatgactattggggccaggggacccaggtcaccgtctcctcaattgaagttatgtatcctcctccttacctagacaatgagaagagcaatggaaccattatccatgtgaaagggaaacacctttgtccaagtcccctatttcccggaccttctaagcccttttgggtgctggtggtggttggtggagtcctggcttgctatagcttgctagtaacagtggcctttattattttctgggtgaggagtaagaggagcaggctcctgcacagtgactacatgaacatgactccccgccgccccgggcccacccgcaagcattaccagccctatgccccaccacgcgacttcgcagcctatcgctccagagtgaagttcagcaggagcgcagacgcccccgcgtaccagcagggccagaaccagctctataacgagctcaatctaggacgaagagaggagtacgatgttttggacaagagacgtggccgggaccctgagatggggggaaagccgagaaggaagaaccctcaggaaggcctgtacaatgaactgcagaaagataagatggcggaggcctacagtgagattgggatgaaaggcgagcgccggaggggcaaggggcacgatggcctttaccagggtctcagtacagccaccaaggacacctacgacgcccttcacatgcaggccctgccccctcgctgataa

SEQ ID NO: 252 - DNA, 23 bp, synthetic construct
  source 1..23: mol_type = other DNA; note = 137P2F primer
gtccttctcctgtcactggttat

SEQ ID NO: 253 - DNA, 23 bp, synthetic construct
  source 1..23: mol_type = other DNA; note = 137P2R primer
tcttcttcttctggaaatcggca

SEQ ID NO: 254 - DNA, 48 bp, synthetic construct
  source 1..48: mol_type = other DNA; note = Linker sequence 3
ggcggcggcagcggcggcggcagcggcggcggcagcggcggcggcagc

SEQ ID NO: 255 - protein, 21 aa, synthetic construct
  source 1..21: note = T2A
GSGEGRGSLLTCGDVEENPGP

SEQ ID NO: 256 - DNA, 63 bp, synthetic construct
  source 1..63: mol_type = other DNA; note = T2A
ggcagtggagagggcagaggaagtctgctaacatgcggtgacgtcgaggagaatcctggccca

SEQ ID NO: 257 - protein, 376 aa, synthetic construct
  source 1..376: note = GSI5011 CAR 269A37346
MALPVTALLLPLALLLHAARPVNRTRRMHQVQLVESGGGLVQPGGSLRLSCEASGFTLDYYAIGWFRQAPGKEREGVICISRSDGSTYYADSVKGRFTISRDNAKKTVYLQMISLKPEDTAAYYCAAGADCSGYLRDYEFRGQGTQVTVSSTSTTTPAPRPPTPAPTIASQPLSLRPEACRPAAGGAVHTRGLDFACDIYIWAPLAGTCGVLLLSLVITLYCKRGRKKLLYIFKQPFMRPVQTTQEEDGCSCRFPEEEEGGCELRVKFSRSADAPAYQQGQNQLYNELNLGRREEYDVLDKRRGRDPEMGGKPRRKNPQEGLYNELQKDKMAEAYSEIGMKGERRRGKGHDGLYQGLSTATKDTYDALHMQALPPR

SEQ ID NO: 258 - protein, 373 aa, synthetic construct
  source 1..373: note = GSI5019 CAR 269A37353
MALPVTALLLPLALLLHAARPVNRTRRMHQVKLEESGGGLVQAGRSLRLSCAASEHTFSSHVMGWFRQAPGKERESVAVIGWRDISTSYADSVKGRFTISRDNAKKTLYLQMNSLKPEDTAVYYCAARRIDAADFDSWGQGTQVTVSSTSTTTPAPRPPTPAPTIASQPLSLRPEACRPAAGGAVHTRGLDFACDIYIWAPLAGTCGVLLLSLVITLYCKRGRKKLLYIFKQPFMRPVQTTQEEDGCSCRFPEEEEGGCELRVKFSRSADAPAYQQGQNQLYNELNLGRREEYDVLDKRRGRDPEMGGKPRRKNPQEGLYNELQKDKMAEAYSEIGMKGERRRGKGHDGLYQGLSTATKDTYDALHMQALPPR

SEQ ID NO: 259 - protein, 372 aa, synthetic construct
  source 1..372: note = GSI5020 CAR 269A37917
MALPVTALLLPLALLLHAARPVNRTRRMHEVQLVESGGGLVQAGGSLRLSCAASGRTFTMGWFRQAPGKEREFVAAISLSPTLAYYAESVKGRFTISRDNAKNTVVLQMNSLKPEDTALYYCAADRKSVMSIRPDYWGQGTQVTVSSTSTTTPAPRPPTPAPTIASQPLSLRPEACRPAAGGAVHTRGLDFACDIYIWAPLAGTCGVLLLSLVITLYCKRGRKKLLYIFKQPFMRPVQTTQEEDGCSCRFPEEEEGGCELRVKFSRSADAPAYQQGQNQLYNELNLGRREEYDVLDKRRGRDPEMGGKPRRKNPQEGLYNELQKDKMAEAYSEIGMKGERRRGKGHDGLYQGLSTATKDTYDALHMQALPPR

SEQ ID NO: 260 - protein, 369 aa, synthetic construct
  source 1..369: note = GSI5012 CAR 38A37717
MALPVTALLLPLALLLHAARPVNEVQLVESGGGLVQAGGSLRLSCIATGKVFSIYDMGWYRQAPGKQRELVAEITSSGTTHYDDFVSGRFTISRDNAKNTVYLQMNTLKAEDTAVYYCRANHVFGGSYWGQGTQVTVSSTRRMHTSTTTPAPRPPTPAPTIASQPLSLRPEACRPAAGGAVHTRGLDFACDIYIWAPLAGTCGVLLLSLVITLYCKRGRKKLLYIFKQPFMRPVQTTQEEDGCSCRFPEEEEGGCELRVKFSRSADAPAYQQGQNQLYNELNLGRREEYDVLDKRRGRDPEMGGKPRRKNPQEGLYNELQKDKMAEAYSEIGMKGERRRGKGHDGLYQGLSTATKDTYDALHMQALPPR

SEQ ID NO: 261 - DNA, 1131 bp, synthetic construct
  source 1..1131: mol_type = other DNA; note = GSI5011 CAR 269A37346
atggccttaccagtgaccgccttgctcctgccgctggccttgctgctccacgccgccaggccggttaaccgcacgcgtcgcatgcatcaggtgcagctggtggagtctgggggaggcttggtgcagcctgggggttctctgaggctctcctgtgaagcctctggattcactttggattattatgccataggctggttccgccaggccccagggaaggagcgcgagggggtcatatgtattagtagaagtgatggtagcacatactatgcagactccgtgaagggccgattcaccatctccagagacaacgccaagaaaacggtgtatctgcaaatgatcagcctgaaacctgaggacacggccgcttattactgtgcagcaggggccgattgttcggggtacctacgagattatgagttccgggggcaggggacccaggtcaccgtctcctcaactagtaccacgacgccagcgccgcgaccaccaacaccggcgcccaccatcgcgtcgcagcccctgtccctgcgcccagaggcgtgccggccagcggcggggggcgcagtgcacacgagggggctggacttcgcctgtgatatctacatctgggcgcccttggccgggacttgtggggtccttctcctgtcactggttatcaccctttactgcaaacggggcagaaagaaactcctgtatatattcaaacaaccatttatgagaccagtacaaactactcaagaggaagatggctgtagctgccgatttccagaagaagaagaaggaggatgtgaactgagagtgaagttcagcaggagcgcagacgcccccgcgtaccagcagggccagaaccagctctataacgagctcaatctaggacgaagagaggagtacgatgttttggacaagagacgtggccgggaccctgagatggggggaaagccgagaaggaagaaccctcaggaaggcctgtacaatgaactgcagaaagataagatggcggaggcctacagtgagattgggatgaaaggcgagcgccggaggggcaaggggcacgatggcctttaccagggtctcagtacagccaccaaggacacctacgacgcccttcacatgcaggccctgccccctcgctaa

SEQ ID NO: 262 - DNA, 1122 bp, synthetic construct
  source 1..1122: mol_type = other DNA; note = GSI5019 CAR 269A37353
atggccttaccagtgaccgccttgctcctgccgctggccttgctgctccacgccgccaggccggttaaccgcacgcgtcgcatgcatcaggtaaagctggaggagtctgggggaggcttggtgcaggctgggcggtctctgagactctcctgtgcagcctctgaacacaccttcagtagccatgtcatgggctggttccgccaggctccagggaaggagcgtgagtctgttgcagttattggctggagagatattagcacaagctatgcagactccgtgaagggccgattcaccatctccagagacaacgccaagaagacgctgtatctgcaaatgaatagcctgaaacctgaggacacggccgtttactactgtgcagcacgtcggatcgacgcagctgactttgattcctgggggcaggggacccaggtcaccgtctcctcgactagtaccacgacgccagcgccgcgaccaccaacaccggcgcccaccatcgcgtcgcagcccctgtccctgcgcccagaggcgtgccggccagcggcggggggcgcagtgcacacgagggggctggacttcgcctgtgatatctacatctgggcgcccttggccgggacttgtggggtccttctcctgtcactggttatcaccctttactgcaaacggggcagaaagaaactcctgtatatattcaaacaaccatttatgagaccagtacaaactactcaagaggaagatggctgtagctgccgatttccagaagaagaagaaggaggatgtgaactgagagtgaagttcagcaggagcgcagacgcccccgcgtaccagcagggccagaaccagctctataacgagctcaatctaggacgaagagaggagtacgatgttttggacaagagacgtggccgggaccctgagatggggggaaagccgagaaggaagaaccctcaggaaggcctgtacaatgaactgcagaaagataagatggcggaggcctacagtgagattgggatgaaaggcgagcgccggaggggcaaggggcacgatggcctttaccagggtctcagtacagccaccaaggacacctacgacgcccttcacatgcaggccctgccccctcgctaa

SEQ ID NO: 263 - DNA, 1119 bp, synthetic construct
  source 1..1119: mol_type = other DNA; note = GSI5020 CAR 269A37917
atggccttaccagtgaccgccttgctcctgccgctggccttgctgctccacgccgccaggccggttaaccgcacgcgtcgcatgcatgaggtgcagctggtggagtctgggggaggcttggtgcaggctggggggtctctgagactctcctgtgcagcctctggacgcaccttcaccatggggtggttccgtcaggctccagggaaggagcgtgagtttgtagcagctattagtttgagtcctactttagcatattatgcagagtccgtgaagggccgattcaccatcagccgagacaacgccaagaacacggtggttttgcaaatgaacagcctgaaacctgaggacacggccctttattactgtgcagcagaccggaaatcagtaatgtctattcggcccgactactggggccaggggacccaggtcaccgtctcctcaactagtaccacgacgccagcgccgcgaccaccaacaccggcgcccaccatcgcgtcgcagcccctgtccctgcgcccagaggcgtgccggccagcggcggggggcgcagtgcacacgagggggctggacttcgcctgtgatatctacatctgggcgcccttggccgggacttgtggggtccttctcctgtcactggttatcaccctttactgcaaacggggcagaaagaaactcctgtatatattcaaacaaccatttatgagaccagtacaaactactcaagaggaagatggctgtagctgccgatttccagaagaagaagaaggaggatgtgaactgagagtgaagttcagcaggagcgcagacgcccccgcgtaccagcagggccagaaccagctctataacgagctcaatctaggacgaagagaggagtacgatgttttggacaagagacgtggccgggaccctgagatggggggaaagccgagaaggaagaaccctcaggaaggcctgtacaatgaactgcagaaagataagatggcggaggcctacagtgagattgggatgaaaggcgagcgccggaggggcaaggggcacgatggcctttaccagggtctcagtacagccaccaaggacacctacgacgcccttcacatgcaggccctgccccctcgctaa

SEQ ID NO: 264 - DNA, 1110 bp, synthetic construct
  source 1..1110: mol_type = other DNA; note = GSI5012 CAR 38A37717
atggccttaccagtgaccgccttgctcctgccgctggccttgctgctccacgccgccaggccggttaacgaggtgcagctggtggaaagcggggggggactggtgcaggcaggcgggtcactgagactgtcatgtatcgcaactgggaaggtgtttagcatctacgacatgggctggtataggcaggcaccaggaaagcagagggagctggtggccgagatcaccagctccggcaccacacactacgacgatttcgtgtctggccggtttaccatcagcagagacaacgccaagaatacagtgtatctgcagatgaacaccctgaaggccgaggatacagccgtgtactattgccgggctaatcacgtcttcggcggctcctactgggggcagggaactcaggtcactgtgtcatccacgcgtcgcatgcatactagtaccacgacgccagcgccgcgaccaccaacaccggcgcccaccatcgcgtcgcagcccctgtccctgcgcccagaggcgtgccggccagcggcggggggcgcagtgcacacgagggggctggacttcgcctgtgatatctacatctgggcgcccttggccgggacttgtggggtccttctcctgtcactggttatcaccctttactgcaaacggggcagaaagaaactcctgtatatattcaaacaaccatttatgagaccagtacaaactactcaagaggaagatggctgtagctgccgatttccagaagaagaagaaggaggatgtgaactgagagtgaagttcagcaggagcgcagacgcccccgcgtaccagcagggccagaaccagctctataacgagctcaatctaggacgaagagaggagtacgatgttttggacaagagacgtggccgggaccctgagatggggggaaagccgagaaggaagaaccctcaggaaggcctgtacaatgaactgcagaaagataagatggcggaggcctacagtgagattgggatgaaaggcgagcgccggaggggcaaggggcacgatggcctttaccagggtctcagtacagccaccaaggacacctacgacgcccttcacatgcaggccctgccccctcgctaa

SEQ ID NO: 265 - protein, 488 aa, synthetic construct
  source 1..488: note = GSI5021 CAR
MALPVTALLLPLALLLHAARPQVKLEESGGGLVQAGRSLRLSCAASEHTFSSHVMGWFRQAPGKERESVAVIGWRDISTSYADSVKGRFTISRDNAKKTLYLQMNSLKPEDTAVYYCAARRIDAADFDSWGQGTQVTVSSGGGGSEVQLVESGGGLVQAGGSLRLSCAASGRTFTMGWFRQAPGKEREFVAAISLSPTLAYYAESVKGRFTISRDNAKNTVVLQMNSLKPEDTALYYCAADRKSVMSIRPDYWGQGTQVTVSSTSTTTPAPRPPTPAPTIASQPLSLRPEACRPAAGGAVHTRGLDFACDIYIWAPLAGTCGVLLLSLVITLYCKRGRKKLLYIFKQPFMRPVQTTQEEDGCSCRFPEEEEGGCELRVKFSRSADAPAYQQGQNQLYNELNLGRREEYDVLDKRRGRDPEMGGKPRRKNPQEGLYNELQKDKMAEAYSEIGMKGERRRGKGHDGLYQGLSTATKDTYDALHMQALPPR

SEQ ID NO: 266 - protein, 498 aa, synthetic construct
  source 1..498: note = GSI5022 CAR
MALPVTALLLPLALLLHAARPQVKLEESGGGLVQAGRSLRLSCAASEHTFSSHVMGWFRQAPGKERESVAVIGWRDISTSYADSVKGRFTISRDNAKKTLYLQMNSLKPEDTAVYYCAARRIDAADFDSWGQGTQVTVSSGGGGSGGGGSGGGGSEVQLVESGGGLVQAGGSLRLSCAASGRTFTMGWFRQAPGKEREFVAAISLSPTLAYYAESVKGRFTISRDNAKNTVVLQMNSLKPEDTALYYCAADRKSVMSIRPDYWGQGTQVTVSSTSTTTPAPRPPTPAPTIASQPLSLRPEACRPAAGGAVHTRGLDFACDIYIWAPLAGTCGVLLLSLVITLYCKRGRKKLLYIFKQPFMRPVQTTQEEDGCSCRFPEEEEGGCELRVKFSRSADAPAYQQGQNQLYNELNLGRREEYDVLDKRRGRDPEMGGKPRRKNPQEGLYNELQKDKMAEAYSEIGMKGERRRGKGHDGLYQGLSTATKDTYDALHMQALPPR

SEQ ID NO: 267 - protein, 508 aa, synthetic construct
  source 1..508: note = GSI5023 CAR
MALPVTALLLPLALLLHAARPQVKLEESGGGLVQAGRSLRLSCAASEHTFSSHVMGWFRQAPGKERESVAVIGWRDISTSYADSVKGRFTISRDNAKKTLYLQMNSLKPEDTAVYYCAARRIDAADFDSWGQGTQVTVSSGGGGSGGGGSGGGGSGGGGSGGGGSEVQLVESGGGLVQAGGSLRLSCAASGRTFTMGWFRQAPGKEREFVAAISLSPTLAYYAESVKGRFTISRDNAKNTVVLQMNSLKPEDTALYYCAADRKSVMSIRPDYWGQGTQVTVSSTSTTTPAPRPPTPAPTIASQPLSLRPEACRPAAGGAVHTRGLDFACDIYIWAPLAGTCGVLLLSLVITLYCKRGRKKLLYIFKQPFMRPVQTTQEEDGCSCRFPEEEEGGCELRVKFSRSADAPAYQQGQNQLYNELNLGRREEYDVLDKRRGRDPEMGGKPRRKNPQEGLYNELQKDKMAEAYSEIGMKGERRRGKGHDGLYQGLSTATKDTYDALHMQALPPR

SEQ ID NO: 268 - protein, 493 aa, synthetic construct
  source 1..493: note = GSI5024 CAR
MALPVTALLLPLALLLHAARPEVQLVESGGGLVQAGGSLRLSCAASGRTFTMGWFRQAPGKEREFVAAISLSPTLAYYAESVKGRFTISRDNAKNTVVLQMNSLKPEDTALYYCAADRKSVMSIRPDYWGQGTQVTVSSGGGGSGGGGSQVKLEESGGGLVQAGRSLRLSCAASEHTFSSHVMGWFRQAPGKERESVAVIGWRDISTSYADSVKGRFTISRDNAKKTLYLQMNSLKPEDTAVYYCAARRIDAADFDSWGQGTQVTVSSTSTTTPAPRPPTPAPTIASQPLSLRPEACRPAAGGAVHTRGLDFACDIYIWAPLAGTCGVLLLSLVITLYCKRGRKKLLYIFKQPFMRPVQTTQEEDGCSCRFPEEEEGGCELRVKFSRSADAPAYQQGQNQLYNELNLGRREEYDVLDKRRGRDPEMGGKPRRKNPQEGLYNELQKDKMAEAYSEIGMKGERRRGKGHDGLYQGLSTATKDTYDALHMQALPPR

SEQ ID NO: 269 - protein, 498 aa, synthetic construct
  source 1..498: note = GSI5025 CAR
MALPVTALLLPLALLLHAARPEVQLVESGGGLVQAGGSLRLSCAASGRTFTMGWFRQAPGKEREFVAAISLSPTLAYYAESVKGRFTISRDNAKNTVVLQMNSLKPEDTALYYCAADRKSVMSIRPDYWGQGTQVTVSSGGGGSGGGGSGGGGSQVKLEESGGGLVQAGRSLRLSCAASEHTFSSHVMGWFRQAPGKERESVAVIGWRDISTSYADSVKGRFTISRDNAKKTLYLQMNSLKPEDTAVYYCAARRIDAADFDSWGQGTQVTVSSTSTTTPAPRPPTPAPTIASQPLSLRPEACRPAAGGAVHTRGLDFACDIYIWAPLAGTCGVLLLSLVITLYCKRGRKKLLYIFKQPFMRPVQTTQEEDGCSCRFPEEEEGGCELRVKFSRSADAPAYQQGQNQLYNELNLGRREEYDVLDKRRGRDPEMGGKPRRKNPQEGLYNELQKDKMAEAYSEIGMKGERRRGKGHDGLYQGLSTATKDTYDALHMQALPPR

SEQ ID NO: 270 - protein, 503 aa, synthetic construct
  source 1..503: note = GSI5026 CAR
MALPVTALLLPLALLLHAARPEVQLVESGGGLVQAGGSLRLSCAASGRTFTMGWFRQAPGKEREFVAAISLSPTLAYYAESVKGRFTISRDNAKNTVVLQMNSLKPEDTALYYCAADRKSVMSIRPDYWGQGTQVTVSSGGGGSGGGGSGGGGSGGGGSQVKLEESGGGLVQAGRSLRLSCAASEHTFSSHVMGWFRQAPGKERESVAVIGWRDISTSYADSVKGRFTISRDNAKKTLYLQMNSLKPEDTAVYYCAARRIDAADFDSWGQGTQVTVSSTSTTTPAPRPPTPAPTIASQPLSLRPEACRPAAGGAVHTRGLDFACDIYIWAPLAGTCGVLLLSLVITLYCKRGRKKLLYIFKQPFMRPVQTTQEEDGCSCRFPEEEEGGCELRVKFSRSADAPAYQQGQNQLYNELNLGRREEYDVLDKRRGRDPEMGGKPRRKNPQEGLYNELQKDKMAEAYSEIGMKGERRRGKGHDGLYQGLSTATKDTYDALHMQALPPR

SEQ ID NO: 271 - DNA, 1467 bp, synthetic construct
  source 1..1467: mol_type = other DNA; note = GSI5021 CAR
atggctctgcccgtcaccgctctgctgctgcctctggctctgctgctgcacgctgctcgccctcaggtcaaactggaagaatctggcggaggcctggtgcaggcaggacggagcctgcgcctgagctgcgcagcatccgagcacaccttcagctcccacgtgatgggctggtttcggcaggccccaggcaaggagagagagagcgtggccgtgatcggctggagggacatctccacatcttacgccgattccgtgaagggccggttcaccatcagccgggacaacgccaagaagacactgtatctgcagatgaacagcctgaagcccgaggacaccgccgtgtactattgcgcagcaaggagaatcgacgcagcagactttgattcctggggccagggcacccaggtgacagtgtctagcggaggaggaggatctgaggtgcagctggtggagagcggaggcggcctggtgcaggccggaggctctctgaggctgagctgtgcagcatccggaagaaccttcacaatgggctggtttaggcaggcaccaggaaaggagagggagttcgtggcagcaatcagcctgtcccctaccctggcctactatgccgagagcgtgaagggcaggtttaccatctcccgcgataacgccaagaatacagtggtgctgcagatgaactccctgaaacctgaggacacagccctgtactattgtgccgccgatcggaagagcgtgatgagcattagaccagactattgggggcagggaacacaggtgaccgtgagcagcactagtaccacgacgccagcgccgcgaccaccaacaccggcgcccaccatcgcgtcgcagcccctgtccctgcgcccagaggcgtgccggccagcggcggggggcgcagtgcacacgagggggctggacttcgcctgtgatatctacatctgggcgcccttggccgggacttgtggggtccttctcctgtcactggttatcaccctttactgcaaacggggcagaaagaaactcctgtatatattcaaacaaccatttatgagaccagtacaaactactcaagaggaagatggctgtagctgccgatttccagaagaagaagaaggaggatgtgaactgagagtgaagttcagcaggagcgcagacgcccccgcgtaccagcagggccagaaccagctctataacgagctcaatctaggacgaagagaggagtacgatgttttggacaagagacgtggccgggaccctgagatggggggaaagccgagaaggaagaaccctcaggaaggcctgtacaatgaactgcagaaagataagatggcggaggcctacagtgagattgggatgaaaggcgagcgccggaggggcaaggggcacgatggcctttaccagggtctcagtacagccaccaaggacacctacgacgcccttcacatgcaggccctgccccctcgctaa

SEQ ID NO: 272 - DNA, 1497 bp, synthetic construct
  source 1..1497: mol_type = other DNA; note = GSI5022 CAR
atggctctgcctgtcaccgctctgctgctgcctctggctctgctgctgcacgctgctcgccctcaggtcaaactggaagaaagtgggggaggcctggtgcaggcaggacggagcctgcgcctgagctgcgcagcatccgagcacaccttcagctcccacgtgatgggctggtttcggcaggccccaggcaaggagagagagtccgtggccgtgatcggctggagggacatctccacatcttacgccgattctgtgaagggccggttcaccatcagcagagacaacgccaagaagacactgtatctgcagatgaatagcctgaagcccgaggacaccgccgtgtactattgcgcagcaaggagaatcgacgcagcagactttgattcctggggccagggcacccaggtgacagtgtctagcggaggaggaggatctggaggaggaggaagcggaggaggaggatccgaggtgcagctggtggagtctggaggcggcctggtgcaggccggaggctctctgaggctgagctgtgcagcatccggaagaaccttcacaatgggctggtttaggcaggcaccaggaaaggagagggagttcgtggcagcaatcagcctgtcccctaccctggcctactatgccgagtccgtgaagggcaggtttaccatctctcgcgataacgccaagaatacagtggtgctgcagatgaacagcctgaaacctgaggacacagccctgtactattgtgccgccgatcggaagagcgtgatgagcattagacccgattattggggacagggcacacaggtgacagtgagtagcactagtaccacgacgccagcgccgcgaccaccaacaccggcgcccaccatcgcgtcgcagcccctgtccctgcgcccagaggcgtgccggccagcggcggggggcgcagtgcacacgagggggctggacttcgcctgtgatatctacatctgggcgcccttggccgggacttgtggggtccttctcctgtcactggttatcaccctttactgcaaacggggcagaaagaaactcctgtatatattcaaacaaccatttatgagaccagtacaaactactcaagaggaagatggctgtagctgccgatttccagaagaagaagaaggaggatgtgaactgagagtgaagttcagcaggagcgcagacgcccccgcgtaccagcagggccagaaccagctctataacgagctcaatctaggacgaagagaggagtacgatgttttggacaagagacgtggccgggaccctgagatggggggaaagccgagaaggaagaaccctcaggaaggcctgtacaatgaactgcagaaagataagatggcggaggcctacagtgagattgggatgaaaggcgagcgccggaggggcaaggggcacgatggcctttaccagggtctcagtacagccaccaaggacacctacgacgcccttcacatgcaggccctgccccctcgctaa

SEQ ID NO: 273 - DNA, 1527 bp, synthetic construct
  source 1..1527: mol_type = other DNA; note = GSI5023 CAR
atggctctgcccgtcaccgcactgctgctgcctctggctctgctgctgcacgccgcaagaccacaggtcaaactggaagaatcaggaggaggcctggtgcaggcaggacggagcctgcgcctgagctgcgcagcatccgagcacaccttcagctcccacgtgatgggctggtttcggcaggccccaggcaaggagagagagtccgtggccgtgatcggctggagggacatctccacatcttacgccgattccgtgaagggccggttcaccatcagccgggacaacgccaagaagacactgtatctgcagatgaacagcctgaagcccgaggacaccgccgtgtactattgcgcagcaaggagaatcgacgcagcagactttgatagctggggccagggcacccaggtgacagtgtctagcggaggaggaggatctggaggaggaggaagcggaggaggaggaagcggcggcggcggctctggcggcggcggcagcgaggtgcagctggtggagagcggcggcggcctggtgcaggccggcggctctctgaggctgagctgtgcagcatccggaagaaccttcacaatgggctggtttaggcaggcaccaggaaaggagagggagttcgtggcagcaatcagcctgtcccctaccctggcctactatgccgagagcgtgaagggcaggtttaccatctcccgcgataacgccaagaatacagtggtgttacaaatgaacagcctgaaacctgaggacacagccctgtactattgtgccgccgatcggaagagcgtgatgagcattagacccgattattgggggcaggggacacaggtgaccgtgagcagcactagtaccacgacgccagcgccgcgaccaccaacaccggcgcccaccatcgcgtcgcagcccctgtccctgcgcccagaggcgtgccggccagcggcggggggcgcagtgcacacgagggggctggacttcgcctgtgatatctacatctgggcgcccttggccgggacttgtggggtccttctcctgtcactggttatcaccctttactgcaaacggggcagaaagaaactcctgtatatattcaaacaaccatttatgagaccagtacaaactactcaagaggaagatggctgtagctgccgatttccagaagaagaagaaggaggatgtgaactgagagtgaagttcagcaggagcgcagacgcccccgcgtaccagcagggccagaaccagctctataacgagctcaatctaggacgaagagaggagtacgatgttttggacaagagacgtggccgggaccctgagatggggggaaagccgagaaggaagaaccctcaggaaggcctgtacaatgaactgcagaaagataagatggcggaggcctacagtgagattgggatgaaaggcgagcgccggaggggcaaggggcacgatggcctttaccagggtctcagtacagccaccaaggacacctacgacgcccttcacatgcaggccctgccccctcgctaa

SEQ ID NO: 274 - DNA, 1482 bp, synthetic construct
  source 1..1482: mol_type = other DNA; note = GSI5024 CAR
atggctctgcctgtgaccgcactgctgctgcctctggctctgctgctgcacgccgcacgacctgaagtccagctggtggaatccgggggaggcctggtgcaggcaggaggctccctgaggctgtcttgcgcagcaagcggaagaaccttcacaatgggctggtttaggcaggcaccaggaaaggagagggagttcgtggccgccatctccctgtctcctaccctggcctactatgccgagagcgtgaagggcaggtttaccatctcccgcgacaacgccaagaatacagtggtgctgcagatgaacagcctgaagccagaggacacagccctgtactattgcgccgccgatcggaagtctgtgatgagcatcagacccgattactggggccagggcacccaggtgacagtgagctccggaggaggaggatccggcggaggaggctctcaggtgaagctggaggagtccggaggcggcctggtgcaggccggacggtccctgagactgtcttgtgccgccagcgagcacaccttctctagccacgtgatgggatggttcaggcaggcacctggaaaggagagggagtccgtggcagtgatcggatggagggacatcagcacatcctacgccgattctgtgaagggccggttcaccatcagcagagacaacgccaagaagacactgtatttacaaatgaacagcctgaagcccgaggataccgccgtgtactattgtgccgcccggcggattgacgccgcagactttgactcatgggggcagggaactcaggtgaccgtgtcctcaactagtaccacgacgccagcgccgcgaccaccaacaccggcgcccaccatcgcgtcgcagcccctgtccctgcgcccagaggcgtgccggccagcggcggggggcgcagtgcacacgagggggctggacttcgcctgtgatatctacatctgggcgcccttggccgggacttgtggggtccttctcctgtcactggttatcaccctttactgcaaacggggcagaaagaaactcctgtatatattcaaacaaccatttatgagaccagtacaaactactcaagaggaagatggctgtagctgccgatttccagaagaagaagaaggaggatgtgaactgagagtgaagttcagcaggagcgcagacgcccccgcgtaccagcagggccagaaccagctctataacgagctcaatctaggacgaagagaggagtacgatgttttggacaagagacgtggccgggaccctgagatggggggaaagccgagaaggaagaaccctcaggaaggcctgtacaatgaactgcagaaagataagatggcggaggcctacagtgagattgggatgaaaggcgagcgccggaggggcaaggggcacgatggcctttaccagggtctcagtacagccaccaaggacacctacgacgcccttcacatgcaggccctgccccctcgctaa

SEQ ID NO: 275 - DNA, 1497 bp, synthetic construct
  source 1..1497: mol_type = other DNA; note = GSI5025 CAR
atggccctgcctgtcaccgctctgctgctgcccctggccctgctgctgcacgccgcacgccctgaggtccagctggtcgagtccgggggaggcctggtgcaggcaggaggctccctgaggctgtcttgcgcagcaagcggaagaaccttcacaatgggctggtttaggcaggcaccaggaaaggagagggagttcgtggccgccatctccctgtctcctaccctggcctactatgccgagtccgtgaagggcaggtttaccatctctcgcgacaacgccaagaatacagtggtgctgcagatgaactccctgaagccagaggacacagccctgtactattgcgccgccgatcggaagtctgtgatgagcatcagacccgattactggggccagggcacccaggtgacagtgagctccggaggaggaggatccggcggaggaggctctggcggcggcggcagccaggtgaagctggaggagagcggaggcggcctggtgcaggccggacggtccctgagactgtcttgtgccgccagcgagcacaccttctctagccacgtgatgggatggttcaggcaggcacctggaaaggagagggagtctgtggccgtgatcggctggagggacatcagcacatcctacgccgatagcgtgaagggccggttcaccatctccagagacaacgccaagaagacactgtatctgcagatgaatagcctgaagcccgaggataccgccgtgtactattgtgccgcccggcggattgacgccgcagattttgattcttgggggcagggaactcaggtgaccgtgtcctcaactagtaccacgacgccagcgccgcgaccaccaacaccggcgcccaccatcgcgtcgcagcccctgtccctgcgcccagaggcgtgccggccagcggcggggggcgcagtgcacacgagggggctggacttcgcctgtgatatctacatctgggcgcccttggccgggacttgtggggtccttctcctgtcactggttatcaccctttactgcaaacggggcagaaagaaactcctgtatatattcaaacaaccatttatgagaccagtacaaactactcaagaggaagatggctgtagctgccgatttccagaagaagaagaaggaggatgtgaactgagagtgaagttcagcaggagcgcagacgcccccgcgtaccagcagggccagaaccagctctataacgagctcaatctaggacgaagagaggagtacgatgttttggacaagagacgtggccgggaccctgagatggggggaaagccgagaaggaagaaccctcaggaaggcctgtacaatgaactgcagaaagataagatggcggaggcctacagtgagattgggatgaaaggcgagcgccggaggggcaaggggcacgatggcctttaccagggtctcagtacagccaccaaggacacctacgacgcccttcacatgcaggccctgccccctcgctaa

SEQ ID NO: 276 - DNA, 1512 bp, synthetic construct
  source 1..1512: mol_type = other DNA; note = GSI5026 CAR
atggctctgcctgtgaccgccctgctgctgcccctggccctgctgctgcacgccgcacgacctgaagtccagctggtggaatctggcggaggcctggtgcaggcaggaggctccctgaggctgtcttgcgcagcaagcggaagaaccttcacaatgggctggtttaggcaggcaccaggaaaggagagggagttcgtggccgccatctccctgtctcctaccctggcctactatgccgagtctgtgaagggcaggtttaccatcagccgcgacaacgccaagaatacagtggtgctgcagatgaacagcctgaagccagaggacacagccctgtactattgcgccgccgatcggaagtctgtgatgagcatcagacccgattactggggccagggcacccaggtgacagtgagctccggaggaggaggatccggcggaggaggctctggcggcggcggctccggcggcggcggctcccaggtgaagctggaggagtccggaggcggcctggtgcaggccggacggtccctgagactgtcttgtgccgccagcgagcacaccttctctagccacgtgatgggatggttcaggcaggcacctggaaaggagagggagagcgtggcagtgatcggatggagggacatcagcacatcctacgccgattccgtgaagggccggttcaccatcagccgggacaacgccaagaagacactgtatttacaaatgaacagcctgaagcccgaggataccgccgtgtactattgtgccgcccggcggattgatgccgcagactttgatagttggggacaggggactcaggtcaccgtcagcagcactagtaccacgacgccagcgccgcgaccaccaacaccggcgcccaccatcgcgtcgcagcccctgtccctgcgcccagaggcgtgccggccagcggcggggggcgcagtgcacacgagggggctggacttcgcctgtgatatctacatctgggcgcccttggccgggacttgtggggtccttctcctgtcactggttatcaccctttactgcaaacggggcagaaagaaactcctgtatatattcaaacaaccatttatgagaccagtacaaactactcaagaggaagatggctgtagctgccgatttccagaagaagaagaaggaggatgtgaactgagagtgaagttcagcaggagcgcagacgcccccgcgtaccagcagggccagaaccagctctataacgagctcaatctaggacgaagagaggagtacgatgttttggacaagagacgtggccgggaccctgagatggggggaaagccgagaaggaagaaccctcaggaaggcctgtacaatgaactgcagaaagataagatggcggaggcctacagtgagattgggatgaaaggcgagcgccggaggggcaaggggcacgatggcctttaccagggtctcagtacagccaccaaggacacctacgacgcccttcacatgcaggccctgccccctcgctaa

SEQ ID NO: 277 - protein, 768 aa, synthetic construct
  source 1..768: note = tandem BCMA, CD38 269A37346 38A37717 GSI5013 CARs
MALPVTALLLPLALLLHAARPVNEVQLVESGGGLVQAGGSLRLSCIATGKVFSIYDMGWYRQAPGKQRELVAEITSSGTTHYDDFVSGRFTISRDNAKNTVYLQMNTLKAEDTAVYYCRANHVFGGSYWGQGTQVTVSSTRRMHTSTTTPAPRPPTPAPTIASQPLSLRPEACRPAAGGAVHTRGLDFACDIYIWAPLAGTCGVLLLSLVITLYCKRGRKKLLYIFKQPFMRPVQTTQEEDGCSCRFPEEEEGGCELRVKFSRSADAPAYQQGQNQLYNELNLGRREEYDVLDKRRGRDPEMGGKPRRKNPQEGLYNELQKDKMAEAYSEIGMKGERRRGKGHDGLYQGLSTATKDTYDALHMQALPPRGSGEGRGSLLTCGDVEENPGPGSMALPVTALLLPLALLLHAARPVNRTRRMHQVQLVESGGGLVQPGGSLRLSCEASGFTLDYYAIGWFRQAPGKEREGVICISRSDGSTYYADSVKGRFTISRDNAKKTVYLQMISLKPEDTAAYYCAAGADCSGYLRDYEFRGQGTQVTVSSTSTTTPAPRPPTPAPTIASQPLSLRPEACRPAAGGAVHTRGLDFACDIYIWAPLAGTCGVLLLSLVITLYCKRGRKKLLYIFKQPFMRPVQTTQEEDGCSCRFPEEEEGGCELRVKFSRSADAPAYQQGQNQLYNELNLGRREEYDVLDKRRGRDPEMGGKPRRKNPQEGLYNELQKDKMAEAYSEIGMKGERRRGKGHDGLYQGLSTATKDTYDALHMQALPPR